European Patent Specification EP 3 390 632 B1, published September 10, 2025. Title: METHODS AND COMPOSITIONS FOR POL-II BASED GUIDE RNA EXPRESSION. Applicant: E. I. du Pont de Nemours and Company Bendezu, Felipe  Oseas Fan, Xiaochun Frisch, Ryan L HONG, SEUNG-PYO. The sequence listing filed with the application follows.

SEQUENCE LISTING (70 sequences)

SEQ ID NO: 1 - protein, 1372 aa, Streptococcus pyogenes
MDKKYSIGLDIGTNSVGWAVITDEYKVPSKKFKVLGNTDRHSIKKNLIGALLFDSGETAEATRLKRTARRRYTRRKNRICYLQEIFSNEMAKVDDSFFHRLEESFLVEEDKKHERHPIFGNIVDEVAYHEKYPTIYHLRKKLVDSTDKADLRLIYLALAHMIKFRGHFLIEGDLNPDNSDVDKLFIQLVQTYNQLFEENPINASGVDAKAILSARLSKSRRLENLIAQLPGEKKNGLFGNLIALSLGLTPNFKSNFDLAEDAKLQLSKDTYDDDLDNLLAQIGDQYADLFLAAKNLSDAILLSDILRVNTEITKAPLSASMIKRYDEHHQDLTLLKALVRQQLPEKYKEIFFDQSKNGYAGYIDGGASQEEFYKFIKPILEKMDGTEELLVKLNREDLLRKQRTFDNGSIPHQIHLGELHAILRRQEDFYPFLKDNREKIEKILTFRIPYYVGPLARGNSRFAWMTRKSEETITPWNFEEVVDKGASAQSFIERMTNFDKNLPNEKVLPKHSLLYEYFTVYNELTKVKYVTEGMRKPAFLSGEQKKAIVDLLFKTNRKVTVKQLKEDYFKKIECFDSVEISGVEDRFNASLGTYHDLLKIIKDKDFLDNEENEDILEDIVLTLTLFEDREMIEERLKTYAHLFDDKVMKQLKRRRYTGWGRLSRKLINGIRDKQSGKTILDFLKSDGFANRNFMQLIHDDSLTFKEDIQKAQVSGQGDSLHEHIANLAGSPAIKKGILQTVKVVDELVKVMGRHKPENIVIEMARENQTTQKGQKNSRERMKRIEEGIKELGSQILKEHPVENTQLQNEKLYLYYLQNGRDMYVDQELDINRLSDYDVDHIVPQSFLKDDSIDNKVLTRSDKNRGKSDNVPSEEVVKKMKNYWRQLLNAKLITQRKFDNLTKAERGGLSELDKAGFIKRQLVETRQITKHVAQILDSRMNTKYDENDKLIREVKVITLKSKLVSDFRKDFQFYKVREINNYHHAHDAYLNAVVGTALIKKYPKLESEFVYGDYKVYDVRKMIAKSEQEIGKATAKYFFYSNIMNFFKTEITLANGEIRKRPLIETNGETGEIVWDKGRDFATVRKVLSMPQVNIVKKTEVQTGGFSKESILPKRNSDKLIARKKDWDPKKYGGFDSPTVAYSVLVVAKVEKGKSKKLKSVKELLGITIMERSSFEKNPIDFLEAKGYKEVKKDLIIKLPKYSLFELENGRKRMLASAGELQKGNELALPSKYVNFLYLASHYEKLKGSPEDNEQKQLFVEQHKHYLDEIIEQISEFSKRVILADANLDKVLSAYNKHRDKPIREQAENIIHLFTLTNLGAPAAFKYFDTTIDRKRYTSTKEVLDATLIHQSITGLYETRIDLSQLGGDSRAD

SEQ ID NO: 2 - DNA, 543 bp, Yarrowia lipolytica
tcgacgtttaaaccatcatctaagggcctcaaaactacctcggaactgctgcgctgatctggacaccacagaggttccgagcactttaggttgcaccaaatgtcccaccaggtgcaggcagaaaacgctggaacagcgtgtacagtttgtcttaacaaaaagtgagggcgctgaggtcgagcagggtggtgtgacttgttatagcctttagagctgcgaaagcgcgtatggatttggctcatcaggccagattgagggtctgtggacacatgtcatgttagtgtacttcaatcgccccctggatatagccccgacaataggccgtggcctcatttttttgccttccgcacatttccattgctcggtacccacaccttgcttctcctgcacttgccaaccttaatactggtttacattgaccaacatcttacaagcggggggcttgtctagggtatatataaacagtggctctcccaatcggttgccagtctcttttttcctttctttccccacagattcgaaatctaaactacacatcacacc

SEQ ID NO: 3 - DNA, 564 bp, Artificial Sequence
  Yarrowia codon optimized P. aeruginosa Csy4
atggaccactacctggatatcagactccgacccgacccagagttccctcctgcccagctcatgtccgtcttgtttggcaagctgcaccaagctctcgtggcccagggtggagaccgaattggcgtgtcgttccccgatttggacgagtcccgttctcgacttggagaaagactccgtattcatgcttctgcagacgatctcagagctctgcttgcccgaccctggctggagggtctccgagatcatctgcagttcggcgagcctgccgtggttccccatcctaccccataccgacaggtgtctcgggttcaggccaaaagcaaccccgagcgactcagacggcgtcttatgcgaagacacgacctgtccgaggaggaagcccgaaagcggatccccgacaccgttgctcgagcgttggaccttcctttcgtcacactgcgatctcaatcgactggtcagcactttcgactgttcatcagacacggacccctgcaggtcaccgcagaggaaggcggttttacttgctatggactgtccaagggtggctttgtcccctggttctaa

SEQ ID NO: 4 - DNA, 659 bp, Artificial Sequence
  TDH1:28bp-gCAN1-28bp
cggcggactgcgtccgaaccagctccagcagcgttttttccgggccattgagccgactgcgaccccgccaacgtgtcttggcccacgcactcatgtcatgttggtgttgggaggccactttttaagtagcacaaggcacctagctcgcagcaaggtgtccgaaccaaagaagcggctgcagtggtgcaaacggggcggaaacggcgggaaaaagccacgggggcacgaattgaggcacgccctcgaatttgagacgagtcacggccccattcgcccgcgcaatggctcgccaacgcccggtcttttgcaccacatcaggttaccccaagccaaacctttgtgttaaaaagcttaacatattataccgaacgtaggtttgggcgggcttgctccgtctgtccaaggcaacatttatataagggtctgcatcgccggctcaattgaatcttttttcttcttctcttctctatattcattcttgaattaaacacacatcaacaatggttcactgccgtataggcagctaagaaatcaaacgattacccaccctcgttttagagctagaaatagcaagttaaaataaggctagtccgttatcaacttgaaaaagtggcaccgagtcggtgcttttgttcactgccgtataggcagctaagaaa

SEQ ID NO: 5 - RNA, 28 nt, Pseudomonas aeruginosa
guucacugccguauaggcagcuaagaaa

SEQ ID NO: 6 - RNA, 156 nt, Artificial Sequence
  Csy4 recognition sequence flanked sgRNA
guucacugccguauaggcagcuaagaaaucaaacgauuacccacccucguuuuagagcuagaaauagcaaguuaaaauaaggcuaguccguuaucaacuugaaaaaguggcaccgagucggugcuuuuguucacugccguauaggcagcuaagaaa

SEQ ID NO: 7 - DNA, 23 bp, Yarrowia lipolytica
tcaaacgattacccaccctccgg

SEQ ID NO: 8 - DNA, 500 bp, Yarrowia lipolytica
cggcggactgcgtccgaaccagctccagcagcgttttttccgggccattgagccgactgcgaccccgccaacgtgtcttggcccacgcactcatgtcatgttggtgttgggaggccactttttaagtagcacaaggcacctagctcgcagcaaggtgtccgaaccaaagaagcggctgcagtggtgcaaacggggcggaaacggcgggaaaaagccacgggggcacgaattgaggcacgccctcgaatttgagacgagtcacggccccattcgcccgcgcaatggctcgccaacgcccggtcttttgcaccacatcaggttaccccaagccaaacctttgtgttaaaaagcttaacatattataccgaacgtaggtttgggcgggcttgctccgtctgtccaaggcaacatttatataagggtctgcatcgccggctcaattgaatcttttttcttcttctcttctctatattcattcttgaattaaacacacatcaaca

SEQ ID NO: 9 - DNA, 585 bp, Artificial Sequence
  NLS fused to Yarrowia codon optimized P. aeruginosa Csy4
atgcccaagaagaagcgaaaagtcgaccactacctggatatcagactccgacccgacccagagttccctcctgcccagctcatgtccgtcttgtttggcaagctgcaccaagctctcgtggcccagggtggagaccgaattggcgtgtcgttccccgatttggacgagtcccgttctcgacttggagaaagactccgtattcatgcttctgcagacgatctcagagctctgcttgcccgaccctggctggagggtctccgagatcatctgcagttcggcgagcctgccgtggttccccatcctaccccataccgacaggtgtctcgggttcaggccaaaagcaaccccgagcgactcagacggcgtcttatgcgaagacacgacctgtccgaggaggaagcccgaaagcggatccccgacaccgttgctcgagcgttggaccttcctttcgtcacactgcgatctcaatcgactggtcagcactttcgactgttcatcagacacggacccctgcaggtcaccgcagaggaaggcggttttacttgctatggactgtccaagggtggctttgtcccctggttctaa

SEQ ID NO: 10 - protein, 7 aa, Simian virus 40
PKKKRKV

SEQ ID NO: 11 - DNA, 1347 bp, Artificial Sequence
  ARS18 sequence
aattcatgtcacacaaaccgatcttcgcctcaaggaaacctaattctacatccgagagactgccgagatccagtctacactgattaattttcgggccaataatttaaaaaaatcgtgttatataatattatatgtattatatatatacatcatgatgatactgacagtcatgtcccattgctaaatagacagactccatctgccgcctccaactgatgttctcaatatttaaggggtcatctcgcattgtttaataataaacagactccatctaccgcctccaaatgatgttctcaaaatatattgtatgaacttatttttattacttagtattattagacaacttacttgctttatgaaaaacacttcctatttaggaaacaatttataatggcagttcgttcatttaacaatttatgtagaataaatgttataaatgcgtatgggaaatcttaaatatggatagcataaatgatatctgcattgcctaattcgaaatcaacagcaacgaaaaaaatcccttgtacaacataaatagtcatcgagaaatatcaactatcaaagaacagctattcacacgttactattgagattattattggacgagaatcacacactcaactgtctttctctcttctagaaatacaggtacaagtatgtactattctcattgttcatacttctagtcatttcatcccacatattccttggatttctctccaatgaatgacattctatcttgcaaattcaacaattataataagatataccaaagtagcggtatagtggcaatcaaaaagcttctctggtgtgcttctcgtatttatttttattctaatgatccattaaaggtatatatttatttcttgttatataatccttttgtttattacatgggctggatacataaaggtattttgatttaattttttgcttaaattcaatcccccctcgttcagtgtcaactgtaatggtaggaaattaccatacttttgaagaagcaaaaaaaatgaaagaaaaaaaaaatcgtatttccaggttagacgttccgcagaatctagaatgcggtatgcggtacattgttcttcgaacgtaaaagttgcgctccctgagatattgtacatttttgcttttacaagtacaagtacatcgtacaactatgtactactgttgatgcatccacaacagtttgttttgtttttttttgttttttttttttctaatgattcattaccgctatgtatacctacttgtacttgtagtaagccgggttattggcgttcaattaatcatagacttatgaatctgcacggtgtgcgctgcgagttacttttagcttatgcatgc

SEQ ID NO: 12 - DNA, 1374 bp, Artificial Sequence
  full length ARS18 sequence
aattcatgtcacacaaaccgatcttcgcctcaaggaaacctaattctacatccgagagactgccgagatccagtctacactgattaattttcgggccaataatttaaaaaaatcgtgttatataatattatatgtattatatatatacatcatgatgatactgacagtcatgtcccattgctaaatagacagactccatctgccgcctccaactgatgttctcaatatttaaggggtcatctcgcattgtttaataataaacagactccatctaccgcctccaaatgatgttctcaaaatatattgtatgaacttatttttattacttagtattattagacaacttacttgctttatgaaaaacacttcctatttaggaaacaatttataatggcagttcgttcatttaacaatttatgtagaataaatgttataaatgcgtatgggaaatcttaaatatggatagcataaatgatatctgcattgcctaattcgaaatcaacagcaacgaaaaaaatcccttgtacaacataaatagtcatcgagaaatatcaactatcaaagaacagctattcacacgttactattgagattattattggacgagaatcacacactcaactgtctttctctcttctagaaatacaggtacaagtatgtactattctcattgttcatacttctagtcatttcatcccacatattccttggatttctctccaatgaatgacattctatcttgcaaattcaacaattataataagatataccaaagtagcggtatagtggcaatcaaaaagcttctctggtgtgcttctcgtatttatttttattctaatgatccattaaaggtatatatttatttcttgttatataatccttttgtttattacatgggctggatacataaaggtattttgatttaattttttgcttaaattcaatcccccctcgttcagtgtcaactgtaatggtaggaaattaccatacttttgaagaagcaaaaaaaatgaaagaaaaaaaaaatcgtatttccaggttagacgttccgcagaatctagaatgcggtatgcggtacattgttcttcgaacgtaaaagttgcgctccctgagatattgtacatttttgcttttacaagtacaagtacatcgtacaactatgtactactgttgatgcatccacaacagtttgttttgtttttttttgttttttttttttctaatgattcattaccgctatgtatacctacttgtacttgtagtaagccgggttattggcgttcaattaatcatagacttatgaatctgcacggtgtgcgctgcgagttacttttagcttatgcatgctacttgggtgtaatattgggatctgtt

SEQ ID NO: 13 - DNA, 320 bp, Yarrowia lipolytica
tagctatccgaagatcaagagcgaagcaagttgtaagtccaggacatgtttcccgcccacgcgagtgatttataacacctctcttttttgacacccgctcgccttgaaattcatgtcacataaattatagtcaacgacgtttgaataacttgtcttgtagttcgatgatgatcatatgattacattaatagtaattactgtatttgatatatatactaattacaatagtacatattagaacatacaatagttagtgccgtgaagtggcttaaaataccgcgagtcgattacgtaatattatatataatgtcaaagtgggg

SEQ ID NO: 14 - DNA, 4140 bp, Artificial sequence
  Yarrowia codon optimized Cas9
atggacaagaaatactccatcggcctggacattggaaccaactctgtcggctgggctgtcatcaccgacgagtacaaggtgccctccaagaaattcaaggtcctcggaaacaccgatcgacactccatcaagaaaaacctcattggtgccctgttgttcgattctggcgagactgccgaagctaccagactcaagcgaactgctcggcgacgttacacccgacggaagaaccgaatctgctacctgcaggagatcttttccaacgagatggccaaggtggacgattcgttctttcatcgactggaggaatccttcctcgtcgaggaagacaagaaacacgagcgtcatcccatctttggcaacattgtggacgaggttgcttaccacgagaagtatcctaccatctaccatctccgaaagaaactcgtcgattccaccgacaaggcggatctcagacttatctacctcgctctggcacacatgatcaagtttcgaggtcatttcctcatcgagggcgatctcaatcccgacaacagcgatgtggacaagctgttcattcagctcgttcagacctacaaccagctgttcgaggaaaaccccatcaatgcctccggagtcgatgcaaaggccatcttgtctgctcgactctcgaagagcagacgactggagaacctcattgcccaacttcctggcgagaaaaagaacggactgtttggcaacctcattgccctttctcttggtctcacacccaacttcaagtccaacttcgatctggcggaggacgccaagctccagctgtccaaggacacctacgacgatgacctcgacaacctgcttgcacagattggcgatcagtacgccgacctgtttctcgctgccaagaacctttcggatgctattctcttgtctgacattctgcgagtcaacaccgagatcacaaaggctcccctttctgcctccatgatcaagcgatacgacgagcaccatcaggatctcacactgctcaaggctcttgtccgacagcaactgcccgagaagtacaaggagatctttttcgatcagtcgaagaacggctacgctggatacatcgacggcggagcctctcaggaagagttctacaagttcatcaagccaattctcgagaagatggacggaaccgaggaactgcttgtcaagctcaatcgagaggatctgcttcggaagcaacgaaccttcgacaacggcagcattcctcatcagatccacctcggtgagctgcacgccattcttcgacgtcaggaagacttctacccctttctcaaggacaaccgagagaagatcgagaagattcttacctttcgaatcccctactatgttggtcctcttgccagaggaaactctcgatttgcttggatgactcgaaagtccgaggaaaccatcactccctggaacttcgaggaagtcgtggacaagggtgcctctgcacagtccttcatcgagcgaatgaccaacttcgacaagaatctgcccaacgagaaggttcttcccaagcattcgctgctctacgagtactttacagtctacaacgaactcaccaaagtcaagtacgttaccgagggaatgcgaaagcctgccttcttgtctggcgaacagaagaaagccattgtcgatctcctgttcaagaccaaccgaaaggtcactgttaagcagctcaaggaggactacttcaagaaaatcgagtgtttcgacagcgtcgagatttccggagttgaggaccgattcaacgcctctttgggcacctatcacgatctgctcaagattatcaaggacaaggattttctcgacaacgaggaaaacgaggacattctggaggacatcgtgctcactcttaccctgttcgaagatcgggagatgatcgaggaacgactcaagacatacgctcacctgttcgacgacaaggtcatgaaacaactcaagcgacgtagatacaccggctggggaagactttcgcgaaagctcatcaacggcatcagagacaagcagtccggaaagaccattctggactttctcaagtccgatggctttgccaaccgaaacttcatgcagctcattcacgacgattctcttaccttcaaggaggacatccagaaggcacaagtgtccggtcagggcgacagcttgcacgaacatattgccaacctggctggttcgccagccatcaagaaaggcattctccagactgtcaaggttgtcgacgagctggtgaaggtcatgggacgtcacaagcccgagaacattgtgatcgagatggccagagagaaccagacaactcaaaagggtcagaaaaactcgcgagagcggatgaagcgaatcgaggaaggcatcaaggagctgggatcccagattctcaaggagcatcccgtcgagaacactcaactgcagaacgagaagctgtatctctactatctgcagaatggtcgagacatgtacgtggatcaggaactggacatcaatcgtctcagcgactacgatgtggaccacattgtccctcaatcctttctcaaggacgattctatcgacaacaaggtccttacacgatccgacaagaacagaggcaagtcggacaacgttcccagcgaagaggtggtcaaaaagatgaagaactactggcgacagctgctcaacgccaagctcattacccagcgaaagttcgacaatcttaccaaggccgagcgaggcggtctgtccgagctcgacaaggctggcttcatcaagcgtcaactcgtcgagaccagacagatcacaaagcacgtcgcacagattctcgattctcggatgaacaccaagtacgacgagaacgacaagctcatccgagaggtcaaggtgattactctcaagtccaaactggtctccgatttccgaaaggactttcagttctacaaggtgcgagagatcaacaattaccaccatgcccacgatgcttacctcaacgccgtcgttggcactgcgctcatcaagaaataccccaagctcgaaagcgagttcgtttacggcgattacaaggtctacgacgttcgaaagatgattgccaagtccgaacaggagattggcaaggctactgccaagtacttcttttactccaacatcatgaactttttcaagaccgagatcaccttggccaacggagagattcgaaagagaccacttatcgagaccaacggcgaaactggagagatcgtgtgggacaagggtcgagactttgcaaccgtgcgaaaggttctgtcgatgcctcaggtcaacatcgtcaagaaaaccgaggttcagactggcggattctccaaggagtcgattctgcccaagcgaaactccgacaagctcatcgctcgaaagaaagactgggatcccaagaaatacggtggcttcgattctcctaccgtcgcctattccgtgcttgtcgttgcgaaggtcgagaagggcaagtccaaaaagctcaagtccgtcaaggagctgctcggaattaccatcatggagcgatcgagcttcgagaagaatcccatcgacttcttggaagccaagggttacaaggaggtcaagaaagacctcattatcaagctgcccaagtactctctgttcgaactggagaacggtcgaaagcgtatgctcgcctccgctggcgagctgcagaagggaaacgagcttgccttgccttcgaagtacgtcaactttctctatctggcttctcactacgagaagctcaagggttctcccgaggacaacgaacagaagcaactcttcgttgagcagcacaaacattacctcgacgagattatcgagcagatttccgagttttcgaagcgagtcatcctggctgatgccaacttggacaaggtgctctctgcctacaacaagcatcgggacaaacccattcgagaacaggcggagaacatcattcacctgtttactcttaccaacctgggtgctcctgcagctttcaagtacttcgataccactatcgaccgaaagcggtacacatccaccaaggaggttctcgatgccaccctgattcaccagtccatcactggcctgtacgagacccgaatcgacctgtctcagcttggtggcgactccagagccgatcccaagaaaaagcgaaaggtctaa

SEQ ID NO: 15 - protein, 7 aa, Simian virus 40
PKKKRKV

SEQ ID NO: 16 - DNA, 543 bp, Yarrowia lipolytica; identical to SEQ ID NO: 2

SEQ ID NO: 17 - DNA, 4683 bp, Artificial sequence
  Yarrowia optimized expression cassette
tcgacgtttaaaccatcatctaagggcctcaaaactacctcggaactgctgcgctgatctggacaccacagaggttccgagcactttaggttgcaccaaatgtcccaccaggtgcaggcagaaaacgctggaacagcgtgtacagtttgtcttaacaaaaagtgagggcgctgaggtcgagcagggtggtgtgacttgttatagcctttagagctgcgaaagcgcgtatggatttggctcatcaggccagattgagggtctgtggacacatgtcatgttagtgtacttcaatcgccccctggatatagccccgacaataggccgtggcctcatttttttgccttccgcacatttccattgctcggtacccacaccttgcttctcctgcacttgccaaccttaatactggtttacattgaccaacatcttacaagcggggggcttgtctagggtatatataaacagtggctctcccaatcggttgccagtctcttttttcctttctttccccacagattcgaaatctaaactacacatcacaccatggacaagaaatactccatcggcctggacattggaaccaactctgtcggctgggctgtcatcaccgacgagtacaaggtgccctccaagaaattcaaggtcctcggaaacaccgatcgacactccatcaagaaaaacctcattggtgccctgttgttcgattctggcgagactgccgaagctaccagactcaagcgaactgctcggcgacgttacacccgacggaagaaccgaatctgctacctgcaggagatcttttccaacgagatggccaaggtggacgattcgttctttcatcgactggaggaatccttcctcgtcgaggaagacaagaaacacgagcgtcatcccatctttggcaacattgtggacgaggttgcttaccacgagaagtatcctaccatctaccacctgcgaaagaaactcgtcgattccaccgacaaggcggatctcagacttatctacctcgctctggcacacatgatcaagtttcgaggtcatttcctcatcgagggcgatctcaatcccgacaacagcgatgtggacaagctgttcattcagctcgttcagacctacaaccagctgttcgaggaaaaccccatcaatgcctccggagtcgatgcaaaggccatcttgtctgctcgactctcgaagagcagacgactggagaacctcattgcccaacttcctggcgagaaaaagaacggactgtttggcaacctcattgccctttctcttggtctcacacccaacttcaagtccaacttcgatctggcggaggacgccaagctccagctgtccaaggacacctacgacgatgacctcgacaacctgcttgcacagattggcgatcagtacgccgacctgtttctcgctgccaagaacctttcggatgctattctcttgtctgacattctgcgagtcaacaccgagatcacaaaggctcccctttctgcctccatgatcaagcgatacgacgagcaccatcaggatctcacactgctcaaggctcttgtccgacagcaactgcccgagaagtacaaggagatctttttcgatcagtcgaagaacggctacgctggatacatcgacggcggagcctctcaggaagagttctacaagttcatcaagccaattctcgagaagatggacggaaccgaggaactgcttgtcaagctcaatcgagaggatctgcttcggaagcaacgaaccttcgacaacggcagcattcctcatcagatccacctcggtgagctgcacgccattcttcgacgtcaggaagacttctacccctttctcaaggacaaccgagagaagatcgagaagattcttacctttcgaatcccctactatgttggtcctcttgccagaggaaactctcgatttgcttggatgactcgaaagtccgaggaaaccatcactccctggaacttcgaggaagtcgtggacaagggtgcctctgcacagtccttcatcgagcgaatgaccaacttcgacaagaatctgcccaacgagaaggttcttcccaagcattcgctgctctacgagtactttacagtctacaacgaactcaccaaagtcaagtacgttaccgagggaatgcgaaagcctgccttcttgtctggcgaacagaagaaagccattgtcgatctcctgttcaagaccaaccgaaaggtcactgttaagcagctcaaggaggactacttcaagaaaatcgagtgtttcgacagcgtcgagatttccggagttgaggaccgattcaacgcctctttgggcacctatcacgatctgctcaagattatcaaggacaaggattttctcgacaacgaggaaaacgaggacattctggaggacatcgtgctcactcttaccctgttcgaagatcgggagatgatcgaggaacgactcaagacatacgctcacctgttcgacgacaaggtcatgaaacaactcaagcgacgtagatacaccggctggggaagactttcgcgaaagctcatcaacggcatcagagacaagcagtccggaaagaccattctggactttctcaagtccgatggctttgccaaccgaaacttcatgcagctcattcacgacgattctcttaccttcaaggaggacatccagaaggcacaagtgtccggtcagggcgacagcttgcacgaacatattgccaacctggctggttcgccagccatcaagaaaggcattctccagactgtcaaggttgtcgacgagctggtgaaggtcatgggacgtcacaagcccgagaacattgtgatcgagatggccagagagaaccagacaactcaaaagggtcagaaaaactcgcgagagcggatgaagcgaatcgaggaaggcatcaaggagctgggatcccagattctcaaggagcatcccgtcgagaacactcaactgcagaacgagaagctgtatctctactatctgcagaatggtcgagacatgtacgtggatcaggaactggacatcaatcgtctcagcgactacgatgtggaccacattgtccctcaatcctttctcaaggacgattctatcgacaacaaggtccttacacgatccgacaagaacagaggcaagtcggacaacgttcccagcgaagaggtggtcaaaaagatgaagaactactggcgacagctgctcaacgccaagctcattacccagcgaaagttcgacaatcttaccaaggccgagcgaggcggtctgtccgagctcgacaaggctggcttcatcaagcgtcaactcgtcgagaccagacagatcacaaagcacgtcgcacagattctcgattctcggatgaacaccaagtacgacgagaacgacaagctcatccgagaggtcaaggtgattactctcaagtccaaactggtctccgatttccgaaaggactttcagttctacaaggtgcgagagatcaacaattaccaccatgcccacgatgcttacctcaacgccgtcgttggcactgcgctcatcaagaaataccccaagctcgaaagcgagttcgtttacggcgattacaaggtctacgacgttcgaaagatgattgccaagtccgaacaggagattggcaaggctactgccaagtacttcttttactccaacatcatgaactttttcaagaccgagatcaccttggccaacggagagattcgaaagagaccacttatcgagaccaacggcgaaactggagagatcgtgtgggacaagggtcgagactttgcaaccgtgcgaaaggttctgtcgatgcctcaggtcaacatcgtcaagaaaaccgaggttcagactggcggattctccaaggagtcgattctgcccaagcgaaactccgacaagctcatcgctcgaaagaaagactgggatcccaagaaatacggtggcttcgattctcctaccgtcgcctattccgtgcttgtcgttgcgaaggtcgagaagggcaagtccaaaaagctcaagtccgtcaaggagctgctcggaattaccatcatggagcgatcgagcttcgagaagaatcccatcgacttcttggaagccaagggttacaaggaggtcaagaaagacctcattatcaagctgcccaagtactctctgttcgaactggagaacggtcgaaagcgtatgctcgcctccgctggcgagctgcagaagggaaacgagcttgccttgccttcgaagtacgtcaactttctctatctggcttctcactacgagaagctcaagggttctcccgaggacaacgaacagaagcaactcttcgttgagcagcacaaacattacctcgacgagattatcgagcagatttccgagttttcgaagcgagtcatcctggctgatgccaacttggacaaggtgctctctgcctacaacaagcatcgggacaaacccattcgagaacaggcggagaacatcattcacctgtttactcttaccaacctgggtgctcctgcagctttcaagtacttcgataccactatcgaccgaaagcggtacacatccaccaaggaggttctcgatgccaccctgattcaccagtccatcactggcctgtacgagacccgaatcgacctgtctcagcttggtggcgactccagagccgatcccaagaaaaagcgaaaggtctaa

SEQ ID NO: 18 - DNA, 10706 bp, Artificial sequence
  pZufCas9
catggacaagaaatactccatcggcctggacattggaaccaactctgtcggctgggctgtcatcaccgacgagtacaaggtgccctccaagaaattcaaggtcctcggaaacaccgatcgacactccatcaagaaaaacctcattggtgccctgttgttcgattctggcgagactgccgaagctaccagactcaagcgaactgctcggcgacgttacacccgacggaagaaccgaatctgctacctgcaggagatcttttccaacgagatggccaaggtggacgattcgttctttcatcgactggaggaatccttcctcgtcgaggaagacaagaaacacgagcgtcatcccatctttggcaacattgtggacgaggttgcttaccacgagaagtatcctaccatctaccacctgcgaaagaaactcgtcgattccaccgacaaggcggatctcagacttatctacctcgctctggcacacatgatcaagtttcgaggtcatttcctcatcgagggcgatctcaatcccgacaacagcgatgtggacaagctgttcattcagctcgttcagacctacaaccagctgttcgaggaaaaccccatcaatgcctccggagtcgatgcaaaggccatcttgtctgctcgactctcgaagagcagacgactggagaacctcattgcccaacttcctggcgagaaaaagaacggactgtttggcaacctcattgccctttctcttggtctcacacccaacttcaagtccaacttcgatctggcggaggacgccaagctccagctgtccaaggacacctacgacgatgacctcgacaacctgcttgcacagattggcgatcagtacgccgacctgtttctcgctgccaagaacctttcggatgctattctcttgtctgacattctgcgagtcaacaccgagatcacaaaggctcccctttctgcctccatgatcaagcgatacgacgagcaccatcaggatctcacactgctcaaggctcttgtccgacagcaactgcccgagaagtacaaggagatctttttcgatcagtcgaagaacggctacgctggatacatcgacggcggagcctctcaggaagagttctacaagttcatcaagccaattctcgagaagatggacggaaccgaggaactgcttgtcaagctcaatcgagaggatctgcttcggaagcaacgaaccttcgacaacggcagcattcctcatcagatccacctcggtgagctgcacgccattcttcgacgtcaggaagacttctacccctttctcaaggacaaccgagagaagatcgagaagattcttacctttcgaatcccctactatgttggtcctcttgccagaggaaactctcgatttgcttggatgactcgaaagtccgaggaaaccatcactccctggaacttcgaggaagtcgtggacaagggtgcctctgcacagtccttcatcgagcgaatgaccaacttcgacaagaatctgcccaacgagaaggttcttcccaagcattcgctgctctacgagtactttacagtctacaacgaactcaccaaagtcaagtacgttaccgagggaatgcgaaagcctgccttcttgtctggcgaacagaagaaagccattgtcgatctcctgttcaagaccaaccgaaaggtcactgttaagcagctcaaggaggactacttcaagaaaatcgagtgtttcgacagcgtcgagatttccggagttgaggaccgattcaacgcctctttgggcacctatcacgatctgctcaagattatcaaggacaaggattttctcgacaacgaggaaaacgaggacattctggaggacatcgtgctcactcttaccctgttcgaagatcgggagatgatcgaggaacgactcaagacatacgctcacctgttcgacgacaaggtcatgaaacaactcaagcgacgtagatacaccggctggggaagactttcgcgaaagctcatcaacggcatcagagacaagcagtccggaaagaccattctggactttctcaagtccgatggctttgccaaccgaaacttcatgcagctcattcacgacgattctcttaccttcaaggaggacatccagaaggcacaagtgtccggtcagggcgacagcttgcacgaacatattgccaacctggctggttcgccagccatcaagaaaggcattctccagactgtcaaggttgtcgacgagctggtgaaggtcatgggacgtcacaagcccgagaacattgtgatcgagatggccagagagaaccagacaactcaaaagggtcagaaaaactcgcgagagcggatgaagcgaatcgaggaaggcatcaaggagctgggatcccagattctcaaggagcatcccgtcgagaacactcaactgcagaacgagaagctgtatctctactatctgcagaatggtcgagacatgtacgtggatcaggaactggacatcaatcgtctcagcgactacgatgtggaccacattgtccctcaatcctttctcaaggacgattctatcgacaacaaggtccttacacgatccgacaagaacagaggcaagtcggacaacgttcccagcgaagaggtggtcaaaaagatgaagaactactggcgacagctgctcaacgccaagctcattacccagcgaaagttcgacaatcttaccaaggccgagcgaggcggtctgtccgagctcgacaaggctggcttcatcaagcgtcaactcgtcgagaccagacagatcacaaagcacgtcgcacagattctcgattctcggatgaacaccaagtacgacgagaacgacaagctcatccgagaggtcaaggtgattactctcaagtccaaactggtctccgatttccgaaaggactttcagttctacaaggtgcgagagatcaacaattaccaccatgcccacgatgcttacctcaacgccgtcgttggcactgcgctcatcaagaaataccccaagctcgaaagcgagttcgtttacggcgattacaaggtctacgacgttcgaaagatgattgccaagtccgaacaggagattggcaaggctactgccaagtacttcttttactccaacatcatgaactttttcaagaccgagatcaccttggccaacggagagattcgaaagagaccacttatcgagaccaacggcgaaactggagagatcgtgtgggacaagggtcgagactttgcaaccgtgcgaaaggttctgtcgatgcctcaggtcaacatcgtcaagaaaaccgaggttcagactggcggattctccaaggagtcgattctgcccaagcgaaactccgacaagctcatcgctcgaaagaaagactgggatcccaagaaatacggtggcttcgattctcctaccgtcgcctattccgtgcttgtcgttgcgaaggtcgagaagggcaagtccaaaaagctcaagtccgtcaaggagctgctcggaattaccatcatggagcgatcgagcttcgagaagaatcccatcgacttcttggaagccaagggttacaaggaggtcaagaaagacctcattatcaagctgcccaagtactctctgttcgaactggagaacggtcgaaagcgtatgctcgcctccgctggcgagctgcagaagggaaacgagcttgccttgccttcgaagtacgtcaactttctctatctggcttctcactacgagaagctcaagggttctcccgaggacaacgaacagaagcaactcttcgttgagcagcacaaacattacctcgacgagattatcgagcagatttccgagttttcgaagcgagtcatcctggctgatgccaacttggacaaggtgctctctgcctacaacaagcatcgggacaaacccattcgagaacaggcggagaacatcattcacctgtttactcttaccaacctgggtgctcctgcagctttcaagtacttcgataccactatcgaccgaaagcggtacacatccaccaaggaggttctcgatgccaccctgattcaccagtccatcactggcctgtacgagacccgaatcgacctgtctcagcttggtggcgactccagagccgatcccaagaaaaagcgaaaggtctaagcggccgcaagtgtggatggggaagtgagtgcccggttctgtgtgcacaattggcaatccaagatggatggattcaacacagggatatagcgagctacgtggtggtgcgaggatatagcaacggatatttatgtttgacacttgagaatgtacgatacaagcactgtccaagtacaatactaaacatactgtacatactcatactcgtacccgggcaacggtttcacttgagtgcagtggctagtgctcttactcgtacagtgtgcaatactgcgtatcatagtctttgatgtatatcgtattcattcatgttagttgcgtacgagccggaagcataaagtgtaaagcctggggtgcctaatgagtgagctaactcacattaattgcgttgcgctcactgcccgctttccagtcgggaaacctgtcgtgccagctgcattaatgaatcggccaacgcgcggggagaggcggtttgcgtattgggcgctcttccgcttcctcgctcactgactcgctgcgctcggtcgttcggctgcggcgagcggtatcagctcactcaaaggcggtaatacggttatccacagaatcaggggataacgcaggaaagaacatgtgagcaaaaggccagcaaaaggccaggaaccgtaaaaaggccgcgttgctggcgtttttccataggctccgcccccctgacgagcatcacaaaaatcgacgctcaagtcagaggtggcgaaacccgacaggactataaagataccaggcgtttccccctggaagctccctcgtgcgctctcctgttccgaccctgccgcttaccggatacctgtccgcctttctcccttcgggaagcgtggcgctttctcatagctcacgctgtaggtatctcagttcggtgtaggtcgttcgctccaagctgggctgtgtgcacgaaccccccgttcagcccgaccgctgcgccttatccggtaactatcgtcttgagtccaacccggtaagacacgacttatcgccactggcagcagccactggtaacaggattagcagagcgaggtatgtaggcggtgctacagagttcttgaagtggtggcctaactacggctacactagaaggacagtatttggtatctgcgctctgctgaagccagttaccttcggaaaaagagttggtagctcttgatccggcaaacaaaccaccgctggtagcggtggtttttttgtttgcaagcagcagattacgcgcagaaaaaaaggatctcaagaagatcctttgatcttttctacggggtctgacgctcagtggaacgaaaactcacgttaagggattttggtcatgagattatcaaaaaggatcttcacctagatccttttaaattaaaaatgaagttttaaatcaatctaaagtatatatgagtaaacttggtctgacagttaccaatgcttaatcagtgaggcacctatctcagcgatctgtctatttcgttcatccatagttgcctgactccccgtcgtgtagataactacgatacgggagggcttaccatctggccccagtgctgcaatgataccgcgagacccacgctcaccggctccagatttatcagcaataaaccagccagccggaagggccgagcgcagaagtggtcctgcaactttatccgcctccatccagtctattaattgttgccgggaagctagagtaagtagttcgccagttaatagtttgcgcaacgttgttgccattgctacaggcatcgtggtgtcacgctcgtcgtttggtatggcttcattcagctccggttcccaacgatcaaggcgagttacatgatcccccatgttgtgcaaaaaagcggttagctccttcggtcctccgatcgttgtcagaagtaagttggccgcagtgttatcactcatggttatggcagcactgcataattctcttactgtcatgccatccgtaagatgcttttctgtgactggtgagtactcaaccaagtcattctgagaatagtgtatgcggcgaccgagttgctcttgcccggcgtcaatacgggataataccgcgccacatagcagaactttaaaagtgctcatcattggaaaacgttcttcggggcgaaaactctcaaggatcttaccgctgttgagatccagttcgatgtaacccactcgtgcacccaactgatcttcagcatcttttactttcaccagcgtttctgggtgagcaaaaacaggaaggcaaaatgccgcaaaaaagggaataagggcgacacggaaatgttgaatactcatactcttcctttttcaatattattgaagcatttatcagggttattgtctcatgagcggatacatatttgaatgtatttagaaaaataaacaaataggggttccgcgcacatttccccgaaaagtgccacctgacgcgccctgtagcggcgcattaagcgcggcgggtgtggtggttacgcgcagcgtgaccgctacacttgccagcgccctagcgcccgctcctttcgctttcttcccttcctttctcgccacgttcgccggctttccccgtcaagctctaaatcgggggctccctttagggttccgatttagtgctttacggcacctcgaccccaaaaaacttgattagggtgatggttcacgtagtgggccatcgccctgatagacggtttttcgccctttgacgttggagtccacgttctttaatagtggactcttgttccaaactggaacaacactcaaccctatctcggtctattcttttgatttataagggattttgccgatttcggcctattggttaaaaaatgagctgatttaacaaaaatttaacgcgaattttaacaaaatattaacgcttacaatttccattcgccattcaggctgcgcaactgttgggaagggcgatcggtgcgggcctcttcgctattacgccagctggcgaaagggggatgtgctgcaaggcgattaagttgggtaacgccagggttttcccagtcacgacgttgtaaaacgacggccagtgaattgtaatacgactcactatagggcgaattgggtaccgggccccccctcgaggtcgatggtgtcgataagcttgatatcgaattcatgtcacacaaaccgatcttcgcctcaaggaaacctaattctacatccgagagactgccgagatccagtctacactgattaattttcgggccaataatttaaaaaaatcgtgttatataatattatatgtattatatatatacatcatgatgatactgacagtcatgtcccattgctaaatagacagactccatctgccgcctccaactgatgttctcaatatttaaggggtcatctcgcattgtttaataataaacagactccatctaccgcctccaaatgatgttctcaaaatatattgtatgaacttatttttattacttagtattattagacaacttacttgctttatgaaaaacacttcctatttaggaaacaatttataatggcagttcgttcatttaacaatttatgtagaataaatgttataaatgcgtatgggaaatcttaaatatggatagcataaatgatatctgcattgcctaattcgaaatcaacagcaacgaaaaaaatcccttgtacaacataaatagtcatcgagaaatatcaactatcaaagaacagctattcacacgttactattgagattattattggacgagaatcacacactcaactgtctttctctcttctagaaatacaggtacaagtatgtactattctcattgttcatacttctagtcatttcatcccacatattccttggatttctctccaatgaatgacattctatcttgcaaattcaacaattataataagatataccaaagtagcggtatagtggcaatcaaaaagcttctctggtgtgcttctcgtatttatttttattctaatgatccattaaaggtatatatttatttcttgttatataatccttttgtttattacatgggctggatacataaaggtattttgatttaattttttgcttaaattcaatcccccctcgttcagtgtcaactgtaatggtaggaaattaccatacttttgaagaagcaaaaaaaatgaaagaaaaaaaaaatcgtatttccaggttagacgttccgcagaatctagaatgcggtatgcggtacattgttcttcgaacgtaaaagttgcgctccctgagatattgtacatttttgcttttacaagtacaagtacatcgtacaactatgtactactgttgatgcatccacaacagtttgttttgtttttttttgttttttttttttctaatgattcattaccgctatgtatacctacttgtacttgtagtaagccgggttattggcgttcaattaatcatagacttatgaatctgcacggtgtgcgctgcgagttacttttagcttatgcatgctacttgggtgtaatattgggatctgttcggaaatcaacggatgctcaatcgatttcgacagtaattaattaagtcatacacaagtcagctttcttcgagcctcatataagtataagtagttcaacgtattagcactgtacccagcatctccgtatcgagaaacacaacaacatgccccattggacagatcatgcggatacacaggttgtgcagtatcatacatactcgatcagacaggtcgtctgaccatcatacaagctgaacaagcgctccatacttgcacgctctctatatacacagttaaattacatatccatagtctaacctctaacagttaatcttctggtaagcctcccagccagccttctggtatcgcttggcctcctcaataggatctcggttctggccgtacagacctcggccgacaattatgatatccgttccggtagacatgacatcctcaacagttcggtactgctgtccgagagcgtctcccttgtcgtcaagacccaccccgggggtcagaataagccagtcctcagagtcgcccttaggtcggttctgggcaatgaagccaaccacaaactcggggtcggatcgggcaagctcaatggtctgcttggagtactcgccagtggccagagagcccttgcaagacagctcggccagcatgagcagacctctggccagcttctcgttgggagaggggactaggaactccttgtactgggagttctcgtagtcagagacgtcctccttcttctgttcagagacagtttcctcggcaccagctcgcaggccagcaatgattccggttccgggtacaccgtgggcgttggtgatatcggaccactcggcgattcggtgacaccggtactggtgcttgacagtgttgccaatatctgcgaactttctgtcctcgaacaggaagaaaccgtgcttaagagcaagttccttgagggggagcacagtgccggcgtaggtgaagtcgtcaatgatgtcgatatgggttttgatcatgcacacataaggtccgaccttatcggcaagctcaatgagctccttggtggtggtaacatccagagaagcacacaggttggttttcttggctgccacgagcttgagcactcgagcggcaaaggcggacttgtggacgttagctcgagcttcgtaggagggcattttggtggtgaagaggagactgaaataaatttagtctgcagaactttttatcggaaccttatctggggcagtgaagtatatgttatggtaatagttacgagttagttgaacttatagatagactggactatacggctatcggtccaaattagaaagaacgtcaatggctctctgggcgtcgcctttgccgacaaaaatgtgatcatgatgaaagccagcaatgacgttgcagctgatattgttgtcggccaaccgcgccgaaaacgcagctgtcagacccacagcctccaacgaagaatgtatcgtcaaagtgatccaagcacactcatagttggagtcgtactccaaaggcggcaatgacgagtcagacagatactcgtcgacgtttaaaccatcatctaagggcctcaaaactacctcggaactgctgcgctgatctggacaccacagaggttccgagcactttaggttgcaccaaatgtcccaccaggtgcaggcagaaaacgctggaacagcgtgtacagtttgtcttaacaaaaagtgagggcgctgaggtcgagcagggtggtgtgacttgttatagcctttagagctgcgaaagcgcgtatggatttggctcatcaggccagattgagggtctgtggacacatgtcatgttagtgtacttcaatcgccccctggatatagccccgacaataggccgtggcctcatttttttgccttccgcacatttccattgctcggtacccacaccttgcttctcctgcacttgccaaccttaatactggtttacattgaccaacatcttacaagcggggggcttgtctagggtatatataaacagtggctctcccaatcggttgccagtctcttttttcctttctttccccacagattcgaaatctaaactacacatcacac

SEQ ID NO: 19 - DNA, 385 bp, Artificial sequence
  TEF1tss promoter fragment
gggttaattaaagagaccgggttggcggcgcatttgtgtcccaaaaaacagccccaattgccccaattgaccccaaattgacccagtagcgggcccaaccccggcgagagcccccttctccccacatatcaaacctcccccggttcccacacttgccgttaagggcgtagggtactgcagtctggaatctacgcttgttcagactttgtactagtttctttgtctggccatccgggtaacccatgccggacgcaaaatagactactgaaaatttttttgctttgtggttgggactttagccaagggtataaaagaccaccgtccccgaattacctttcctcttcttttctctctctccttgtcaatcaaacgattacccaccctc

SEQ ID NO: 20 - DNA, 31 bp, Artificial sequence
  tef1 promoter forward
gggttaattaaagagaccgggttggcggcgc

SEQ ID NO: 21 - DNA, 40 bp, Artificial sequence
  tef1tss promoter reverse
gagggtgggtaatcgtttgattgacaaggagagagagaaa

SEQ ID NO: 22 - DNA, 437 bp, Artificial sequence
  TEF1UTR promoter fragment
gggttaattaaagagaccgggttggcggcgcatttgtgtcccaaaaaacagccccaattgccccaattgaccccaaattgacccagtagcgggcccaaccccggcgagagcccccttctccccacatatcaaacctcccccggttcccacacttgccgttaagggcgtagggtactgcagtctggaatctacgcttgttcagactttgtactagtttctttgtctggccatccgggtaacccatgccggacgcaaaatagactactgaaaatttttttgctttgtggttgggactttagccaagggtataaaagaccaccgtccccgaattacctttcctcttcttttctctctctccttgtcaactcacacccgaaatcgttaagcatttccttctgagtataagaatcattcaaatcaaacgattacccaccctc

SEQ ID NO: 23 - DNA, 40 bp, Artificial sequence
  Tef1utr promoter reverse
gagggtgggtaatcgtttgatttgaatgattcttatactc

SEQ ID NO: 24 - DNA, 513 bp, Artificial sequence
  FBA1tss promoter fragment
gggttaattaagtttaaaccatcatctaagggcctcaaaactacctcggaactgctgcgctgatctggacaccacagaggttccgagcactttaggttgcaccaaatgtcccaccaggtgcaggcagaaaacgctggaacagcgtgtacagtttgtcttaacaaaaagtgagggcgctgaggtcgagcagggtggtgtgacttgttatagcctttagagctgcgaaagcgcgtatggatttggctcatcaggccagattgagggtctgtggacacatgtcatgttagtgtacttcaatcgccccctggatatagccccgacaataggccgtggcctcatttttttgccttccgcacatttccattgctcggtacccacaccttgcttctcctgcacttgccaaccttaatactggtttacattgaccaacatcttacaagcggggggcttgtctagggtatatataaacagtggctctcccaatcggttgccatcaaacgattacccaccctc

SEQ ID NO: 25 - DNA, 34 bp, Artificial sequence
  FBA1 promoter forward
gggttaattaagtttaaaccatcatctaagggcc

SEQ ID NO: 26 - DNA, 40 bp, Artificial sequence
  FBA1tss reverse
gagggtgggtaatcgtttgatggcaaccgattgggagagc

SEQ ID NO: 27 - DNA, 569 bp, Artificial sequence
  FBA1utr promoter fragment
gggttaattaagtttaaaccatcatctaagggcctcaaaactacctcggaactgctgcgctgatctggacaccacagaggttccgagcactttaggttgcaccaaatgtcccaccaggtgcaggcagaaaacgctggaacagcgtgtacagtttgtcttaacaaaaagtgagggcgctgaggtcgagcagggtggtgtgacttgttatagcctttagagctgcgaaagcgcgtatggatttggctcatcaggccagattgagggtctgtggacacatgtcatgttagtgtacttcaatcgccccctggatatagccccgacaataggccgtggcctcatttttttgccttccgcacatttccattgctcggtacccacaccttgcttctcctgcacttgccaaccttaatactggtttacattgaccaacatcttacaagcggggggcttgtctagggtatatataaacagtggctctcccaatcggttgccagtctcttttttcctttctttccccacagattcgaaatctaaactacacatcacacctcaaacgattacccaccctc

SEQ ID NO: 28 - DNA, 40 bp, Artificial sequence
  FBA1utr reverse
gagggtgggtaatcgtttgaggtgtgatgtgtagtttaga

SEQ ID NO: 29 - DNA, 804 bp, Artificial sequence
  ACT1 for gRNA
cttcggcatggcgaatgggaggccgcgtgtggtgattgctgttgtgcaagcctttgctcgttttctgctgtatgtaatttaaagaacgattgtatgaatcgaagtcaaggtgagtgtagtttgagaagtgtaaccccagtgtcatagctgtgtactccattcattgaagggtgtagtcgtgttttattgcatgagctcctattactcgtataagtaactgttttgtaacacttcatgaacggagatggtatgaacagaagtaataatatcctggaagtcagctgtgcccagaggtgtgtgtgggtgtggcatactttgggacaacaacacttgggcagtatgcttagtgaccacgaagagagtgttaccttctgaggtgcgacgtgcagtagttctattgtttttaaatgcgcagtcgtctttcagaggctgattcaagcagacgcattcagttgtgttcagttgaggctgatatctcagcacctacagtttagggaaagcagggttaagatgatgacaactctgggtggtaacctgggatatgcggcgatatagcaggtaatgacttaataactgctcaatgatgagtatatacatccctcctatctatatatccatatttagtatttacatattcatcttcaccgagctacaagtagaaggatgtacatgctgtatcttgcggtgcctgtcgccatgttttcgacaagttaagttcggagtatgcatgcaaacaaaaatacaagtagtcaaaatattggagtatcaaacaacgtgcttcgaaatctcttccaatcgatcccc

SEQ ID NO: 30 - DNA, 7973 bp, Artificial sequence
  pFB23
ggccgcgtgtggtgattgctgttgtgcaagcctttgctcgttttctgctgtatgtaatttaaagaacgattgtatgaatcgaagtcaaggtgagtgtagtttgagaagtgtaaccccagtgtcatagctgtgtactccattcattgaagggtgtagtcgtgttttattgcatgagctcctattactcgtataagtaactgttttgtaacacttcatgaacggagatggtatgaacagaagtaataatatcctggaagtcagctgtgcccagaggtgtgtgtgggtgtggcatactttgggacaacaacacttgggcagtatgcttagtgaccacgaagagagtgttaccttctgaggtgcgacgtgcagtagttctattgtttttaaatgcgcagtcgtctttcagaggctgattcaagcagacgcattcagttgtgttcagttgaggctgatatctcagcacctacagtttagggaaagcagggttaagatgatgacaactctgggtggtaacctgggatatgcggcgatatagcaggtaatgacttaataactgctcaatgatgagtatatacatccctcctatctatatatccatatttagtatttacatattcatcttcaccgagctacaagtagaaggatgtacatgctgtatcttgcggtgcctgtcgccatgttttcgacaagttaagttcggagtatgcatgcaaacaaaaatacaagtagtcaaaatattggagtatcaaacaacgtgcttcgaaatctcttccacaattggcaatccaagatggatggattcaacacagggatatagcgagctacgtggtggtgcgaggatatagcaacggatatttatgtttgacacttgagaatgtacgatacaagcactgtccaagtacaatactaaacatactgtacatactcatactcgtacccgggcaacggtttcacttgagtgcagtggctagtgctcttactcgtacagtgtgcaatactgcgtatcatagtctttgatgtatatcgtattcattcatgttagttgcgtacgagccggaagcataaagtgtaaagcctggggtgcctaatgagtgagctaactcacattaattgcgttgcgctcactgcccgctttccagtcgggaaacctgtcgtgccagctgcattaatgaatcggccaacgcgcggggagaggcggtttgcgtattgggcgctcttccgcttcctcgctcactgactcgctgcgctcggtcgttcggctgcggcgagcggtatcagctcactcaaaggcggtaatacggttatccacagaatcaggggataacgcaggaaagaacatgtgagcaaaaggccagcaaaaggccaggaaccgtaaaaaggccgcgttgctggcgtttttccataggctccgcccccctgacgagcatcacaaaaatcgacgctcaagtcagaggtggcgaaacccgacaggactataaagataccaggcgtttccccctggaagctccctcgtgcgctctcctgttccgaccctgccgcttaccggatacctgtccgcctttctcccttcgggaagcgtggcgctttctcatagctcacgctgtaggtatctcagttcggtgtaggtcgttcgctccaagctgggctgtgtgcacgaaccccccgttcagcccgaccgctgcgccttatccggtaactatcgtcttgagtccaacccggtaagacacgacttatcgccactggcagcagccactggtaacaggattagcagagcgaggtatgtaggcggtgctacagagttcttgaagtggtggcctaactacggctacactagaaggacagtatttggtatctgcgctctgctgaagccagttaccttcggaaaaagagttggtagctcttgatccggcaaacaaaccaccgctggtagcggtggtttttttgtttgcaagcagcagattacgcgcagaaaaaaaggatctcaagaagatcctttgatcttttctacggggtctgacgctcagtggaacgaaaactcacgttaagggattttggtcatgagattatcaaaaaggatcttcacctagatccttttaaattaaaaatgaagttttaaatcaatctaaagtatatatgagtaaacttggtctgacagttaccaatgcttaatcagtgaggcacctatctcagcgatctgtctatttcgttcatccatagttgcctgactccccgtcgtgtagataactacgatacgggagggcttaccatctggccccagtgctgcaatgataccgcgagacccacgctcaccggctccagatttatcagcaataaaccagccagccggaagggccgagcgcagaagtggtcctgcaactttatccgcctccatccagtctattaattgttgccgggaagctagagtaagtagttcgccagttaatagtttgcgcaacgttgttgccattgctacaggcatcgtggtgtcacgctcgtcgtttggtatggcttcattcagctccggttcccaacgatcaaggcgagttacatgatcccccatgttgtgcaaaaaagcggttagctccttcggtcctccgatcgttgtcagaagtaagttggccgcagtgttatcactcatggttatggcagcactgcataattctcttactgtcatgccatccgtaagatgcttttctgtgactggtgagtactcaaccaagtcattctgagaatagtgtatgcggcgaccgagttgctcttgcccggcgtcaatacgggataataccgcgccacatagcagaactttaaaagtgctcatcattggaaaacgttcttcggggcgaaaactctcaaggatcttaccgctgttgagatccagttcgatgtaacccactcgtgcacccaactgatcttcagcatcttttactttcaccagcgtttctgggtgagcaaaaacaggaaggcaaaatgccgcaaaaaagggaataagggcgacacggaaatgttgaatactcatactcttcctttttcaatattattgaagcatttatcagggttattgtctcatgagcggatacatatttgaatgtatttagaaaaataaacaaataggggttccgcgcacatttccccgaaaagtgccacctgacgcgccctgtagcggcgcattaagcgcggcgggtgtggtggttacgcgcagcgtgaccgctacacttgccagcgccctagcgcccgctcctttcgctttcttcccttcctttctcgccacgttcgccggctttccccgtcaagctctaaatcgggggctccctttagggttccgatttagtgctttacggcacctcgaccccaaaaaacttgattagggtgatggttcacgtagtgggccatcgccctgatagacggtttttcgccctttgacgttggagtccacgttctttaatagtggactcttgttccaaactggaacaacactcaaccctatctcggtctattcttttgatttataagggattttgccgatttcggcctattggttaaaaaatgagctgatttaacaaaaatttaacgcgaattttaacaaaatattaacgcttacaatttccattcgccattcaggctgcgcaactgttgggaagggcgatcggtgcgggcctcttcgctattacgccagctggcgaaagggggatgtgctgcaaggcgattaagttgggtaacgccagggttttcccagtcacgacgttgtaaaacgacggccagtgaattgtaatacgactcactatagggcgaattgggtaccgggccccccctcgaggtcgatggtgtcgataagcttgatatcgaattcatgtcacacaaaccgatcttcgcctcaaggaaacctaattctacatccgagagactgccgagatccagtctacactgattaattttcgggccaataatttaaaaaaatcgtgttatataatattatatgtattatatatatacatcatgatgatactgacagtcatgtcccattgctaaatagacagactccatctgccgcctccaactgatgttctcaatatttaaggggtcatctcgcattgtttaataataaacagactccatctaccgcctccaaatgatgttctcaaaatatattgtatgaacttatttttattacttagtattattagacaacttacttgctttatgaaaaacacttcctatttaggaaacaatttataatggcagttcgttcatttaacaatttatgtagaataaatgttataaatgcgtatgggaaatcttaaatatggatagcataaatgatatctgcattgcctaattcgaaatcaacagcaacgaaaaaaatcccttgtacaacataaatagtcatcgagaaatatcaactatcaaagaacagctattcacacgttactattgagattattattggacgagaatcacacactcaactgtctttctctcttctagaaatacaggtacaagtatgtactattctcattgttcatacttctagtcatttcatcccacatattccttggatttctctccaatgaatgacattctatcttgcaaattcaacaattataataagatataccaaagtagcggtatagtggcaatcaaaaagcttctctggtgtgcttctcgtatttatttttattctaatgatccattaaaggtatatatttatttcttgttatataatccttttgtttattacatgggctggatacataaaggtattttgatttaattttttgcttaaattcaatcccccctcgttcagtgtcaactgtaatggtaggaaattaccatacttttgaagaagcaaaaaaaatgaaagaaaaaaaaaatcgtatttccaggttagacgttccgcagaatctagaatgcggtatgcggtacattgttcttcgaacgtaaaagttgcgctccctgagatattgtacatttttgcttttacaagtacaagtacatcgtacaactatgtactactgttgatgcatccacaacagtttgttttgtttttttttgttttttttttttctaatgattcattaccgctatgtatacctacttgtacttgtagtaagccgggttattggcgttcaattaatcatagacttatgaatctgcacggtgtgcgctgcgagttacttttagcttatgcatgctacttgggtgtaatattgggatctgttcggaaatcaacggatgctcaatcgatttcgacagtaattaattaagtcatacacaagtcagctttcttcgagcctcatataagtataagtagttcaacgtattagcactgtacccagcatctccgtatcgagaaacacaacaacatgccccattggacagatcatgcggatacacaggttgtgcagtatcatacatactcgatcagacaggtcgtctgaccatcatacaagctgaacaagcgctccatacttgcacgctctctatatacacagttaaattacatatccatagtctaacctctaacagttaatcttctggtaagcctcccagccagccttctggtatcgcttggcctcctcaataggatctcggttctggccgtacagacctcggccgacaattatgatatccgttccggtagacatgacatcctcaacagttcggtactgctgtccgagagcgtctcccttgtcgtcaagacccaccccgggggtcagaataagccagtcctcagagtcgcccttaggtcggttctgggcaatgaagccaaccacaaactcggggtcggatcgggcaagctcaatggtctgcttggagtactcgccagtggccagagagcccttgcaagacagctcggccagcatgagcagacctctggccagcttctcgttgggagaggggactaggaactccttgtactgggagttctcgtagtcagagacgtcctccttcttctgttcagagacagtttcctcggcaccagctcgcaggccagcaatgattccggttccgggtacaccgtgggcgttggtgatatcggaccactcggcgattcggtgacaccggtactggtgcttgacagtgttgccaatatctgcgaactttctgtcctcgaacaggaagaaaccgtgcttaagagcaagttccttgagggggagcacagtgccggcgtaggtgaagtcgtcaatgatgtcgatatgggttttgatcatgcacacataaggtccgaccttatcggcaagctcaatgagctccttggtggtggtaacatccagagaagcacacaggttggttttcttggctgccacgagcttgagcactcgagcggcaaaggcggacttgtggacgttagctcgagcttcgtaggagggcattttggtggtgaagaggagactgaaataaatttagtctgcagaactttttatcggaaccttatctggggcagtgaagtatatgttatggtaatagttacgagttagttgaacttatagatagactggactatacggctatcggtccaaattagaaagaacgtcaatggctctctgggcgtcgcctttgccgacaaaaatgtgatcatgatgaaagccagcaatgacgttgcagctgatattgttgtcggccaaccgcgccgaaaacgcagctgtcagacccacagcctccaacgaagaatgtatcgtcaaagtgatccaagcacactcatagttggagtcgtactccaaaggcggcaatgacgagtcagacagatactcgtcgacgtttaaaccatcatctaagggcctcaaaactacctcggaactgctgcgctgatctggacaccacagaggttccgagcactttaggttgcaccaaatgtcccaccaggtgcaggcagaaaacgctggaacagcgtgtacagtttgtcttaacaaaaagtgagggcgctgaggtcgagcagggtggtgtgacttgttatagcctttagagctgcgaaagcgcgtatggatttggctcatcaggccagattgagggtctgtggacacatgtcatgttagtgtacttcaatcgccccctggatatagccccgacaataggccgtggcctcatttttttgccttccgcacatttccattgctcggtacccacaccttgcttctcctgcacttgccaaccttaatactggtttacattgaccaacatcttacaagcggggggcttgtctagggtatatataaacagtggctctcccaatcggttgccagtctcttttttcctttctttccccacagattcgaaatctaaactacacatcacaccatggcctcctcggaggacgtcatcaaggagttcatgcgattcaaggtccgaatggaaggctccgtgaacggtcacgagtttgagattgagggagagggtgaaggccgaccctacgaaggcacccagaccgcgaagctgaaggtgaccaagggtggacccctgcccttcgcctgggacattctgtctcctcagtttcagtacggttctaaggtgtacgtgaagcaccctgctgacattcccgactacaagaaactttcctttcccgagggcttcaagtgggagcgagttatgaacttcgaggatggcggtgtcgttaccgttactcaggactcctcgctccaggacggctcgttcatctacaaggttaagttcatcggtgtcaacttccctagcgatggacccgtcatgcaaaagaaaactatgggatgggaagcctctacagagcggctgtaccctcgagacggagtgttgaagggcgagattcacaaggccctgaagctcaaggacggtggacactatctcgttgagtttaagtctatctacatggcaaagaaacccgtgcagcttccaggctactattacgtcgattccaagctcgatatcaccagccataatgaggactacactattgtcgaacagtacgagcgtgctgagggaagacaccatctgtttctttaagc

SEQ ID NO: 31 - DNA, 40 bp, Artificial sequence
  Act1 CER forward
accgagtcggtggtgcttttggccgcgtgtggtgattgct

SEQ ID NO: 32 - DNA, 31 bp, Artificial sequence
  ACT1 reverse
ggggatcgattggaagagatttcgaagcacg

SEQ ID NO: 33 - DNA, 804 bp, Artificial sequence
  ACT1 for HDV gRNA
accgagtcggtggtgcttttggccgcgtgtggtgattgctgttgtgcaagcctttgctcgttttctgctgtatgtaatttaaagaacgattgtatgaatcgaagtcaaggtgagtgtagtttgagaagtgtaaccccagtgtcatagctgtgtactccattcattgaagggtgtagtcgtgttttattgcatgagctcctattactcgtataagtaactgttttgtaacacttcatgaacggagatggtatgaacagaagtaataatatcctggaagtcagctgtgcccagaggtgtgtgtgggtgtggcatactttgggacaacaacacttgggcagtatgcttagtgaccacgaagagagtgttaccttctgaggtgcgacgtgcagtagttctattgtttttaaatgcgcagtcgtctttcagaggctgattcaagcagacgcattcagttgtgttcagttgaggctgatatctcagcacctacagtttagggaaagcagggttaagatgatgacaactctgggtggtaacctgggatatgcggcgatatagcaggtaatgacttaataactgctcaatgatgagtatatacatccctcctatctatatatccatatttagtatttacatattcatcttcaccgagctacaagtagaaggatgtacatgctgtatcttgcggtgcctgtcgccatgttttcgacaagttaagttcggagtatgcatgcaaacaaaaatacaagtagtcaaaatattggagtatcaaacaacgtgcttcgaaatctcttccaatcgatcccc

SEQ ID NO: 34 - DNA, 40 bp, Artificial sequence
  ACT1 HDV forward
cttcggcatggcgaatgggaggccgcgtgtggtgattgct

SEQ ID NO: 35 - DNA, 143 bp, Artificial sequence
  Can1-1 for FBA1tss
gctctcccaatcggttgccatcaaacgattacccaccctcgttttagagctagaaatagcaagttaaaataaggctagtccgttatcaacttgaaaaagtggcaccgagtcggtggtgcttttggccgcgtgtggtgattgct

SEQ ID NO: 36 - DNA, 11568 bp, Artificial sequence
  pRF84
cgatccctgtgttgaatccatccatcttggattgccaattgtgcacacagaaccgggcactcacttccccatccacacttgcggccgcccccaagcttgtcccattcgccatgccgaagcatgttgcccagccggcgccagcgaggaggctgggaccatgccggccaaaagcaccaccgactcggtgccactttttcaagttgataacggactagccttattttaacttgctatttctagctctaaaacgagggtgggtaatcgtttgagacgagcttactcgtttcgtcctcacggactcatcagtcaaaccatggtgtgatgtgtagtttagatttcgaatctgtggggaaagaaaggaaaaaagagactggcaaccgattgggagagccactgtttatatataccctagacaagccccccgcttgtaagatgttggtcaatgtaaaccagtattaaggttggcaagtgcaggagaagcaaggtgtgggtaccgagcaatggaaatgtgcggaaggcaaaaaaatgaggccacggcctattgtcggggctatatccagggggcgattgaagtacactaacatgacatgtgtccacagaccctcaatctggcctgatgagccaaatccatacgcgctttcgcagctctaaaggctataacaagtcacaccaccctgctcgacctcagcgccctcactttttgttaagacaaactgtacacgctgttccagcgttttctgcctgcacctggtgggacatttggtgcaacctaaagtgctcggaacctctgtggtgtccagatcagcgcagcagttccgaggtagttttgaggcccttagatgatggtttaaacgtcgacgagtatctgtctgactcgttaattaagtcatacacaagtcagctttcttcgagcctcatataagtataagtagttcaacgtattagcactgtacccagcatctccgtatcgagaaacacaacaacatgccccattggacagatcatgcggatacacaggttgtgcagtatcatacatactcgatcagacaggtcgtctgaccatcatacaagctgaacaagcgctccatacttgcacgctctctatatacacagttaaattacatatccatagtctaacctctaacagttaatcttctggtaagcctcccagccagccttctggtatcgcttggcctcctcaataggatctcggttctggccgtacagacctcggccgacaattatgatatccgttccggtagacatgacatcctcaacagttcggtactgctgtccgagagcgtctcccttgtcgtcaagacccaccccgggggtcagaataagccagtcctcagagtcgcccttaggtcggttctgggcaatgaagccaaccacaaactcggggtcggatcgggcaagctcaatggtctgcttggagtactcgccagtggccagagagcccttgcaagacagctcggccagcatgagcagacctctggccagcttctcgttgggagaggggactaggaactccttgtactgggagttctcgtagtcagagacgtcctccttcttctgttcagagacagtttcctcggcaccagctcgcaggccagcaatgattccggttccgggtacaccgtgggcgttggtgatatcggaccactcggcgattcggtgacaccggtactggtgcttgacagtgttgccaatatctgcgaactttctgtcctcgaacaggaagaaaccgtgcttaagagcaagttccttgagggggagcacagtgccggcgtaggtgaagtcgtcaatgatgtcgatatgggttttgatcatgcacacataaggtccgaccttatcggcaagctcaatgagctccttggtggtggtaacatccagagaagcacacaggttggttttcttggctgccacgagcttgagcactcgagcggcaaaggcggacttgtggacgttagctcgagcttcgtaggagggcattttggtggtgaagaggagactgaaataaatttagtctgcagaactttttatcggaaccttatctggggcagtgaagtatatgttatggtaatagttacgagttagttgaacttatagatagactggactatacggctatcggtccaaattagaaagaacgtcaatggctctctgggcgtcgcctttgccgacaaaaatgtgatcatgatgaaagccagcaatgacgttgcagctgatattgttgtcggccaaccgcgccgaaaacgcagctgtcagacccacagcctccaacgaagaatgtatcgtcaaagtgatccaagcacactcatagttggagtcgtactccaaaggcggcaatgacgagtcagacagatactcgtcgacgtttaaaccatcatctaagggcctcaaaactacctcggaactgctgcgctgatctggacaccacagaggttccgagcactttaggttgcaccaaatgtcccaccaggtgcaggcagaaaacgctggaacagcgtgtacagtttgtcttaacaaaaagtgagggcgctgaggtcgagcagggtggtgtgacttgttatagcctttagagctgcgaaagcgcgtatggatttggctcatcaggccagattgagggtctgtggacacatgtcatgttagtgtacttcaatcgccccctggatatagccccgacaataggccgtggcctcatttttttgccttccgcacatttccattgctcggtacccacaccttgcttctcctgcacttgccaaccttaatactggtttacattgaccaacatcttacaagcggggggcttgtctagggtatatataaacagtggctctcccaatcggttgccagtctcttttttcctttctttccccacagattcgaaatctaaactacacatcacaccatggacaagaaatactccatcggcctggacattggaaccaactctgtcggctgggctgtcatcaccgacgagtacaaggtgccctccaagaaattcaaggtcctcggaaacaccgatcgacactccatcaagaaaaacctcattggtgccctgttgttcgattctggcgagactgccgaagctaccagactcaagcgaactgctcggcgacgttacacccgacggaagaaccgaatctgctacctgcaggagatcttttccaacgagatggccaaggtggacgattcgttctttcatcgactggaggaatccttcctcgtcgaggaagacaagaaacacgagcgtcatcccatctttggcaacattgtggacgaggttgcttaccacgagaagtatcctaccatctaccacctgcgaaagaaactcgtcgattccaccgacaaggcggatctcagacttatctacctcgctctggcacacatgatcaagtttcgaggtcatttcctcatcgagggcgatctcaatcccgacaacagcgatgtggacaagctgttcattcagctcgttcagacctacaaccagctgttcgaggaaaaccccatcaatgcctccggagtcgatgcaaaggccatcttgtctgctcgactctcgaagagcagacgactggagaacctcattgcccaacttcctggcgagaaaaagaacggactgtttggcaacctcattgccctttctcttggtctcacacccaacttcaagtccaacttcgatctggcggaggacgccaagctccagctgtccaaggacacctacgacgatgacctcgacaacctgcttgcacagattggcgatcagtacgccgacctgtttctcgctgccaagaacctttcggatgctattctcttgtctgacattctgcgagtcaacaccgagatcacaaaggctcccctttctgcctccatgatcaagcgatacgacgagcaccatcaggatctcacactgctcaaggctcttgtccgacagcaactgcccgagaagtacaaggagatctttttcgatcagtcgaagaacggctacgctggatacatcgacggcggagcctctcaggaagagttctacaagttcatcaagccaattctcgagaagatggacggaaccgaggaactgcttgtcaagctcaatcgagaggatctgcttcggaagcaacgaaccttcgacaacggcagcattcctcatcagatccacctcggtgagctgcacgccattcttcgacgtcaggaagacttctacccctttctcaaggacaaccgagagaagatcgagaagattcttacctttcgaatcccctactatgttggtcctcttgccagaggaaactctcgatttgcttggatgactcgaaagtccgaggaaaccatcactccctggaacttcgaggaagtcgtggacaagggtgcctctgcacagtccttcatcgagcgaatgaccaacttcgacaagaatctgcccaacgagaaggttcttcccaagcattcgctgctctacgagtactttacagtctacaacgaactcaccaaagtcaagtacgttaccgagggaatgcgaaagcctgccttcttgtctggcgaacagaagaaagccattgtcgatctcctgttcaagaccaaccgaaaggtcactgttaagcagctcaaggaggactacttcaagaaaatcgagtgtttcgacagcgtcgagatttccggagttgaggaccgattcaacgcctctttgggcacctatcacgatctgctcaagattatcaaggacaaggattttctcgacaacgaggaaaacgaggacattctggaggacatcgtgctcactcttaccctgttcgaagatcgggagatgatcgaggaacgactcaagacatacgctcacctgttcgacgacaaggtcatgaaacaactcaagcgacgtagatacaccggctggggaagactttcgcgaaagctcatcaacggcatcagagacaagcagtccggaaagaccattctggactttctcaagtccgatggctttgccaaccgaaacttcatgcagctcattcacgacgattctcttaccttcaaggaggacatccagaaggcacaagtgtccggtcagggcgacagcttgcacgaacatattgccaacctggctggttcgccagccatcaagaaaggcattctccagactgtcaaggttgtcgacgagctggtgaaggtcatgggacgtcacaagcccgagaacattgtgatcgagatggccagagagaaccagacaactcaaaagggtcagaaaaactcgcgagagcggatgaagcgaatcgaggaaggcatcaaggagctgggatcccagattctcaaggagcatcccgtcgagaacactcaactgcagaacgagaagctgtatctctactatctgcagaatggtcgagacatgtacgtggatcaggaactggacatcaatcgtctcagcgactacgatgtggaccacattgtccctcaatcctttctcaaggacgattctatcgacaacaaggtccttacacgatccgacaagaacagaggcaagtcggacaacgttcccagcgaagaggtggtcaaaaagatgaagaactactggcgacagctgctcaacgccaagctcattacccagcgaaagttcgacaatcttaccaaggccgagcgaggcggtctgtccgagctcgacaaggctggcttcatcaagcgtcaactcgtcgagaccagacagatcacaaagcacgtcgcacagattctcgattctcggatgaacaccaagtacgacgagaacgacaagctcatccgagaggtcaaggtgattactctcaagtccaaactggtctccgatttccgaaaggactttcagttctacaaggtgcgagagatcaacaattaccaccatgcccacgatgcttacctcaacgccgtcgttggcactgcgctcatcaagaaataccccaagctcgaaagcgagttcgtttacggcgattacaaggtctacgacgttcgaaagatgattgccaagtccgaacaggagattggcaaggctactgccaagtacttcttttactccaacatcatgaactttttcaagaccgagatcaccttggccaacggagagattcgaaagagaccacttatcgagaccaacggcgaaactggagagatcgtgtgggacaagggtcgagactttgcaaccgtgcgaaaggttctgtcgatgcctcaggtcaacatcgtcaagaaaaccgaggttcagactggcggattctccaaggagtcgattctgcccaagcgaaactccgacaagctcatcgctcgaaagaaagactgggatcccaagaaatacggtggcttcgattctcctaccgtcgcctattccgtgcttgtcgttgcgaaggtcgagaagggcaagtccaaaaagctcaagtccgtcaaggagctgctcggaattaccatcatggagcgatcgagcttcgagaagaatcccatcgacttcttggaagccaagggttacaaggaggtcaagaaagacctcattatcaagctgcccaagtactctctgttcgaactggagaacggtcgaaagcgtatgctcgcctccgctggcgagctgcagaagggaaacgagcttgccttgccttcgaagtacgtcaactttctctatctggcttctcactacgagaagctcaagggttctcccgaggacaacgaacagaagcaactcttcgttgagcagcacaaacattacctcgacgagattatcgagcagatttccgagttttcgaagcgagtcatcctggctgatgccaacttggacaaggtgctctctgcctacaacaagcatcgggacaaacccattcgagaacaggcggagaacatcattcacctgtttactcttaccaacctgggtgctcctgcagctttcaagtacttcgataccactatcgaccgaaagcggtacacatccaccaaggaggttctcgatgccaccctgattcaccagtccatcactggcctgtacgagacccgaatcgacctgtctcagcttggtggcgactccagagccgatcccaagaaaaagcgaaaggtctaagcggccgcaagtgtggatggggaagtgagtgcccggttctgtgtgcacaattggcaatccaagatggatggattcaacacagggatatagcgagctacgtggtggtgcgaggatatagcaacggatatttatgtttgacacttgagaatgtacgatacaagcactgtccaagtacaatactaaacatactgtacatactcatactcgtacccgggcaacggtttcacttgagtgcagtggctagtgctcttactcgtacagtgtgcaatactgcgtatcatagtctttgatgtatatcgtattcattcatgttagttgcgtacgagccggaagcataaagtgtaaagcctggggtgcctaatgagtgagctaactcacattaattgcgttgcgctcactgcccgctttccagtcgggaaacctgtcgtgccagctgcattaatgaatcggccaacgcgcggggagaggcggtttgcgtattgggcgctcttccgcttcctcgctcactgactcgctgcgctcggtcgttcggctgcggcgagcggtatcagctcactcaaaggcggtaatacggttatccacagaatcaggggataacgcaggaaagaacatgtgagcaaaaggccagcaaaaggccaggaaccgtaaaaaggccgcgttgctggcgtttttccataggctccgcccccctgacgagcatcacaaaaatcgacgctcaagtcagaggtggcgaaacccgacaggactataaagataccaggcgtttccccctggaagctccctcgtgcgctctcctgttccgaccctgccgcttaccggatacctgtccgcctttctcccttcgggaagcgtggcgctttctcatagctcacgctgtaggtatctcagttcggtgtaggtcgttcgctccaagctgggctgtgtgcacgaaccccccgttcagcccgaccgctgcgccttatccggtaactatcgtcttgagtccaacccggtaagacacgacttatcgccactggcagcagccactggtaacaggattagcagagcgaggtatgtaggcggtgctacagagttcttgaagtggtggcctaactacggctacactagaaggacagtatttggtatctgcgctctgctgaagccagttaccttcggaaaaagagttggtagctcttgatccggcaaacaaaccaccgctggtagcggtggtttttttgtttgcaagcagcagattacgcgcagaaaaaaaggatctcaagaagatcctttgatcttttctacggggtctgacgctcagtggaacgaaaactcacgttaagggattttggtcatgagattatcaaaaaggatcttcacctagatccttttaaattaaaaatgaagttttaaatcaatctaaagtatatatgagtaaacttggtctgacagttaccaatgcttaatcagtgaggcacctatctcagcgatctgtctatttcgttcatccatagttgcctgactccccgtcgtgtagataactacgatacgggagggcttaccatctggccccagtgctgcaatgataccgcgagacccacgctcaccggctccagatttatcagcaataaaccagccagccggaagggccgagcgcagaagtggtcctgcaactttatccgcctccatccagtctattaattgttgccgggaagctagagtaagtagttcgccagttaatagtttgcgcaacgttgttgccattgctacaggcatcgtggtgtcacgctcgtcgtttggtatggcttcattcagctccggttcccaacgatcaaggcgagttacatgatcccccatgttgtgcaaaaaagcggttagctccttcggtcctccgatcgttgtcagaagtaagttggccgcagtgttatcactcatggttatggcagcactgcataattctcttactgtcatgccatccgtaagatgcttttctgtgactggtgagtactcaaccaagtcattctgagaatagtgtatgcggcgaccgagttgctcttgcccggcgtcaatacgggataataccgcgccacatagcagaactttaaaagtgctcatcattggaaaacgttcttcggggcgaaaactctcaaggatcttaccgctgttgagatccagttcgatgtaacccactcgtgcacccaactgatcttcagcatcttttactttcaccagcgtttctgggtgagcaaaaacaggaaggcaaaatgccgcaaaaaagggaataagggcgacacggaaatgttgaatactcatactcttcctttttcaatattattgaagcatttatcagggttattgtctcatgagcggatacatatttgaatgtatttagaaaaataaacaaataggggttccgcgcacatttccccgaaaagtgccacctgacgcgccctgtagcggcgcattaagcgcggcgggtgtggtggttacgcgcagcgtgaccgctacacttgccagcgccctagcgcccgctcctttcgctttcttcccttcctttctcgccacgttcgccggctttccccgtcaagctctaaatcgggggctccctttagggttccgatttagtgctttacggcacctcgaccccaaaaaacttgattagggtgatggttcacgtagtgggccatcgccctgatagacggtttttcgccctttgacgttggagtccacgttctttaatagtggactcttgttccaaactggaacaacactcaaccctatctcggtctattcttttgatttataagggattttgccgatttcggcctattggttaaaaaatgagctgatttaacaaaaatttaacgcgaattttaacaaaatattaacgcttacaatttccattcgccattcaggctgcgcaactgttgggaagggcgatcggtgcgggcctcttcgctattacgccagctggcgaaagggggatgtgctgcaaggcgattaagttgggtaacgccagggttttcccagtcacgacgttgtaaaacgacggccagtgaattgtaatacgactcactatagggcgaattgggtaccgggccccccctcgaggtcgatggtgtcgataagcttgatatcgaattcatgtcacacaaaccgatcttcgcctcaaggaaacctaattctacatccgagagactgccgagatccagtctacactgattaattttcgggccaataatttaaaaaaatcgtgttatataatattatatgtattatatatatacatcatgatgatactgacagtcatgtcccattgctaaatagacagactccatctgccgcctccaactgatgttctcaatatttaaggggtcatctcgcattgtttaataataaacagactccatctaccgcctccaaatgatgttctcaaaatatattgtatgaacttatttttattacttagtattattagacaacttacttgctttatgaaaaacacttcctatttaggaaacaatttataatggcagttcgttcatttaacaatttatgtagaataaatgttataaatgcgtatgggaaatcttaaatatggatagcataaatgatatctgcattgcctaattcgaaatcaacagcaacgaaaaaaatcccttgtacaacataaatagtcatcgagaaatatcaactatcaaagaacagctattcacacgttactattgagattattattggacgagaatcacacactcaactgtctttctctcttctagaaatacaggtacaagtatgtactattctcattgttcatacttctagtcatttcatcccacatattccttggatttctctccaatgaatgacattctatcttgcaaattcaacaattataataagatataccaaagtagcggtatagtggcaatcaaaaagcttctctggtgtgcttctcgtatttatttttattctaatgatccattaaaggtatatatttatttcttgttatataatccttttgtttattacatgggctggatacataaaggtattttgatttaattttttgcttaaattcaatcccccctcgttcagtgtcaactgtaatggtaggaaattaccatacttttgaagaagcaaaaaaaatgaaagaaaaaaaaaatcgtatttccaggttagacgttccgcagaatctagaatgcggtatgcggtacattgttcttcgaacgtaaaagttgcgctccctgagatattgtacatttttgcttttacaagtacaagtacatcgtacaactatgtactactgttgatgcatccacaacagtttgttttgtttttttttgttttttttttttctaatgattcattaccgctatgtatacctacttgtacttgtagtaagccgggttattggcgttcaattaatcatagacttatgaatctgcacggtgtgcgctgcgagttacttttagcttatgcatgctacttgggtgtaatattgggatctgttcggaaatcaacggatgctcaat

SEQ ID NO: 37 - DNA, 40 bp, Artificial sequence
  Can1-1 FBA1tss forward
gctctcccaatcggttgccatcaaacgattacccaccctc

SEQ ID NO: 38 - DNA, 40 bp, Artificial sequence
  Can1-1 FBA1tss forward
agcaatcaccacacgcggccaaaagcaccaccgactcggt

SEQ ID NO: 39 - DNA, 210 bp, Artificial sequence
  Can1-1-HDV for FBA1tss
gctctcccaatcggttgccatcaaacgattacccaccctcgttttagagctagaaatagcaagttaaaataaggctagtccgttatcaacttgaaaaagtggcaccgagtcggtggtgcttttggccggcatggtcccagcctcctcgctggcgccggctgggcaacatgcttcggcatggcgaatgggaggccgcgtgtggtgattgct

SEQ ID NO: 40 - DNA, 40 bp, Artificial Sequence
  Can1-1-HDV Act 1 reverse
agcaatcaccacacgcggcctcccattcgccatgccgaag

SEQ ID NO: 41 - DNA, 143 bp, Artificial sequence
  Can1-1 for FBA1utr
tctaaactacacatcacacctcaaacgattacccaccctcgttttagagctagaaatagcaagttaaaataaggctagtccgttatcaacttgaaaaagtggcaccgagtcggtggtgcttttggccgcgtgtggtgattgct

SEQ ID NO: 42 - DNA, 40 bp, Artificial sequence
  Can1-1 FBA1utr forward
tctaaactacacatcacacctcaaacgattacccaccctc

SEQ ID NO: 43 - DNA, 210 bp, Artificial sequence
  Can1-1-HDV for FBA1utr
tctaaactacacatcacacctcaaacgattacccaccctcgttttagagctagaaatagcaagttaaaataaggctagtccgttatcaacttgaaaaagtggcaccgagtcggtggtgcttttggccggcatggtcccagcctcctcgctggcgccggctgggcaacatgcttcggcatggcgaatgggaggccgcgtgtggtgattgct

SEQ ID NO: 44 - DNA, 143 bp, Artificial sequence
  Can1-1 for TEF1tss;
tttctctctctccttgtcaatcaaacgattacccaccctcgttttagagctagaaatagcaagttaaaataaggctagtccgttatcaacttgaaaaagtggcaccgagtcggtggtgcttttggccgcgtgtggtgattgct

SEQ ID NO: 45 - DNA, 40 bp, Artificial sequence
  Can1-1 for TEF1tss forward
tttctctctctccttgtcaatcaaacgattacccaccctc

SEQ ID NO: 46 - DNA, 210 bp, Artificial sequence
  Can1-1-HDV for TEF1tss
tttctctctctccttgtcaatcaaacgattacccaccctcgttttagagctagaaatagcaagttaaaataaggctagtccgttatcaacttgaaaaagtggcaccgagtcggtggtgcttttggccggcatggtcccagcctcctcgctggcgccggctgggcaacatgcttcggcatggcgaatgggaggccgcgtgtggtgattgct

SEQ ID NO: 47 - DNA, 143 bp, Artificial sequence
  Can1-1 for TEF1utr
gagtataagaatcattcaaatcaaacgattacccaccctcgttttagagctagaaatagcaagttaaaataaggctagtccgttatcaacttgaaaaagtggcaccgagtcggtggtgcttttggccgcgtgtggtgattgct

SEQ ID NO: 48 - DNA, 40 bp, Artificial sequence; identical to SEQ ID NO: 23
  Can1-1 TEF1utr forward

SEQ ID NO: 49 - DNA, 210 bp, Artificial sequence
  Can1-1-HDV for Tef1utr
gagtataagaatcattcaaatcaaacgattacccaccctcgttttagagctagaaatagcaagttaaaataaggctagtccgttatcaacttgaaaaagtggcaccgagtcggtggtgcttttggccggcatggtcccagcctcctcgctggcgccggctgggcaacatgcttcggcatggcgaatgggaggccgcgtgtggtgattgct

SEQ ID NO: 50 - DNA, 1380 bp, Artificial sequence
  FBA1TSS-Can1-1-ACT1 cassette
gggttaattaagtttaaaccatcatctaagggcctcaaaactacctcggaactgctgcgctgatctggacaccacagaggttccgagcactttaggttgcaccaaatgtcccaccaggtgcaggcagaaaacgctggaacagcgtgtacagtttgtcttaacaaaaagtgagggcgctgaggtcgagcagggtggtgtgacttgttatagcctttagagctgcgaaagcgcgtatggatttggctcatcaggccagattgagggtctgtggacacatgtcatgttagtgtacttcaatcgccccctggatatagccccgacaataggccgtggcctcatttttttgccttccgcacatttccattgctcggtacccacaccttgcttctcctgcacttgccaaccttaatactggtttacattgaccaacatcttacaagcggggggcttgtctagggtatatataaacagtggctctcccaatcggttgccatcaaacgattacccaccctcgttttagagctagaaatagcaagttaaaataaggctagtccgttatcaacttgaaaaagtggcaccgagtcggtggtgcttttggccgcgtgtggtgattgctgttgtgcaagcctttgctcgttttctgctgtatgtaatttaaagaacgattgtatgaatcgaagtcaaggtgagtgtagtttgagaagtgtaaccccagtgtcatagctgtgtactccattcattgaagggtgtagtcgtgttttattgcatgagctcctattactcgtataagtaactgttttgtaacacttcatgaacggagatggtatgaacagaagtaataatatcctggaagtcagctgtgcccagaggtgtgtgtgggtgtggcatactttgggacaacaacacttgggcagtatgcttagtgaccacgaagagagtgttaccttctgaggtgcgacgtgcagtagttctattgtttttaaatgcgcagtcgtctttcagaggctgattcaagcagacgcattcagttgtgttcagttgaggctgatatctcagcacctacagtttagggaaagcagggttaagatgatgacaactctgggtggtaacctgggatatgcggcgatatagcaggtaatgacttaataactgctcaatgatgagtatatacatccctcctatctatatatccatatttagtatttacatattcatcttcaccgagctacaagtagaaggatgtacatgctgtatcttgcggtgcctgtcgccatgttttcgacaagttaagttcggagtatgcatgcaaacaaaaatacaagtagtcaaaatattggagtatcaaacaacgtgcttcgaaatctcttccaatcgatcccc

SEQ ID NO: 51 - DNA, 1447 bp, Artificial sequence
  FBA1TSS-Can1-1HDV-ACT1 cassette
gggttaattaagtttaaaccatcatctaagggcctcaaaactacctcggaactgctgcgctgatctggacaccacagaggttccgagcactttaggttgcaccaaatgtcccaccaggtgcaggcagaaaacgctggaacagcgtgtacagtttgtcttaacaaaaagtgagggcgctgaggtcgagcagggtggtgtgacttgttatagcctttagagctgcgaaagcgcgtatggatttggctcatcaggccagattgagggtctgtggacacatgtcatgttagtgtacttcaatcgccccctggatatagccccgacaataggccgtggcctcatttttttgccttccgcacatttccattgctcggtacccacaccttgcttctcctgcacttgccaaccttaatactggtttacattgaccaacatcttacaagcggggggcttgtctagggtatatataaacagtggctctcccaatcggttgccatcaaacgattacccaccctcgttttagagctagaaatagcaagttaaaataaggctagtccgttatcaacttgaaaaagtggcaccgagtcggtggtgcttttggccggcatggtcccagcctcctcgctggcgccggctgggcaacatgcttcggcatggcgaatgggaggccgcgtgtggtgattgctgttgtgcaagcctttgctcgttttctgctgtatgtaatttaaagaacgattgtatgaatcgaagtcaaggtgagtgtagtttgagaagtgtaaccccagtgtcatagctgtgtactccattcattgaagggtgtagtcgtgttttattgcatgagctcctattactcgtataagtaactgttttgtaacacttcatgaacggagatggtatgaacagaagtaataatatcctggaagtcagctgtgcccagaggtgtgtgtgggtgtggcatactttgggacaacaacacttgggcagtatgcttagtgaccacgaagagagtgttaccttctgaggtgcgacgtgcagtagttctattgtttttaaatgcgcagtcgtctttcagaggctgattcaagcagacgcattcagttgtgttcagttgaggctgatatctcagcacctacagtttagggaaagcagggttaagatgatgacaactctgggtggtaacctgggatatgcggcgatatagcaggtaatgacttaataactgctcaatgatgagtatatacatccctcctatctatatatccatatttagtatttacatattcatcttcaccgagctacaagtagaaggatgtacatgctgtatcttgcggtgcctgtcgccatgttttcgacaagttaagttcggagtatgcatgcaaacaaaaatacaagtagtcaaaatattggagtatcaaacaacgtgcttcgaaatctcttccaatcgatcccc

SEQ ID NO: 52 - DNA, 1436 bp, Artificial sequence
  FBA1UTR-Can1-1-ACT1 cassette
gggttaattaagtttaaaccatcatctaagggcctcaaaactacctcggaactgctgcgctgatctggacaccacagaggttccgagcactttaggttgcaccaaatgtcccaccaggtgcaggcagaaaacgctggaacagcgtgtacagtttgtcttaacaaaaagtgagggcgctgaggtcgagcagggtggtgtgacttgttatagcctttagagctgcgaaagcgcgtatggatttggctcatcaggccagattgagggtctgtggacacatgtcatgttagtgtacttcaatcgccccctggatatagccccgacaataggccgtggcctcatttttttgccttccgcacatttccattgctcggtacccacaccttgcttctcctgcacttgccaaccttaatactggtttacattgaccaacatcttacaagcggggggcttgtctagggtatatataaacagtggctctcccaatcggttgccagtctcttttttcctttctttccccacagattcgaaatctaaactacacatcacacctcaaacgattacccaccctcgttttagagctagaaatagcaagttaaaataaggctagtccgttatcaacttgaaaaagtggcaccgagtcggtggtgcttttggccgcgtgtggtgattgctgttgtgcaagcctttgctcgttttctgctgtatgtaatttaaagaacgattgtatgaatcgaagtcaaggtgagtgtagtttgagaagtgtaaccccagtgtcatagctgtgtactccattcattgaagggtgtagtcgtgttttattgcatgagctcctattactcgtataagtaactgttttgtaacacttcatgaacggagatggtatgaacagaagtaataatatcctggaagtcagctgtgcccagaggtgtgtgtgggtgtggcatactttgggacaacaacacttgggcagtatgcttagtgaccacgaagagagtgttaccttctgaggtgcgacgtgcagtagttctattgtttttaaatgcgcagtcgtctttcagaggctgattcaagcagacgcattcagttgtgttcagttgaggctgatatctcagcacctacagtttagggaaagcagggttaagatgatgacaactctgggtggtaacctgggatatgcggcgatatagcaggtaatgacttaataactgctcaatgatgagtatatacatccctcctatctatatatccatatttagtatttacatattcatcttcaccgagctacaagtagaaggatgtacatgctgtatcttgcggtgcctgtcgccatgttttcgacaagttaagttcggagtatgcatgcaaacaaaaatacaagtagtcaaaatattggagtatcaaacaacgtgcttcgaaatctcttccaatcgatcccc

SEQ ID NO: 53 - DNA, 1503 bp, Artificial sequence
  FBA1UTR-Can1-1HDV-ACT1 cassette
gggttaattaagtttaaaccatcatctaagggcctcaaaactacctcggaactgctgcgctgatctggacaccacagaggttccgagcactttaggttgcaccaaatgtcccaccaggtgcaggcagaaaacgctggaacagcgtgtacagtttgtcttaacaaaaagtgagggcgctgaggtcgagcagggtggtgtgacttgttatagcctttagagctgcgaaagcgcgtatggatttggctcatcaggccagattgagggtctgtggacacatgtcatgttagtgtacttcaatcgccccctggatatagccccgacaataggccgtggcctcatttttttgccttccgcacatttccattgctcggtacccacaccttgcttctcctgcacttgccaaccttaatactggtttacattgaccaacatcttacaagcggggggcttgtctagggtatatataaacagtggctctcccaatcggttgccagtctcttttttcctttctttccccacagattcgaaatctaaactacacatcacacctcaaacgattacccaccctcgttttagagctagaaatagcaagttaaaataaggctagtccgttatcaacttgaaaaagtggcaccgagtcggtggtgcttttggccggcatggtcccagcctcctcgctggcgccggctgggcaacatgcttcggcatggcgaatgggaggccgcgtgtggtgattgctgttgtgcaagcctttgctcgttttctgctgtatgtaatttaaagaacgattgtatgaatcgaagtcaaggtgagtgtagtttgagaagtgtaaccccagtgtcatagctgtgtactccattcattgaagggtgtagtcgtgttttattgcatgagctcctattactcgtataagtaactgttttgtaacacttcatgaacggagatggtatgaacagaagtaataatatcctggaagtcagctgtgcccagaggtgtgtgtgggtgtggcatactttgggacaacaacacttgggcagtatgcttagtgaccacgaagagagtgttaccttctgaggtgcgacgtgcagtagttctattgtttttaaatgcgcagtcgtctttcagaggctgattcaagcagacgcattcagttgtgttcagttgaggctgatatctcagcacctacagtttagggaaagcagggttaagatgatgacaactctgggtggtaacctgggatatgcggcgatatagcaggtaatgacttaataactgctcaatgatgagtatatacatccctcctatctatatatccatatttagtatttacatattcatcttcaccgagctacaagtagaaggatgtacatgctgtatcttgcggtgcctgtcgccatgttttcgacaagttaagttcggagtatgcatgcaaacaaaaatacaagtagtcaaaatattggagtatcaaacaacgtgcttcgaaatctcttccaatcgatcccc

SEQ ID NO: 54 - DNA, 1252 bp, Artificial sequence
  TEF1TSS-Can1-1-ACT1 cassette
gggttaattaaagagaccgggttggcggcgcatttgtgtcccaaaaaacagccccaattgccccaattgaccccaaattgacccagtagcgggcccaaccccggcgagagcccccttctccccacatatcaaacctcccccggttcccacacttgccgttaagggcgtagggtactgcagtctggaatctacgcttgttcagactttgtactagtttctttgtctggccatccgggtaacccatgccggacgcaaaatagactactgaaaatttttttgctttgtggttgggactttagccaagggtataaaagaccaccgtccccgaattacctttcctcttcttttctctctctccttgtcaatcaaacgattacccaccctcgttttagagctagaaatagcaagttaaaataaggctagtccgttatcaacttgaaaaagtggcaccgagtcggtggtgcttttggccgcgtgtggtgattgctgttgtgcaagcctttgctcgttttctgctgtatgtaatttaaagaacgattgtatgaatcgaagtcaaggtgagtgtagtttgagaagtgtaaccccagtgtcatagctgtgtactccattcattgaagggtgtagtcgtgttttattgcatgagctcctattactcgtataagtaactgttttgtaacacttcatgaacggagatggtatgaacagaagtaataatatcctggaagtcagctgtgcccagaggtgtgtgtgggtgtggcatactttgggacaacaacacttgggcagtatgcttagtgaccacgaagagagtgttaccttctgaggtgcgacgtgcagtagttctattgtttttaaatgcgcagtcgtctttcagaggctgattcaagcagacgcattcagttgtgttcagttgaggctgatatctcagcacctacagtttagggaaagcagggttaagatgatgacaactctgggtggtaacctgggatatgcggcgatatagcaggtaatgacttaataactgctcaatgatgagtatatacatccctcctatctatatatccatatttagtatttacatattcatcttcaccgagctacaagtagaaggatgtacatgctgtatcttgcggtgcctgtcgccatgttttcgacaagttaagttcggagtatgcatgcaaacaaaaatacaagtagtcaaaatattggagtatcaaacaacgtgcttcgaaatctcttccaatcgatcccc

SEQ ID NO: 55 - DNA, 1319 bp, Artificial sequence
  TEF1TSS-Can1-1-ACT1 cassette
gggttaattaaagagaccgggttggcggcgcatttgtgtcccaaaaaacagccccaattgccccaattgaccccaaattgacccagtagcgggcccaaccccggcgagagcccccttctccccacatatcaaacctcccccggttcccacacttgccgttaagggcgtagggtactgcagtctggaatctacgcttgttcagactttgtactagtttctttgtctggccatccgggtaacccatgccggacgcaaaatagactactgaaaatttttttgctttgtggttgggactttagccaagggtataaaagaccaccgtccccgaattacctttcctcttcttttctctctctccttgtcaatcaaacgattacccaccctcgttttagagctagaaatagcaagttaaaataaggctagtccgttatcaacttgaaaaagtggcaccgagtcggtggtgcttttggccggcatggtcccagcctcctcgctggcgccggctgggcaacatgcttcggcatggcgaatgggaggccgcgtgtggtgattgctgttgtgcaagcctttgctcgttttctgctgtatgtaatttaaagaacgattgtatgaatcgaagtcaaggtgagtgtagtttgagaagtgtaaccccagtgtcatagctgtgtactccattcattgaagggtgtagtcgtgttttattgcatgagctcctattactcgtataagtaactgttttgtaacacttcatgaacggagatggtatgaacagaagtaataatatcctggaagtcagctgtgcccagaggtgtgtgtgggtgtggcatactttgggacaacaacacttgggcagtatgcttagtgaccacgaagagagtgttaccttctgaggtgcgacgtgcagtagttctattgtttttaaatgcgcagtcgtctttcagaggctgattcaagcagacgcattcagttgtgttcagttgaggctgatatctcagcacctacagtttagggaaagcagggttaagatgatgacaactctgggtggtaacctgggatatgcggcgatatagcaggtaatgacttaataactgctcaatgatgagtatatacatccctcctatctatatatccatatttagtatttacatattcatcttcaccgagctacaagtagaaggatgtacatgctgtatcttgcggtgcctgtcgccatgttttcgacaagttaagttcggagtatgcatgcaaacaaaaatacaagtagtcaaaatattggagtatcaaacaacgtgcttcgaaatctcttccaatcgatcccc

SEQ ID NO: 56 - DNA, 1304 bp, Artificial sequence
  TEF1UTR-Can1-1-ACT1 Cassette
gggttaattaaagagaccgggttggcggcgcatttgtgtcccaaaaaacagccccaattgccccaattgaccccaaattgacccagtagcgggcccaaccccggcgagagcccccttctccccacatatcaaacctcccccggttcccacacttgccgttaagggcgtagggtactgcagtctggaatctacgcttgttcagactttgtactagtttctttgtctggccatccgggtaacccatgccggacgcaaaatagactactgaaaatttttttgctttgtggttgggactttagccaagggtataaaagaccaccgtccccgaattacctttcctcttcttttctctctctccttgtcaactcacacccgaaatcgttaagcatttccttctgagtataagaatcattcaaatcaaacgattacccaccctcgttttagagctagaaatagcaagttaaaataaggctagtccgttatcaacttgaaaaagtggcaccgagtcggtggtgcttttggccgcgtgtggtgattgctgttgtgcaagcctttgctcgttttctgctgtatgtaatttaaagaacgattgtatgaatcgaagtcaaggtgagtgtagtttgagaagtgtaaccccagtgtcatagctgtgtactccattcattgaagggtgtagtcgtgttttattgcatgagctcctattactcgtataagtaactgttttgtaacacttcatgaacggagatggtatgaacagaagtaataatatcctggaagtcagctgtgcccagaggtgtgtgtgggtgtggcatactttgggacaacaacacttgggcagtatgcttagtgaccacgaagagagtgttaccttctgaggtgcgacgtgcagtagttctattgtttttaaatgcgcagtcgtctttcagaggctgattcaagcagacgcattcagttgtgttcagttgaggctgatatctcagcacctacagtttagggaaagcagggttaagatgatgacaactctgggtggtaacctgggatatgcggcgatatagcaggtaatgacttaataactgctcaatgatgagtatatacatccctcctatctatatatccatatttagtatttacatattcatcttcaccgagctacaagtagaaggatgtacatgctgtatcttgcggtgcctgtcgccatgttttcgacaagttaagttcggagtatgcatgcaaacaaaaatacaagtagtcaaaatattggagtatcaaacaacgtgcttcgaaatctcttccaatcgatcccc

SEQ ID NO: 57 - DNA, 1304 bp, Artificial sequence; identical to SEQ ID NO: 56
  TEF1UTR-Can1-1HDV-ACT1 cassette

SEQ ID NO: 58 - DNA, 25 bp, Artificial sequence
  HY009
gtagtaagccgggttattggcgttc

SEQ ID NO: 59 - DNA, 25 bp, Artificial sequence
  HY010
atgatctgtccaatggggcatgttg

SEQ ID NO: 60 - DNA, 20 bp, artificial sequence
  ON476
cctcagaaggtaacactctc

SEQ ID NO: 61 - DNA, 12054 bp, Artificial sequence
  pRF617
catggacaagaaatactccatcggcctggacattggaaccaactctgtcggctgggctgtcatcaccgacgagtacaaggtgccctccaagaaattcaaggtcctcggaaacaccgatcgacactccatcaagaaaaacctcattggtgccctgttgttcgattctggcgagactgccgaagctaccagactcaagcgaactgctcggcgacgttacacccgacggaagaaccgaatctgctacctgcaggagatcttttccaacgagatggccaaggtggacgattcgttctttcatcgactggaggaatccttcctcgtcgaggaagacaagaaacacgagcgtcatcccatctttggcaacattgtggacgaggttgcttaccacgagaagtatcctaccatctaccacctgcgaaagaaactcgtcgattccaccgacaaggcggatctcagacttatctacctcgctctggcacacatgatcaagtttcgaggtcatttcctcatcgagggcgatctcaatcccgacaacagcgatgtggacaagctgttcattcagctcgttcagacctacaaccagctgttcgaggaaaaccccatcaatgcctccggagtcgatgcaaaggccatcttgtctgctcgactctcgaagagcagacgactggagaacctcattgcccaacttcctggcgagaaaaagaacggactgtttggcaacctcattgccctttctcttggtctcacacccaacttcaagtccaacttcgatctggcggaggacgccaagctccagctgtccaaggacacctacgacgatgacctcgacaacctgcttgcacagattggcgatcagtacgccgacctgtttctcgctgccaagaacctttcggatgctattctcttgtctgacattctgcgagtcaacaccgagatcacaaaggctcccctttctgcctccatgatcaagcgatacgacgagcaccatcaggatctcacactgctcaaggctcttgtccgacagcaactgcccgagaagtacaaggagatctttttcgatcagtcgaagaacggctacgctggatacatcgacggcggagcctctcaggaagagttctacaagttcatcaagccaattctcgagaagatggacggaaccgaggaactgcttgtcaagctcaatcgagaggatctgcttcggaagcaacgaaccttcgacaacggcagcattcctcatcagatccacctcggtgagctgcacgccattcttcgacgtcaggaagacttctacccctttctcaaggacaaccgagagaagatcgagaagattcttacctttcgaatcccctactatgttggtcctcttgccagaggaaactctcgatttgcttggatgactcgaaagtccgaggaaaccatcactccctggaacttcgaggaagtcgtggacaagggtgcctctgcacagtccttcatcgagcgaatgaccaacttcgacaagaatctgcccaacgagaaggttcttcccaagcattcgctgctctacgagtactttacagtctacaacgaactcaccaaagtcaagtacgttaccgagggaatgcgaaagcctgccttcttgtctggcgaacagaagaaagccattgtcgatctcctgttcaagaccaaccgaaaggtcactgttaagcagctcaaggaggactacttcaagaaaatcgagtgtttcgacagcgtcgagatttccggagttgaggaccgattcaacgcctctttgggcacctatcacgatctgctcaagattatcaaggacaaggattttctcgacaacgaggaaaacgaggacattctggaggacatcgtgctcactcttaccctgttcgaagatcgggagatgatcgaggaacgactcaagacatacgctcacctgttcgacgacaaggtcatgaaacaactcaagcgacgtagatacaccggctggggaagactttcgcgaaagctcatcaacggcatcagagacaagcagtccggaaagaccattctggactttctcaagtccgatggctttgccaaccgaaacttcatgcagctcattcacgacgattctcttaccttcaaggaggacatccagaaggcacaagtgtccggtcagggcgacagcttgcacgaacatattgccaacctggctggttcgccagccatcaagaaaggcattctccagactgtcaaggttgtcgacgagctggtgaaggtcatgggacgtcacaagcccgagaacattgtgatcgagatggccagagagaaccagacaactcaaaagggtcagaaaaactcgcgagagcggatgaagcgaatcgaggaaggcatcaaggagctgggatcccagattctcaaggagcatcccgtcgagaacactcaactgcagaacgagaagctgtatctctactatctgcagaatggtcgagacatgtacgtggatcaggaactggacatcaatcgtctcagcgactacgatgtggaccacattgtccctcaatcctttctcaaggacgattctatcgacaacaaggtccttacacgatccgacaagaacagaggcaagtcggacaacgttcccagcgaagaggtggtcaaaaagatgaagaactactggcgacagctgctcaacgccaagctcattacccagcgaaagttcgacaatcttaccaaggccgagcgaggcggtctgtccgagctcgacaaggctggcttcatcaagcgtcaactcgtcgagaccagacagatcacaaagcacgtcgcacagattctcgattctcggatgaacaccaagtacgacgagaacgacaagctcatccgagaggtcaaggtgattactctcaagtccaaactggtctccgatttccgaaaggactttcagttctacaaggtgcgagagatcaacaattaccaccatgcccacgatgcttacctcaacgccgtcgttggcactgcgctcatcaagaaataccccaagctcgaaagcgagttcgtttacggcgattacaaggtctacgacgttcgaaagatgattgccaagtccgaacaggagattggcaaggctactgccaagtacttcttttactccaacatcatgaactttttcaagaccgagatcaccttggccaacggagagattcgaaagagaccacttatcgagaccaacggcgaaactggagagatcgtgtgggacaagggtcgagactttgcaaccgtgcgaaaggttctgtcgatgcctcaggtcaacatcgtcaagaaaaccgaggttcagactggcggattctccaaggagtcgattctgcccaagcgaaactccgacaagctcatcgctcgaaagaaagactgggatcccaagaaatacggtggcttcgattctcctaccgtcgcctattccgtgcttgtcgttgcgaaggtcgagaagggcaagtccaaaaagctcaagtccgtcaaggagctgctcggaattaccatcatggagcgatcgagcttcgagaagaatcccatcgacttcttggaagccaagggttacaaggaggtcaagaaagacctcattatcaagctgcccaagtactctctgttcgaactggagaacggtcgaaagcgtatgctcgcctccgctggcgagctgcagaagggaaacgagcttgccttgccttcgaagtacgtcaactttctctatctggcttctcactacgagaagctcaagggttctcccgaggacaacgaacagaagcaactcttcgttgagcagcacaaacattacctcgacgagattatcgagcagatttccgagttttcgaagcgagtcatcctggctgatgccaacttggacaaggtgctctctgcctacaacaagcatcgggacaaacccattcgagaacaggcggagaacatcattcacctgtttactcttaccaacctgggtgctcctgcagctttcaagtacttcgataccactatcgaccgaaagcggtacacatccaccaaggaggttctcgatgccaccctgattcaccagtccatcactggcctgtacgagacccgaatcgacctgtctcagcttggtggcgactccagagccgatcccaagaaaaagcgaaaggtctaagcggccgcaagtgtggatggggaagtgagtgcccggttctgtgtgcacaattggcaatccaagatggatggattcaacacagggatatagcgagctacgtggtggtgcgaggatatagcaacggatatttatgtttgacacttgagaatgtacgatacaagcactgtccaagtacaatactaaacatactgtacatactcatactcgtacccgggcaacggtttcacttgagtgcagtggctagtgctcttactcgtacagtgtgcaatactgcgtatcatagtctttgatgtatatcgtattcattcatgttagttgcgtacgagccggaagcataaagtgtaaagcctggggtgcctaatgagtgagctaactcacattaattgcgttgcgctcactgcccgctttccagtcgggaaacctgtcgtgccagctgcattaatgaatcggccaacgcgcggggagaggcggtttgcgtattgggcgctcttccgcttcctcgctcactgactcgctgcgctcggtcgttcggctgcggcgagcggtatcagctcactcaaaggcggtaatacggttatccacagaatcaggggataacgcaggaaagaacatgtgagcaaaaggccagcaaaaggccaggaaccgtaaaaaggccgcgttgctggcgtttttccataggctccgcccccctgacgagcatcacaaaaatcgacgctcaagtcagaggtggcgaaacccgacaggactataaagataccaggcgtttccccctggaagctccctcgtgcgctctcctgttccgaccctgccgcttaccggatacctgtccgcctttctcccttcgggaagcgtggcgctttctcatagctcacgctgtaggtatctcagttcggtgtaggtcgttcgctccaagctgggctgtgtgcacgaaccccccgttcagcccgaccgctgcgccttatccggtaactatcgtcttgagtccaacccggtaagacacgacttatcgccactggcagcagccactggtaacaggattagcagagcgaggtatgtaggcggtgctacagagttcttgaagtggtggcctaactacggctacactagaaggacagtatttggtatctgcgctctgctgaagccagttaccttcggaaaaagagttggtagctcttgatccggcaaacaaaccaccgctggtagcggtggtttttttgtttgcaagcagcagattacgcgcagaaaaaaaggatctcaagaagatcctttgatcttttctacggggtctgacgctcagtggaacgaaaactcacgttaagggattttggtcatgagattatcaaaaaggatcttcacctagatccttttaaattaaaaatgaagttttaaatcaatctaaagtatatatgagtaaacttggtctgacagttaccaatgcttaatcagtgaggcacctatctcagcgatctgtctatttcgttcatccatagttgcctgactccccgtcgtgtagataactacgatacgggagggcttaccatctggccccagtgctgcaatgataccgcgagacccacgctcaccggctccagatttatcagcaataaaccagccagccggaagggccgagcgcagaagtggtcctgcaactttatccgcctccatccagtctattaattgttgccgggaagctagagtaagtagttcgccagttaatagtttgcgcaacgttgttgccattgctacaggcatcgtggtgtcacgctcgtcgtttggtatggcttcattcagctccggttcccaacgatcaaggcgagttacatgatcccccatgttgtgcaaaaaagcggttagctccttcggtcctccgatcgttgtcagaagtaagttggccgcagtgttatcactcatggttatggcagcactgcataattctcttactgtcatgccatccgtaagatgcttttctgtgactggtgagtactcaaccaagtcattctgagaatagtgtatgcggcgaccgagttgctcttgcccggcgtcaatacgggataataccgcgccacatagcagaactttaaaagtgctcatcattggaaaacgttcttcggggcgaaaactctcaaggatcttaccgctgttgagatccagttcgatgtaacccactcgtgcacccaactgatcttcagcatcttttactttcaccagcgtttctgggtgagcaaaaacaggaaggcaaaatgccgcaaaaaagggaataagggcgacacggaaatgttgaatactcatactcttcctttttcaatattattgaagcatttatcagggttattgtctcatgagcggatacatatttgaatgtatttagaaaaataaacaaataggggttccgcgcacatttccccgaaaagtgccacctgacgcgccctgtagcggcgcattaagcgcggcgggtgtggtggttacgcgcagcgtgaccgctacacttgccagcgccctagcgcccgctcctttcgctttcttcccttcctttctcgccacgttcgccggctttccccgtcaagctctaaatcgggggctccctttagggttccgatttagtgctttacggcacctcgaccccaaaaaacttgattagggtgatggttcacgtagtgggccatcgccctgatagacggtttttcgccctttgacgttggagtccacgttctttaatagtggactcttgttccaaactggaacaacactcaaccctatctcggtctattcttttgatttataagggattttgccgatttcggcctattggttaaaaaatgagctgatttaacaaaaatttaacgcgaattttaacaaaatattaacgcttacaatttccattcgccattcaggctgcgcaactgttgggaagggcgatcggtgcgggcctcttcgctattacgccagctggcgaaagggggatgtgctgcaaggcgattaagttgggtaacgccagggttttcccagtcacgacgttgtaaaacgacggccagtgaattgtaatacgactcactatagggcgaattgggtaccgggccccccctcgaggtcgatggtgtcgataagcttgatatcgaattcatgtcacacaaaccgatcttcgcctcaaggaaacctaattctacatccgagagactgccgagatccagtctacactgattaattttcgggccaataatttaaaaaaatcgtgttatataatattatatgtattatatatatacatcatgatgatactgacagtcatgtcccattgctaaatagacagactccatctgccgcctccaactgatgttctcaatatttaaggggtcatctcgcattgtttaataataaacagactccatctaccgcctccaaatgatgttctcaaaatatattgtatgaacttatttttattacttagtattattagacaacttacttgctttatgaaaaacacttcctatttaggaaacaatttataatggcagttcgttcatttaacaatttatgtagaataaatgttataaatgcgtatgggaaatcttaaatatggatagcataaatgatatctgcattgcctaattcgaaatcaacagcaacgaaaaaaatcccttgtacaacataaatagtcatcgagaaatatcaactatcaaagaacagctattcacacgttactattgagattattattggacgagaatcacacactcaactgtctttctctcttctagaaatacaggtacaagtatgtactattctcattgttcatacttctagtcatttcatcccacatattccttggatttctctccaatgaatgacattctatcttgcaaattcaacaattataataagatataccaaagtagcggtatagtggcaatcaaaaagcttctctggtgtgcttctcgtatttatttttattctaatgatccattaaaggtatatatttatttcttgttatataatccttttgtttattacatgggctggatacataaaggtattttgatttaattttttgcttaaattcaatcccccctcgttcagtgtcaactgtaatggtaggaaattaccatacttttgaagaagcaaaaaaaatgaaagaaaaaaaaaatcgtatttccaggttagacgttccgcagaatctagaatgcggtatgcggtacattgttcttcgaacgtaaaagttgcgctccctgagatattgtacatttttgcttttacaagtacaagtacatcgtacaactatgtactactgttgatgcatccacaacagtttgttttgtttttttttgttttttttttttctaatgattcattaccgctatgtatacctacttgtacttgtagtaagccgggttattggcgttcaattaatcatagacttatgaatctgcacggtgtgcgctgcgagttacttttagcttatgcatgctacttgggtgtaatattgggatctgttcggaaatcaacggatgctcaatcgattggaagagatttcgaagcacgttgtttgatactccaatattttgactacttgtatttttgtttgcatgcatactccgaacttaacttgtcgaaaacatggcgacaggcaccgcaagatacagcatgtacatccttctacttgtagctcggtgaagatgaatatgtaaatactaaatatggatatatagataggagggatgtatatactcatcattgagcagttattaagtcattacctgctatatcgccgcatatcccaggttaccacccagagttgtcatcatcttaaccctgctttccctaaactgtaggtgctgagatatcagcctcaactgaacacaactgaatgcgtctgcttgaatcagcctctgaaagacgactgcgcatttaaaaacaatagaactactgcacgtcgcacctcagaaggtaacactctcttcgtggtcactaagcatactgcccaagtgttgttgtcccaaagtatgccacacccacacacacctctgggcacagctgacttccaggatattattacttctgttcataccatctccgttcatgaagtgttacaaaacagttacttatacgagtaataggagctcatgcaataaaacacgactacacccttcaatgaatggagtacacagctatgacactggggttacacttctcaaactacactcaccttgacttcgattcatacaatcgttctttaaattacatacagcagaaaacgagcaaaggcttgcacaacagcaatcaccacacgcggccaaaagcaccaccgactcggtgccactttttcaagttgataacggactagccttattttaacttgctatttctagctctaaaacgagggtgggtaatcgtttgatggcaaccgattgggagagccactgtttatatataccctagacaagccccccgcttgtaagatgttggtcaatgtaaaccagtattaaggttggcaagtgcaggagaagcaaggtgtgggtaccgagcaatggaaatgtgcggaaggcaaaaaaatgaggccacggcctattgtcggggctatatccagggggcgattgaagtacactaacatgacatgtgtccacagaccctcaatctggcctgatgagccaaatccatacgcgctttcgcagctctaaaggctataacaagtcacaccaccctgctcgacctcagcgccctcactttttgttaagacaaactgtacacgctgttccagcgttttctgcctgcacctggtgggacatttggtgcaacctaaagtgctcggaacctctgtggtgtccagatcagcgcagcagttccgaggtagttttgaggcccttagatgatggtttaaacttaattaagtcatacacaagtcagctttcttcgagcctcatataagtataagtagttcaacgtattagcactgtacccagcatctccgtatcgagaaacacaacaacatgccccattggacagatcatgcggatacacaggttgtgcagtatcatacatactcgatcagacaggtcgtctgaccatcatacaagctgaacaagcgctccatacttgcacgctctctatatacacagttaaattacatatccatagtctaacctctaacagttaatcttctggtaagcctcccagccagccttctggtatcgcttggcctcctcaataggatctcggttctggccgtacagacctcggccgacaattatgatatccgttccggtagacatgacatcctcaacagttcggtactgctgtccgagagcgtctcccttgtcgtcaagacccaccccgggggtcagaataagccagtcctcagagtcgcccttaggtcggttctgggcaatgaagccaaccacaaactcggggtcggatcgggcaagctcaatggtctgcttggagtactcgccagtggccagagagcccttgcaagacagctcggccagcatgagcagacctctggccagcttctcgttgggagaggggactaggaactccttgtactgggagttctcgtagtcagagacgtcctccttcttctgttcagagacagtttcctcggcaccagctcgcaggccagcaatgattccggttccgggtacaccgtgggcgttggtgatatcggaccactcggcgattcggtgacaccggtactggtgcttgacagtgttgccaatatctgcgaactttctgtcctcgaacaggaagaaaccgtgcttaagagcaagttccttgagggggagcacagtgccggcgtaggtgaagtcgtcaatgatgtcgatatgggttttgatcatgcacacataaggtccgaccttatcggcaagctcaatgagctccttggtggtggtaacatccagagaagcacacaggttggttttcttggctgccacgagcttgagcactcgagcggcaaaggcggacttgtggacgttagctcgagcttcgtaggagggcattttggtggtgaagaggagactgaaataaatttagtctgcagaactttttatcggaaccttatctggggcagtgaagtatatgttatggtaatagttacgagttagttgaacttatagatagactggactatacggctatcggtccaaattagaaagaacgtcaatggctctctgggcgtcgcctttgccgacaaaaatgtgatcatgatgaaagccagcaatgacgttgcagctgatattgttgtcggccaaccgcgccgaaaacgcagctgtcagacccacagcctccaacgaagaatgtatcgtcaaagtgatccaagcacactcatagttggagtcgtactccaaaggcggcaatgacgagtcagacagatactcgtcgacgtttaaaccatcatctaagggcctcaaaactacctcggaactgctgcgctgatctggacaccacagaggttccgagcactttaggttgcaccaaatgtcccaccaggtgcaggcagaaaacgctggaacagcgtgtacagtttgtcttaacaaaaagtgagggcgctgaggtcgagcagggtggtgtgacttgttatagcctttagagctgcgaaagcgcgtatggatttggctcatcaggccagattgagggtctgtggacacatgtcatgttagtgtacttcaatcgccccctggatatagccccgacaataggccgtggcctcatttttttgccttccgcacatttccattgctcggtacccacaccttgcttctcctgcacttgccaaccttaatactggtttacattgaccaacatcttacaagcggggggcttgtctagggtatatataaacagtggctctcccaatcggttgccagtctcttttttcctttctttccccacagattcgaaatctaaactacacatcacac

SEQ ID NO: 62 - DNA, 12121 bp, Artificial sequence
  pRF616
catggacaagaaatactccatcggcctggacattggaaccaactctgtcggctgggctgtcatcaccgacgagtacaaggtgccctccaagaaattcaaggtcctcggaaacaccgatcgacactccatcaagaaaaacctcattggtgccctgttgttcgattctggcgagactgccgaagctaccagactcaagcgaactgctcggcgacgttacacccgacggaagaaccgaatctgctacctgcaggagatcttttccaacgagatggccaaggtggacgattcgttctttcatcgactggaggaatccttcctcgtcgaggaagacaagaaacacgagcgtcatcccatctttggcaacattgtggacgaggttgcttaccacgagaagtatcctaccatctaccacctgcgaaagaaactcgtcgattccaccgacaaggcggatctcagacttatctacctcgctctggcacacatgatcaagtttcgaggtcatttcctcatcgagggcgatctcaatcccgacaacagcgatgtggacaagctgttcattcagctcgttcagacctacaaccagctgttcgaggaaaaccccatcaatgcctccggagtcgatgcaaaggccatcttgtctgctcgactctcgaagagcagacgactggagaacctcattgcccaacttcctggcgagaaaaagaacggactgtttggcaacctcattgccctttctcttggtctcacacccaacttcaagtccaacttcgatctggcggaggacgccaagctccagctgtccaaggacacctacgacgatgacctcgacaacctgcttgcacagattggcgatcagtacgccgacctgtttctcgctgccaagaacctttcggatgctattctcttgtctgacattctgcgagtcaacaccgagatcacaaaggctcccctttctgcctccatgatcaagcgatacgacgagcaccatcaggatctcacactgctcaaggctcttgtccgacagcaactgcccgagaagtacaaggagatctttttcgatcagtcgaagaacggctacgctggatacatcgacggcggagcctctcaggaagagttctacaagttcatcaagccaattctcgagaagatggacggaaccgaggaactgcttgtcaagctcaatcgagaggatctgcttcggaagcaacgaaccttcgacaacggcagcattcctcatcagatccacctcggtgagctgcacgccattcttcgacgtcaggaagacttctacccctttctcaaggacaaccgagagaagatcgagaagattcttacctttcgaatcccctactatgttggtcctcttgccagaggaaactctcgatttgcttggatgactcgaaagtccgaggaaaccatcactccctggaacttcgaggaagtcgtggacaagggtgcctctgcacagtccttcatcgagcgaatgaccaacttcgacaagaatctgcccaacgagaaggttcttcccaagcattcgctgctctacgagtactttacagtctacaacgaactcaccaaagtcaagtacgttaccgagggaatgcgaaagcctgccttcttgtctggcgaacagaagaaagccattgtcgatctcctgttcaagaccaaccgaaaggtcactgttaagcagctcaaggaggactacttcaagaaaatcgagtgtttcgacagcgtcgagatttccggagttgaggaccgattcaacgcctctttgggcacctatcacgatctgctcaagattatcaaggacaaggattttctcgacaacgaggaaaacgaggacattctggaggacatcgtgctcactcttaccctgttcgaagatcgggagatgatcgaggaacgactcaagacatacgctcacctgttcgacgacaaggtcatgaaacaactcaagcgacgtagatacaccggctggggaagactttcgcgaaagctcatcaacggcatcagagacaagcagtccggaaagaccattctggactttctcaagtccgatggctttgccaaccgaaacttcatgcagctcattcacgacgattctcttaccttcaaggaggacatccagaaggcacaagtgtccggtcagggcgacagcttgcacgaacatattgccaacctggctggttcgccagccatcaagaaaggcattctccagactgtcaaggttgtcgacgagctggtgaaggtcatgggacgtcacaagcccgagaacattgtgatcgagatggccagagagaaccagacaactcaaaagggtcagaaaaactcgcgagagcggatgaagcgaatcgaggaaggcatcaaggagctgggatcccagattctcaaggagcatcccgtcgagaacactcaactgcagaacgagaagctgtatctctactatctgcagaatggtcgagacatgtacgtggatcaggaactggacatcaatcgtctcagcgactacgatgtggaccacattgtccctcaatcctttctcaaggacgattctatcgacaacaaggtccttacacgatccgacaagaacagaggcaagtcggacaacgttcccagcgaagaggtggtcaaaaagatgaagaactactggcgacagctgctcaacgccaagctcattacccagcgaaagttcgacaatcttaccaaggccgagcgaggcggtctgtccgagctcgacaaggctggcttcatcaagcgtcaactcgtcgagaccagacagatcacaaagcacgtcgcacagattctcgattctcggatgaacaccaagtacgacgagaacgacaagctcatccgagaggtcaaggtgattactctcaagtccaaactggtctccgatttccgaaaggactttcagttctacaaggtgcgagagatcaacaattaccaccatgcccacgatgcttacctcaacgccgtcgttggcactgcgctcatcaagaaataccccaagctcgaaagcgagttcgtttacggcgattacaaggtctacgacgttcgaaagatgattgccaagtccgaacaggagattggcaaggctactgccaagtacttcttttactccaacatcatgaactttttcaagaccgagatcaccttggccaacggagagattcgaaagagaccacttatcgagaccaacggcgaaactggagagatcgtgtgggacaagggtcgagactttgcaaccgtgcgaaaggttctgtcgatgcctcaggtcaacatcgtcaagaaaaccgaggttcagactggcggattctccaaggagtcgattctgcccaagcgaaactccgacaagctcatcgctcgaaagaaagactgggatcccaagaaatacggtggcttcgattctcctaccgtcgcctattccgtgcttgtcgttgcgaaggtcgagaagggcaagtccaaaaagctcaagtccgtcaaggagctgctcggaattaccatcatggagcgatcgagcttcgagaagaatcccatcgacttcttggaagccaagggttacaaggaggtcaagaaagacctcattatcaagctgcccaagtactctctgttcgaactggagaacggtcgaaagcgtatgctcgcctccgctggcgagctgcagaagggaaacgagcttgccttgccttcgaagtacgtcaactttctctatctggcttctcactacgagaagctcaagggttctcccgaggacaacgaacagaagcaactcttcgttgagcagcacaaacattacctcgacgagattatcgagcagatttccgagttttcgaagcgagtcatcctggctgatgccaacttggacaaggtgctctctgcctacaacaagcatcgggacaaacccattcgagaacaggcggagaacatcattcacctgtttactcttaccaacctgggtgctcctgcagctttcaagtacttcgataccactatcgaccgaaagcggtacacatccaccaaggaggttctcgatgccaccctgattcaccagtccatcactggcctgtacgagacccgaatcgacctgtctcagcttggtggcgactccagagccgatcccaagaaaaagcgaaaggtctaagcggccgcaagtgtggatggggaagtgagtgcccggttctgtgtgcacaattggcaatccaagatggatggattcaacacagggatatagcgagctacgtggtggtgcgaggatatagcaacggatatttatgtttgacacttgagaatgtacgatacaagcactgtccaagtacaatactaaacatactgtacatactcatactcgtacccgggcaacggtttcacttgagtgcagtggctagtgctcttactcgtacagtgtgcaatactgcgtatcatagtctttgatgtatatcgtattcattcatgttagttgcgtacgagccggaagcataaagtgtaaagcctggggtgcctaatgagtgagctaactcacattaattgcgttgcgctcactgcccgctttccagtcgggaaacctgtcgtgccagctgcattaatgaatcggccaacgcgcggggagaggcggtttgcgtattgggcgctcttccgcttcctcgctcactgactcgctgcgctcggtcgttcggctgcggcgagcggtatcagctcactcaaaggcggtaatacggttatccacagaatcaggggataacgcaggaaagaacatgtgagcaaaaggccagcaaaaggccaggaaccgtaaaaaggccgcgttgctggcgtttttccataggctccgcccccctgacgagcatcacaaaaatcgacgctcaagtcagaggtggcgaaacccgacaggactataaagataccaggcgtttccccctggaagctccctcgtgcgctctcctgttccgaccctgccgcttaccggatacctgtccgcctttctcccttcgggaagcgtggcgctttctcatagctcacgctgtaggtatctcagttcggtgtaggtcgttcgctccaagctgggctgtgtgcacgaaccccccgttcagcccgaccgctgcgccttatccggtaactatcgtcttgagtccaacccggtaagacacgacttatcgccactggcagcagccactggtaacaggattagcagagcgaggtatgtaggcggtgctacagagttcttgaagtggtggcctaactacggctacactagaaggacagtatttggtatctgcgctctgctgaagccagttaccttcggaaaaagagttggtagctcttgatccggcaaacaaaccaccgctggtagcggtggtttttttgtttgcaagcagcagattacgcgcagaaaaaaaggatctcaagaagatcctttgatcttttctacggggtctgacgctcagtggaacgaaaactcacgttaagggattttggtcatgagattatcaaaaaggatcttcacctagatccttttaaattaaaaatgaagttttaaatcaatctaaagtatatatgagtaaacttggtctgacagttaccaatgcttaatcagtgaggcacctatctcagcgatctgtctatttcgttcatccatagttgcctgactccccgtcgtgtagataactacgatacgggagggcttaccatctggccccagtgctgcaatgataccgcgagacccacgctcaccggctccagatttatcagcaataaaccagccagccggaagggccgagcgcagaagtggtcctgcaactttatccgcctccatccagtctattaattgttgccgggaagctagagtaagtagttcgccagttaatagtttgcgcaacgttgttgccattgctacaggcatcgtggtgtcacgctcgtcgtttggtatggcttcattcagctccggttcccaacgatcaaggcgagttacatgatcccccatgttgtgcaaaaaagcggttagctccttcggtcctccgatcgttgtcagaagtaagttggccgcagtgttatcactcatggttatggcagcactgcataattctcttactgtcatgccatccgtaagatgcttttctgtgactggtgagtactcaaccaagtcattctgagaatagtgtatgcggcgaccgagttgctcttgcccggcgtcaatacgggataataccgcgccacatagcagaactttaaaagtgctcatcattggaaaacgttcttcggggcgaaaactctcaaggatcttaccgctgttgagatccagttcgatgtaacccactcgtgcacccaactgatcttcagcatcttttactttcaccagcgtttctgggtgagcaaaaacaggaaggcaaaatgccgcaaaaaagggaataagggcgacacggaaatgttgaatactcatactcttcctttttcaatattattgaagcatttatcagggttattgtctcatgagcggatacatatttgaatgtatttagaaaaataaacaaataggggttccgcgcacatttccccgaaaagtgccacctgacgcgccctgtagcggcgcattaagcgcggcgggtgtggtggttacgcgcagcgtgaccgctacacttgccagcgccctagcgcccgctcctttcgctttcttcccttcctttctcgccacgttcgccggctttccccgtcaagctctaaatcgggggctccctttagggttccgatttagtgctttacggcacctcgaccccaaaaaacttgattagggtgatggttcacgtagtgggccatcgccctgatagacggtttttcgccctttgacgttggagtccacgttctttaatagtggactcttgttccaaactggaacaacactcaaccctatctcggtctattcttttgatttataagggattttgccgatttcggcctattggttaaaaaatgagctgatttaacaaaaatttaacgcgaattttaacaaaatattaacgcttacaatttccattcgccattcaggctgcgcaactgttgggaagggcgatcggtgcgggcctcttcgctattacgccagctggcgaaagggggatgtgctgcaaggcgattaagttgggtaacgccagggttttcccagtcacgacgttgtaaaacgacggccagtgaattgtaatacgactcactatagggcgaattgggtaccgggccccccctcgaggtcgatggtgtcgataagcttgatatcgaattcatgtcacacaaaccgatcttcgcctcaaggaaacctaattctacatccgagagactgccgagatccagtctacactgattaattttcgggccaataatttaaaaaaatcgtgttatataatattatatgtattatatatatacatcatgatgatactgacagtcatgtcccattgctaaatagacagactccatctgccgcctccaactgatgttctcaatatttaaggggtcatctcgcattgtttaataataaacagactccatctaccgcctccaaatgatgttctcaaaatatattgtatgaacttatttttattacttagtattattagacaacttacttgctttatgaaaaacacttcctatttaggaaacaatttataatggcagttcgttcatttaacaatttatgtagaataaatgttataaatgcgtatgggaaatcttaaatatggatagcataaatgatatctgcattgcctaattcgaaatcaacagcaacgaaaaaaatcccttgtacaacataaatagtcatcgagaaatatcaactatcaaagaacagctattcacacgttactattgagattattattggacgagaatcacacactcaactgtctttctctcttctagaaatacaggtacaagtatgtactattctcattgttcatacttctagtcatttcatcccacatattccttggatttctctccaatgaatgacattctatcttgcaaattcaacaattataataagatataccaaagtagcggtatagtggcaatcaaaaagcttctctggtgtgcttctcgtatttatttttattctaatgatccattaaaggtatatatttatttcttgttatataatccttttgtttattacatgggctggatacataaaggtattttgatttaattttttgcttaaattcaatcccccctcgttcagtgtcaactgtaatggtaggaaattaccatacttttgaagaagcaaaaaaaatgaaagaaaaaaaaaatcgtatttccaggttagacgttccgcagaatctagaatgcggtatgcggtacattgttcttcgaacgtaaaagttgcgctccctgagatattgtacatttttgcttttacaagtacaagtacatcgtacaactatgtactactgttgatgcatccacaacagtttgttttgtttttttttgttttttttttttctaatgattcattaccgctatgtatacctacttgtacttgtagtaagccgggttattggcgttcaattaatcatagacttatgaatctgcacggtgtgcgctgcgagttacttttagcttatgcatgctacttgggtgtaatattgggatctgttcggaaatcaacggatgctcaatcgattggaagagatttcgaagcacgttgtttgatactccaatattttgactacttgtatttttgtttgcatgcatactccgaacttaacttgtcgaaaacatggcgacaggcaccgcaagatacagcatgtacatccttctacttgtagctcggtgaagatgaatatgtaaatactaaatatggatatatagataggagggatgtatatactcatcattgagcagttattaagtcattacctgctatatcgccgcatatcccaggttaccacccagagttgtcatcatcttaaccctgctttccctaaactgtaggtgctgagatatcagcctcaactgaacacaactgaatgcgtctgcttgaatcagcctctgaaagacgactgcgcatttaaaaacaatagaactactgcacgtcgcacctcagaaggtaacactctcttcgtggtcactaagcatactgcccaagtgttgttgtcccaaagtatgccacacccacacacacctctgggcacagctgacttccaggatattattacttctgttcataccatctccgttcatgaagtgttacaaaacagttacttatacgagtaataggagctcatgcaataaaacacgactacacccttcaatgaatggagtacacagctatgacactggggttacacttctcaaactacactcaccttgacttcgattcatacaatcgttctttaaattacatacagcagaaaacgagcaaaggcttgcacaacagcaatcaccacacgcggcctcccattcgccatgccgaagcatgttgcccagccggcgccagcgaggaggctgggaccatgccggccaaaagcaccaccgactcggtgccactttttcaagttgataacggactagccttattttaacttgctatttctagctctaaaacgagggtgggtaatcgtttgatggcaaccgattgggagagccactgtttatatataccctagacaagccccccgcttgtaagatgttggtcaatgtaaaccagtattaaggttggcaagtgcaggagaagcaaggtgtgggtaccgagcaatggaaatgtgcggaaggcaaaaaaatgaggccacggcctattgtcggggctatatccagggggcgattgaagtacactaacatgacatgtgtccacagaccctcaatctggcctgatgagccaaatccatacgcgctttcgcagctctaaaggctataacaagtcacaccaccctgctcgacctcagcgccctcactttttgttaagacaaactgtacacgctgttccagcgttttctgcctgcacctggtgggacatttggtgcaacctaaagtgctcggaacctctgtggtgtccagatcagcgcagcagttccgaggtagttttgaggcccttagatgatggtttaaacttaattaagtcatacacaagtcagctttcttcgagcctcatataagtataagtagttcaacgtattagcactgtacccagcatctccgtatcgagaaacacaacaacatgccccattggacagatcatgcggatacacaggttgtgcagtatcatacatactcgatcagacaggtcgtctgaccatcatacaagctgaacaagcgctccatacttgcacgctctctatatacacagttaaattacatatccatagtctaacctctaacagttaatcttctggtaagcctcccagccagccttctggtatcgcttggcctcctcaataggatctcggttctggccgtacagacctcggccgacaattatgatatccgttccggtagacatgacatcctcaacagttcggtactgctgtccgagagcgtctcccttgtcgtcaagacccaccccgggggtcagaataagccagtcctcagagtcgcccttaggtcggttctgggcaatgaagccaaccacaaactcggggtcggatcgggcaagctcaatggtctgcttggagtactcgccagtggccagagagcccttgcaagacagctcggccagcatgagcagacctctggccagcttctcgttgggagaggggactaggaactccttgtactgggagttctcgtagtcagagacgtcctccttcttctgttcagagacagtttcctcggcaccagctcgcaggccagcaatgattccggttccgggtacaccgtgggcgttggtgatatcggaccactcggcgattcggtgacaccggtactggtgcttgacagtgttgccaatatctgcgaactttctgtcctcgaacaggaagaaaccgtgcttaagagcaagttccttgagggggagcacagtgccggcgtaggtgaagtcgtcaatgatgtcgatatgggttttgatcatgcacacataaggtccgaccttatcggcaagctcaatgagctccttggtggtggtaacatccagagaagcacacaggttggttttcttggctgccacgagcttgagcactcgagcggcaaaggcggacttgtggacgttagctcgagcttcgtaggagggcattttggtggtgaagaggagactgaaataaatttagtctgcagaactttttatcggaaccttatctggggcagtgaagtatatgttatggtaatagttacgagttagttgaacttatagatagactggactatacggctatcggtccaaattagaaagaacgtcaatggctctctgggcgtcgcctttgccgacaaaaatgtgatcatgatgaaagccagcaatgacgttgcagctgatattgttgtcggccaaccgcgccgaaaacgcagctgtcagacccacagcctccaacgaagaatgtatcgtcaaagtgatccaagcacactcatagttggagtcgtactccaaaggcggcaatgacgagtcagacagatactcgtcgacgtttaaaccatcatctaagggcctcaaaactacctcggaactgctgcgctgatctggacaccacagaggttccgagcactttaggttgcaccaaatgtcccaccaggtgcaggcagaaaacgctggaacagcgtgtacagtttgtcttaacaaaaagtgagggcgctgaggtcgagcagggtggtgtgacttgttatagcctttagagctgcgaaagcgcgtatggatttggctcatcaggccagattgagggtctgtggacacatgtcatgttagtgtacttcaatcgccccctggatatagccccgacaataggccgtggcctcatttttttgccttccgcacatttccattgctcggtacccacaccttgcttctcctgcacttgccaaccttaatactggtttacattgaccaacatcttacaagcggggggcttgtctagggtatatataaacagtggctctcccaatcggttgccagtctcttttttcctttctttccccacagattcgaaatctaaactacacatcacac

SEQ ID NO: 63 - DNA, 12110 bp, Artificial sequence
  pRF619
catggacaagaaatactccatcggcctggacattggaaccaactctgtcggctgggctgtcatcaccgacgagtacaaggtgccctccaagaaattcaaggtcctcggaaacaccgatcgacactccatcaagaaaaacctcattggtgccctgttgttcgattctggcgagactgccgaagctaccagactcaagcgaactgctcggcgacgttacacccgacggaagaaccgaatctgctacctgcaggagatcttttccaacgagatggccaaggtggacgattcgttctttcatcgactggaggaatccttcctcgtcgaggaagacaagaaacacgagcgtcatcccatctttggcaacattgtggacgaggttgcttaccacgagaagtatcctaccatctaccacctgcgaaagaaactcgtcgattccaccgacaaggcggatctcagacttatctacctcgctctggcacacatgatcaagtttcgaggtcatttcctcatcgagggcgatctcaatcccgacaacagcgatgtggacaagctgttcattcagctcgttcagacctacaaccagctgttcgaggaaaaccccatcaatgcctccggagtcgatgcaaaggccatcttgtctgctcgactctcgaagagcagacgactggagaacctcattgcccaacttcctggcgagaaaaagaacggactgtttggcaacctcattgccctttctcttggtctcacacccaacttcaagtccaacttcgatctggcggaggacgccaagctccagctgtccaaggacacctacgacgatgacctcgacaacctgcttgcacagattggcgatcagtacgccgacctgtttctcgctgccaagaacctttcggatgctattctcttgtctgacattctgcgagtcaacaccgagatcacaaaggctcccctttctgcctccatgatcaagcgatacgacgagcaccatcaggatctcacactgctcaaggctcttgtccgacagcaactgcccgagaagtacaaggagatctttttcgatcagtcgaagaacggctacgctggatacatcgacggcggagcctctcaggaagagttctacaagttcatcaagccaattctcgagaagatggacggaaccgaggaactgcttgtcaagctcaatcgagaggatctgcttcggaagcaacgaaccttcgacaacggcagcattcctcatcagatccacctcggtgagctgcacgccattcttcgacgtcaggaagacttctacccctttctcaaggacaaccgagagaagatcgagaagattcttacctttcgaatcccctactatgttggtcctcttgccagaggaaactctcgatttgcttggatgactcgaaagtccgaggaaaccatcactccctggaacttcgaggaagtcgtggacaagggtgcctctgcacagtccttcatcgagcgaatgaccaacttcgacaagaatctgcccaacgagaaggttcttcccaagcattcgctgctctacgagtactttacagtctacaacgaactcaccaaagtcaagtacgttaccgagggaatgcgaaagcctgccttcttgtctggcgaacagaagaaagccattgtcgatctcctgttcaagaccaaccgaaaggtcactgttaagcagctcaaggaggactacttcaagaaaatcgagtgtttcgacagcgtcgagatttccggagttgaggaccgattcaacgcctctttgggcacctatcacgatctgctcaagattatcaaggacaaggattttctcgacaacgaggaaaacgaggacattctggaggacatcgtgctcactcttaccctgttcgaagatcgggagatgatcgaggaacgactcaagacatacgctcacctgttcgacgacaaggtcatgaaacaactcaagcgacgtagatacaccggctggggaagactttcgcgaaagctcatcaacggcatcagagacaagcagtccggaaagaccattctggactttctcaagtccgatggctttgccaaccgaaacttcatgcagctcattcacgacgattctcttaccttcaaggaggacatccagaaggcacaagtgtccggtcagggcgacagcttgcacgaacatattgccaacctggctggttcgccagccatcaagaaaggcattctccagactgtcaaggttgtcgacgagctggtgaaggtcatgggacgtcacaagcccgagaacattgtgatcgagatggccagagagaaccagacaactcaaaagggtcagaaaaactcgcgagagcggatgaagcgaatcgaggaaggcatcaaggagctgggatcccagattctcaaggagcatcccgtcgagaacactcaactgcagaacgagaagctgtatctctactatctgcagaatggtcgagacatgtacgtggatcaggaactggacatcaatcgtctcagcgactacgatgtggaccacattgtccctcaatcctttctcaaggacgattctatcgacaacaaggtccttacacgatccgacaagaacagaggcaagtcggacaacgttcccagcgaagaggtggtcaaaaagatgaagaactactggcgacagctgctcaacgccaagctcattacccagcgaaagttcgacaatcttaccaaggccgagcgaggcggtctgtccgagctcgacaaggctggcttcatcaagcgtcaactcgtcgagaccagacagatcacaaagcacgtcgcacagattctcgattctcggatgaacaccaagtacgacgagaacgacaagctcatccgagaggtcaaggtgattactctcaagtccaaactggtctccgatttccgaaaggactttcagttctacaaggtgcgagagatcaacaattaccaccatgcccacgatgcttacctcaacgccgtcgttggcactgcgctcatcaagaaataccccaagctcgaaagcgagttcgtttacggcgattacaaggtctacgacgttcgaaagatgattgccaagtccgaacaggagattggcaaggctactgccaagtacttcttttactccaacatcatgaactttttcaagaccgagatcaccttggccaacggagagattcgaaagagaccacttatcgagaccaacggcgaaactggagagatcgtgtgggacaagggtcgagactttgcaaccgtgcgaaaggttctgtcgatgcctcaggtcaacatcgtcaagaaaaccgaggttcagactggcggattctccaaggagtcgattctgcccaagcgaaactccgacaagctcatcgctcgaaagaaagactgggatcccaagaaatacggtggcttcgattctcctaccgtcgcctattccgtgcttgtcgttgcgaaggtcgagaagggcaagtccaaaaagctcaagtccgtcaaggagctgctcggaattaccatcatggagcgatcgagcttcgagaagaatcccatcgacttcttggaagccaagggttacaaggaggtcaagaaagacctcattatcaagctgcccaagtactctctgttcgaactggagaacggtcgaaagcgtatgctcgcctccgctggcgagctgcagaagggaaacgagcttgccttgccttcgaagtacgtcaactttctctatctggcttctcactacgagaagctcaagggttctcccgaggacaacgaacagaagcaactcttcgttgagcagcacaaacattacctcgacgagattatcgagcagatttccgagttttcgaagcgagtcatcctggctgatgccaacttggacaaggtgctctctgcctacaacaagcatcgggacaaacccattcgagaacaggcggagaacatcattcacctgtttactcttaccaacctgggtgctcctgcagctttcaagtacttcgataccactatcgaccgaaagcggtacacatccaccaaggaggttctcgatgccaccctgattcaccagtccatcactggcctgtacgagacccgaatcgacctgtctcagcttggtggcgactccagagccgatcccaagaaaaagcgaaaggtctaagcggccgcaagtgtggatggggaagtgagtgcccggttctgtgtgcacaattggcaatccaagatggatggattcaacacagggatatagcgagctacgtggtggtgcgaggatatagcaacggatatttatgtttgacacttgagaatgtacgatacaagcactgtccaagtacaatactaaacatactgtacatactcatactcgtacccgggcaacggtttcacttgagtgcagtggctagtgctcttactcgtacagtgtgcaatactgcgtatcatagtctttgatgtatatcgtattcattcatgttagttgcgtacgagccggaagcataaagtgtaaagcctggggtgcctaatgagtgagctaactcacattaattgcgttgcgctcactgcccgctttccagtcgggaaacctgtcgtgccagctgcattaatgaatcggccaacgcgcggggagaggcggtttgcgtattgggcgctcttccgcttcctcgctcactgactcgctgcgctcggtcgttcggctgcggcgagcggtatcagctcactcaaaggcggtaatacggttatccacagaatcaggggataacgcaggaaagaacatgtgagcaaaaggccagcaaaaggccaggaaccgtaaaaaggccgcgttgctggcgtttttccataggctccgcccccctgacgagcatcacaaaaatcgacgctcaagtcagaggtggcgaaacccgacaggactataaagataccaggcgtttccccctggaagctccctcgtgcgctctcctgttccgaccctgccgcttaccggatacctgtccgcctttctcccttcgggaagcgtggcgctttctcatagctcacgctgtaggtatctcagttcggtgtaggtcgttcgctccaagctgggctgtgtgcacgaaccccccgttcagcccgaccgctgcgccttatccggtaactatcgtcttgagtccaacccggtaagacacgacttatcgccactggcagcagccactggtaacaggattagcagagcgaggtatgtaggcggtgctacagagttcttgaagtggtggcctaactacggctacactagaaggacagtatttggtatctgcgctctgctgaagccagttaccttcggaaaaagagttggtagctcttgatccggcaaacaaaccaccgctggtagcggtggtttttttgtttgcaagcagcagattacgcgcagaaaaaaaggatctcaagaagatcctttgatcttttctacggggtctgacgctcagtggaacgaaaactcacgttaagggattttggtcatgagattatcaaaaaggatcttcacctagatccttttaaattaaaaatgaagttttaaatcaatctaaagtatatatgagtaaacttggtctgacagttaccaatgcttaatcagtgaggcacctatctcagcgatctgtctatttcgttcatccatagttgcctgactccccgtcgtgtagataactacgatacgggagggcttaccatctggccccagtgctgcaatgataccgcgagacccacgctcaccggctccagatttatcagcaataaaccagccagccggaagggccgagcgcagaagtggtcctgcaactttatccgcctccatccagtctattaattgttgccgggaagctagagtaagtagttcgccagttaatagtttgcgcaacgttgttgccattgctacaggcatcgtggtgtcacgctcgtcgtttggtatggcttcattcagctccggttcccaacgatcaaggcgagttacatgatcccccatgttgtgcaaaaaagcggttagctccttcggtcctccgatcgttgtcagaagtaagttggccgcagtgttatcactcatggttatggcagcactgcataattctcttactgtcatgccatccgtaagatgcttttctgtgactggtgagtactcaaccaagtcattctgagaatagtgtatgcggcgaccgagttgctcttgcccggcgtcaatacgggataataccgcgccacatagcagaactttaaaagtgctcatcattggaaaacgttcttcggggcgaaaactctcaaggatcttaccgctgttgagatccagttcgatgtaacccactcgtgcacccaactgatcttcagcatcttttactttcaccagcgtttctgggtgagcaaaaacaggaaggcaaaatgccgcaaaaaagggaataagggcgacacggaaatgttgaatactcatactcttcctttttcaatattattgaagcatttatcagggttattgtctcatgagcggatacatatttgaatgtatttagaaaaataaacaaataggggttccgcgcacatttccccgaaaagtgccacctgacgcgccctgtagcggcgcattaagcgcggcgggtgtggtggttacgcgcagcgtgaccgctacacttgccagcgccctagcgcccgctcctttcgctttcttcccttcctttctcgccacgttcgccggctttccccgtcaagctctaaatcgggggctccctttagggttccgatttagtgctttacggcacctcgaccccaaaaaacttgattagggtgatggttcacgtagtgggccatcgccctgatagacggtttttcgccctttgacgttggagtccacgttctttaatagtggactcttgttccaaactggaacaacactcaaccctatctcggtctattcttttgatttataagggattttgccgatttcggcctattggttaaaaaatgagctgatttaacaaaaatttaacgcgaattttaacaaaatattaacgcttacaatttccattcgccattcaggctgcgcaactgttgggaagggcgatcggtgcgggcctcttcgctattacgccagctggcgaaagggggatgtgctgcaaggcgattaagttgggtaacgccagggttttcccagtcacgacgttgtaaaacgacggccagtgaattgtaatacgactcactatagggcgaattgggtaccgggccccccctcgaggtcgatggtgtcgataagcttgatatcgaattcatgtcacacaaaccgatcttcgcctcaaggaaacctaattctacatccgagagactgccgagatccagtctacactgattaattttcgggccaataatttaaaaaaatcgtgttatataatattatatgtattatatatatacatcatgatgatactgacagtcatgtcccattgctaaatagacagactccatctgccgcctccaactgatgttctcaatatttaaggggtcatctcgcattgtttaataataaacagactccatctaccgcctccaaatgatgttctcaaaatatattgtatgaacttatttttattacttagtattattagacaacttacttgctttatgaaaaacacttcctatttaggaaacaatttataatggcagttcgttcatttaacaatttatgtagaataaatgttataaatgcgtatgggaaatcttaaatatggatagcataaatgatatctgcattgcctaattcgaaatcaacagcaacgaaaaaaatcccttgtacaacataaatagtcatcgagaaatatcaactatcaaagaacagctattcacacgttactattgagattattattggacgagaatcacacactcaactgtctttctctcttctagaaatacaggtacaagtatgtactattctcattgttcatacttctagtcatttcatcccacatattccttggatttctctccaatgaatgacattctatcttgcaaattcaacaattataataagatataccaaagtagcggtatagtggcaatcaaaaagcttctctggtgtgcttctcgtatttatttttattctaatgatccattaaaggtatatatttatttcttgttatataatccttttgtttattacatgggctggatacataaaggtattttgatttaattttttgcttaaattcaatcccccctcgttcagtgtcaactgtaatggtaggaaattaccatacttttgaagaagcaaaaaaaatgaaagaaaaaaaaaatcgtatttccaggttagacgttccgcagaatctagaatgcggtatgcggtacattgttcttcgaacgtaaaagttgcgctccctgagatattgtacatttttgcttttacaagtacaagtacatcgtacaactatgtactactgttgatgcatccacaacagtttgttttgtttttttttgttttttttttttctaatgattcattaccgctatgtatacctacttgtacttgtagtaagccgggttattggcgttcaattaatcatagacttatgaatctgcacggtgtgcgctgcgagttacttttagcttatgcatgctacttgggtgtaatattgggatctgttcggaaatcaacggatgctcaatcgattggaagagatttcgaagcacgttgtttgatactccaatattttgactacttgtatttttgtttgcatgcatactccgaacttaacttgtcgaaaacatggcgacaggcaccgcaagatacagcatgtacatccttctacttgtagctcggtgaagatgaatatgtaaatactaaatatggatatatagataggagggatgtatatactcatcattgagcagttattaagtcattacctgctatatcgccgcatatcccaggttaccacccagagttgtcatcatcttaaccctgctttccctaaactgtaggtgctgagatatcagcctcaactgaacacaactgaatgcgtctgcttgaatcagcctctgaaagacgactgcgcatttaaaaacaatagaactactgcacgtcgcacctcagaaggtaacactctcttcgtggtcactaagcatactgcccaagtgttgttgtcccaaagtatgccacacccacacacacctctgggcacagctgacttccaggatattattacttctgttcataccatctccgttcatgaagtgttacaaaacagttacttatacgagtaataggagctcatgcaataaaacacgactacacccttcaatgaatggagtacacagctatgacactggggttacacttctcaaactacactcaccttgacttcgattcatacaatcgttctttaaattacatacagcagaaaacgagcaaaggcttgcacaacagcaatcaccacacgcggccaaaagcaccaccgactcggtgccactttttcaagttgataacggactagccttattttaacttgctatttctagctctaaaacgagggtgggtaatcgtttgaggtgtgatgtgtagtttagatttcgaatctgtggggaaagaaaggaaaaaagagactggcaaccgattgggagagccactgtttatatataccctagacaagccccccgcttgtaagatgttggtcaatgtaaaccagtattaaggttggcaagtgcaggagaagcaaggtgtgggtaccgagcaatggaaatgtgcggaaggcaaaaaaatgaggccacggcctattgtcggggctatatccagggggcgattgaagtacactaacatgacatgtgtccacagaccctcaatctggcctgatgagccaaatccatacgcgctttcgcagctctaaaggctataacaagtcacaccaccctgctcgacctcagcgccctcactttttgttaagacaaactgtacacgctgttccagcgttttctgcctgcacctggtgggacatttggtgcaacctaaagtgctcggaacctctgtggtgtccagatcagcgcagcagttccgaggtagttttgaggcccttagatgatggtttaaacttaattaagtcatacacaagtcagctttcttcgagcctcatataagtataagtagttcaacgtattagcactgtacccagcatctccgtatcgagaaacacaacaacatgccccattggacagatcatgcggatacacaggttgtgcagtatcatacatactcgatcagacaggtcgtctgaccatcatacaagctgaacaagcgctccatacttgcacgctctctatatacacagttaaattacatatccatagtctaacctctaacagttaatcttctggtaagcctcccagccagccttctggtatcgcttggcctcctcaataggatctcggttctggccgtacagacctcggccgacaattatgatatccgttccggtagacatgacatcctcaacagttcggtactgctgtccgagagcgtctcccttgtcgtcaagacccaccccgggggtcagaataagccagtcctcagagtcgcccttaggtcggttctgggcaatgaagccaaccacaaactcggggtcggatcgggcaagctcaatggtctgcttggagtactcgccagtggccagagagcccttgcaagacagctcggccagcatgagcagacctctggccagcttctcgttgggagaggggactaggaactccttgtactgggagttctcgtagtcagagacgtcctccttcttctgttcagagacagtttcctcggcaccagctcgcaggccagcaatgattccggttccgggtacaccgtgggcgttggtgatatcggaccactcggcgattcggtgacaccggtactggtgcttgacagtgttgccaatatctgcgaactttctgtcctcgaacaggaagaaaccgtgcttaagagcaagttccttgagggggagcacagtgccggcgtaggtgaagtcgtcaatgatgtcgatatgggttttgatcatgcacacataaggtccgaccttatcggcaagctcaatgagctccttggtggtggtaacatccagagaagcacacaggttggttttcttggctgccacgagcttgagcactcgagcggcaaaggcggacttgtggacgttagctcgagcttcgtaggagggcattttggtggtgaagaggagactgaaataaatttagtctgcagaactttttatcggaaccttatctggggcagtgaagtatatgttatggtaatagttacgagttagttgaacttatagatagactggactatacggctatcggtccaaattagaaagaacgtcaatggctctctgggcgtcgcctttgccgacaaaaatgtgatcatgatgaaagccagcaatgacgttgcagctgatattgttgtcggccaaccgcgccgaaaacgcagctgtcagacccacagcctccaacgaagaatgtatcgtcaaagtgatccaagcacactcatagttggagtcgtactccaaaggcggcaatgacgagtcagacagatactcgtcgacgtttaaaccatcatctaagggcctcaaaactacctcggaactgctgcgctgatctggacaccacagaggttccgagcactttaggttgcaccaaatgtcccaccaggtgcaggcagaaaacgctggaacagcgtgtacagtttgtcttaacaaaaagtgagggcgctgaggtcgagcagggtggtgtgacttgttatagcctttagagctgcgaaagcgcgtatggatttggctcatcaggccagattgagggtctgtggacacatgtcatgttagtgtacttcaatcgccccctggatatagccccgacaataggccgtggcctcatttttttgccttccgcacatttccattgctcggtacccacaccttgcttctcctgcacttgccaaccttaatactggtttacattgaccaacatcttacaagcggggggcttgtctagggtatatataaacagtggctctcccaatcggttgccagtctcttttttcctttctttccccacagattcgaaatctaaactacacatcacac

SEQ ID NO: 64 - DNA, 12177 bp, Artificial sequencce
  pRF618
catggacaagaaatactccatcggcctggacattggaaccaactctgtcggctgggctgtcatcaccgacgagtacaaggtgccctccaagaaattcaaggtcctcggaaacaccgatcgacactccatcaagaaaaacctcattggtgccctgttgttcgattctggcgagactgccgaagctaccagactcaagcgaactgctcggcgacgttacacccgacggaagaaccgaatctgctacctgcaggagatcttttccaacgagatggccaaggtggacgattcgttctttcatcgactggaggaatccttcctcgtcgaggaagacaagaaacacgagcgtcatcccatctttggcaacattgtggacgaggttgcttaccacgagaagtatcctaccatctaccacctgcgaaagaaactcgtcgattccaccgacaaggcggatctcagacttatctacctcgctctggcacacatgatcaagtttcgaggtcatttcctcatcgagggcgatctcaatcccgacaacagcgatgtggacaagctgttcattcagctcgttcagacctacaaccagctgttcgaggaaaaccccatcaatgcctccggagtcgatgcaaaggccatcttgtctgctcgactctcgaagagcagacgactggagaacctcattgcccaacttcctggcgagaaaaagaacggactgtttggcaacctcattgccctttctcttggtctcacacccaacttcaagtccaacttcgatctggcggaggacgccaagctccagctgtccaaggacacctacgacgatgacctcgacaacctgcttgcacagattggcgatcagtacgccgacctgtttctcgctgccaagaacctttcggatgctattctcttgtctgacattctgcgagtcaacaccgagatcacaaaggctcccctttctgcctccatgatcaagcgatacgacgagcaccatcaggatctcacactgctcaaggctcttgtccgacagcaactgcccgagaagtacaaggagatctttttcgatcagtcgaagaacggctacgctggatacatcgacggcggagcctctcaggaagagttctacaagttcatcaagccaattctcgagaagatggacggaaccgaggaactgcttgtcaagctcaatcgagaggatctgcttcggaagcaacgaaccttcgacaacggcagcattcctcatcagatccacctcggtgagctgcacgccattcttcgacgtcaggaagacttctacccctttctcaaggacaaccgagagaagatcgagaagattcttacctttcgaatcccctactatgttggtcctcttgccagaggaaactctcgatttgcttggatgactcgaaagtccgaggaaaccatcactccctggaacttcgaggaagtcgtggacaagggtgcctctgcacagtccttcatcgagcgaatgaccaacttcgacaagaatctgcccaacgagaaggttcttcccaagcattcgctgctctacgagtactttacagtctacaacgaactcaccaaagtcaagtacgttaccgagggaatgcgaaagcctgccttcttgtctggcgaacagaagaaagccattgtcgatctcctgttcaagaccaaccgaaaggtcactgttaagcagctcaaggaggactacttcaagaaaatcgagtgtttcgacagcgtcgagatttccggagttgaggaccgattcaacgcctctttgggcacctatcacgatctgctcaagattatcaaggacaaggattttctcgacaacgaggaaaacgaggacattctggaggacatcgtgctcactcttaccctgttcgaagatcgggagatgatcgaggaacgactcaagacatacgctcacctgttcgacgacaaggtcatgaaacaactcaagcgacgtagatacaccggctggggaagactttcgcgaaagctcatcaacggcatcagagacaagcagtccggaaagaccattctggactttctcaagtccgatggctttgccaaccgaaacttcatgcagctcattcacgacgattctcttaccttcaaggaggacatccagaaggcacaagtgtccggtcagggcgacagcttgcacgaacatattgccaacctggctggttcgccagccatcaagaaaggcattctccagactgtcaaggttgtcgacgagctggtgaaggtcatgggacgtcacaagcccgagaacattgtgatcgagatggccagagagaaccagacaactcaaaagggtcagaaaaactcgcgagagcggatgaagcgaatcgaggaaggcatcaaggagctgggatcccagattctcaaggagcatcccgtcgagaacactcaactgcagaacgagaagctgtatctctactatctgcagaatggtcgagacatgtacgtggatcaggaactggacatcaatcgtctcagcgactacgatgtggaccacattgtccctcaatcctttctcaaggacgattctatcgacaacaaggtccttacacgatccgacaagaacagaggcaagtcggacaacgttcccagcgaagaggtggtcaaaaagatgaagaactactggcgacagctgctcaacgccaagctcattacccagcgaaagttcgacaatcttaccaaggccgagcgaggcggtctgtccgagctcgacaaggctggcttcatcaagcgtcaactcgtcgagaccagacagatcacaaagcacgtcgcacagattctcgattctcggatgaacaccaagtacgacgagaacgacaagctcatccgagaggtcaaggtgattactctcaagtccaaactggtctccgatttccgaaaggactttcagttctacaaggtgcgagagatcaacaattaccaccatgcccacgatgcttacctcaacgccgtcgttggcactgcgctcatcaagaaataccccaagctcgaaagcgagttcgtttacggcgattacaaggtctacgacgttcgaaagatgattgccaagtccgaacaggagattggcaaggctactgccaagtacttcttttactccaacatcatgaactttttcaagaccgagatcaccttggccaacggagagattcgaaagagaccacttatcgagaccaacggcgaaactggagagatcgtgtgggacaagggtcgagactttgcaaccgtgcgaaaggttctgtcgatgcctcaggtcaacatcgtcaagaaaaccgaggttcagactggcggattctccaaggagtcgattctgcccaagcgaaactccgacaagctcatcgctcgaaagaaagactgggatcccaagaaatacggtggcttcgattctcctaccgtcgcctattccgtgcttgtcgttgcgaaggtcgagaagggcaagtccaaaaagctcaagtccgtcaaggagctgctcggaattaccatcatggagcgatcgagcttcgagaagaatcccatcgacttcttggaagccaagggttacaaggaggtcaagaaagacctcattatcaagctgcccaagtactctctgttcgaactggagaacggtcgaaagcgtatgctcgcctccgctggcgagctgcagaagggaaacgagcttgccttgccttcgaagtacgtcaactttctctatctggcttctcactacgagaagctcaagggttctcccgaggacaacgaacagaagcaactcttcgttgagcagcacaaacattacctcgacgagattatcgagcagatttccgagttttcgaagcgagtcatcctggctgatgccaacttggacaaggtgctctctgcctacaacaagcatcgggacaaacccattcgagaacaggcggagaacatcattcacctgtttactcttaccaacctgggtgctcctgcagctttcaagtacttcgataccactatcgaccgaaagcggtacacatccaccaaggaggttctcgatgccaccctgattcaccagtccatcactggcctgtacgagacccgaatcgacctgtctcagcttggtggcgactccagagccgatcccaagaaaaagcgaaaggtctaagcggccgcaagtgtggatggggaagtgagtgcccggttctgtgtgcacaattggcaatccaagatggatggattcaacacagggatatagcgagctacgtggtggtgcgaggatatagcaacggatatttatgtttgacacttgagaatgtacgatacaagcactgtccaagtacaatactaaacatactgtacatactcatactcgtacccgggcaacggtttcacttgagtgcagtggctagtgctcttactcgtacagtgtgcaatactgcgtatcatagtctttgatgtatatcgtattcattcatgttagttgcgtacgagccggaagcataaagtgtaaagcctggggtgcctaatgagtgagctaactcacattaattgcgttgcgctcactgcccgctttccagtcgggaaacctgtcgtgccagctgcattaatgaatcggccaacgcgcggggagaggcggtttgcgtattgggcgctcttccgcttcctcgctcactgactcgctgcgctcggtcgttcggctgcggcgagcggtatcagctcactcaaaggcggtaatacggttatccacagaatcaggggataacgcaggaaagaacatgtgagcaaaaggccagcaaaaggccaggaaccgtaaaaaggccgcgttgctggcgtttttccataggctccgcccccctgacgagcatcacaaaaatcgacgctcaagtcagaggtggcgaaacccgacaggactataaagataccaggcgtttccccctggaagctccctcgtgcgctctcctgttccgaccctgccgcttaccggatacctgtccgcctttctcccttcgggaagcgtggcgctttctcatagctcacgctgtaggtatctcagttcggtgtaggtcgttcgctccaagctgggctgtgtgcacgaaccccccgttcagcccgaccgctgcgccttatccggtaactatcgtcttgagtccaacccggtaagacacgacttatcgccactggcagcagccactggtaacaggattagcagagcgaggtatgtaggcggtgctacagagttcttgaagtggtggcctaactacggctacactagaaggacagtatttggtatctgcgctctgctgaagccagttaccttcggaaaaagagttggtagctcttgatccggcaaacaaaccaccgctggtagcggtggtttttttgtttgcaagcagcagattacgcgcagaaaaaaaggatctcaagaagatcctttgatcttttctacggggtctgacgctcagtggaacgaaaactcacgttaagggattttggtcatgagattatcaaaaaggatcttcacctagatccttttaaattaaaaatgaagttttaaatcaatctaaagtatatatgagtaaacttggtctgacagttaccaatgcttaatcagtgaggcacctatctcagcgatctgtctatttcgttcatccatagttgcctgactccccgtcgtgtagataactacgatacgggagggcttaccatctggccccagtgctgcaatgataccgcgagacccacgctcaccggctccagatttatcagcaataaaccagccagccggaagggccgagcgcagaagtggtcctgcaactttatccgcctccatccagtctattaattgttgccgggaagctagagtaagtagttcgccagttaatagtttgcgcaacgttgttgccattgctacaggcatcgtggtgtcacgctcgtcgtttggtatggcttcattcagctccggttcccaacgatcaaggcgagttacatgatcccccatgttgtgcaaaaaagcggttagctccttcggtcctccgatcgttgtcagaagtaagttggccgcagtgttatcactcatggttatggcagcactgcataattctcttactgtcatgccatccgtaagatgcttttctgtgactggtgagtactcaaccaagtcattctgagaatagtgtatgcggcgaccgagttgctcttgcccggcgtcaatacgggataataccgcgccacatagcagaactttaaaagtgctcatcattggaaaacgttcttcggggcgaaaactctcaaggatcttaccgctgttgagatccagttcgatgtaacccactcgtgcacccaactgatcttcagcatcttttactttcaccagcgtttctgggtgagcaaaaacaggaaggcaaaatgccgcaaaaaagggaataagggcgacacggaaatgttgaatactcatactcttcctttttcaatattattgaagcatttatcagggttattgtctcatgagcggatacatatttgaatgtatttagaaaaataaacaaataggggttccgcgcacatttccccgaaaagtgccacctgacgcgccctgtagcggcgcattaagcgcggcgggtgtggtggttacgcgcagcgtgaccgctacacttgccagcgccctagcgcccgctcctttcgctttcttcccttcctttctcgccacgttcgccggctttccccgtcaagctctaaatcgggggctccctttagggttccgatttagtgctttacggcacctcgaccccaaaaaacttgattagggtgatggttcacgtagtgggccatcgccctgatagacggtttttcgccctttgacgttggagtccacgttctttaatagtggactcttgttccaaactggaacaacactcaaccctatctcggtctattcttttgatttataagggattttgccgatttcggcctattggttaaaaaatgagctgatttaacaaaaatttaacgcgaattttaacaaaatattaacgcttacaatttccattcgccattcaggctgcgcaactgttgggaagggcgatcggtgcgggcctcttcgctattacgccagctggcgaaagggggatgtgctgcaaggcgattaagttgggtaacgccagggttttcccagtcacgacgttgtaaaacgacggccagtgaattgtaatacgactcactatagggcgaattgggtaccgggccccccctcgaggtcgatggtgtcgataagcttgatatcgaattcatgtcacacaaaccgatcttcgcctcaaggaaacctaattctacatccgagagactgccgagatccagtctacactgattaattttcgggccaataatttaaaaaaatcgtgttatataatattatatgtattatatatatacatcatgatgatactgacagtcatgtcccattgctaaatagacagactccatctgccgcctccaactgatgttctcaatatttaaggggtcatctcgcattgtttaataataaacagactccatctaccgcctccaaatgatgttctcaaaatatattgtatgaacttatttttattacttagtattattagacaacttacttgctttatgaaaaacacttcctatttaggaaacaatttataatggcagttcgttcatttaacaatttatgtagaataaatgttataaatgcgtatgggaaatcttaaatatggatagcataaatgatatctgcattgcctaattcgaaatcaacagcaacgaaaaaaatcccttgtacaacataaatagtcatcgagaaatatcaactatcaaagaacagctattcacacgttactattgagattattattggacgagaatcacacactcaactgtctttctctcttctagaaatacaggtacaagtatgtactattctcattgttcatacttctagtcatttcatcccacatattccttggatttctctccaatgaatgacattctatcttgcaaattcaacaattataataagatataccaaagtagcggtatagtggcaatcaaaaagcttctctggtgtgcttctcgtatttatttttattctaatgatccattaaaggtatatatttatttcttgttatataatccttttgtttattacatgggctggatacataaaggtattttgatttaattttttgcttaaattcaatcccccctcgttcagtgtcaactgtaatggtaggaaattaccatacttttgaagaagcaaaaaaaatgaaagaaaaaaaaaatcgtatttccaggttagacgttccgcagaatctagaatgcggtatgcggtacattgttcttcgaacgtaaaagttgcgctccctgagatattgtacatttttgcttttacaagtacaagtacatcgtacaactatgtactactgttgatgcatccacaacagtttgttttgtttttttttgttttttttttttctaatgattcattaccgctatgtatacctacttgtacttgtagtaagccgggttattggcgttcaattaatcatagacttatgaatctgcacggtgtgcgctgcgagttacttttagcttatgcatgctacttgggtgtaatattgggatctgttcggaaatcaacggatgctcaatcgattggaagagatttcgaagcacgttgtttgatactccaatattttgactacttgtatttttgtttgcatgcatactccgaacttaacttgtcgaaaacatggcgacaggcaccgcaagatacagcatgtacatccttctacttgtagctcggtgaagatgaatatgtaaatactaaatatggatatatagataggagggatgtatatactcatcattgagcagttattaagtcattacctgctatatcgccgcatatcccaggttaccacccagagttgtcatcatcttaaccctgctttccctaaactgtaggtgctgagatatcagcctcaactgaacacaactgaatgcgtctgcttgaatcagcctctgaaagacgactgcgcatttaaaaacaatagaactactgcacgtcgcacctcagaaggtaacactctcttcgtggtcactaagcatactgcccaagtgttgttgtcccaaagtatgccacacccacacacacctctgggcacagctgacttccaggatattattacttctgttcataccatctccgttcatgaagtgttacaaaacagttacttatacgagtaataggagctcatgcaataaaacacgactacacccttcaatgaatggagtacacagctatgacactggggttacacttctcaaactacactcaccttgacttcgattcatacaatcgttctttaaattacatacagcagaaaacgagcaaaggcttgcacaacagcaatcaccacacgcggcctcccattcgccatgccgaagcatgttgcccagccggcgccagcgaggaggctgggaccatgccggccaaaagcaccaccgactcggtgccactttttcaagttgataacggactagccttattttaacttgctatttctagctctaaaacgagggtgggtaatcgtttgaggtgtgatgtgtagtttagatttcgaatctgtggggaaagaaaggaaaaaagagactggcaaccgattgggagagccactgtttatatataccctagacaagccccccgcttgtaagatgttggtcaatgtaaaccagtattaaggttggcaagtgcaggagaagcaaggtgtgggtaccgagcaatggaaatgtgcggaaggcaaaaaaatgaggccacggcctattgtcggggctatatccagggggcgattgaagtacactaacatgacatgtgtccacagaccctcaatctggcctgatgagccaaatccatacgcgctttcgcagctctaaaggctataacaagtcacaccaccctgctcgacctcagcgccctcactttttgttaagacaaactgtacacgctgttccagcgttttctgcctgcacctggtgggacatttggtgcaacctaaagtgctcggaacctctgtggtgtccagatcagcgcagcagttccgaggtagttttgaggcccttagatgatggtttaaacttaattaagtcatacacaagtcagctttcttcgagcctcatataagtataagtagttcaacgtattagcactgtacccagcatctccgtatcgagaaacacaacaacatgccccattggacagatcatgcggatacacaggttgtgcagtatcatacatactcgatcagacaggtcgtctgaccatcatacaagctgaacaagcgctccatacttgcacgctctctatatacacagttaaattacatatccatagtctaacctctaacagttaatcttctggtaagcctcccagccagccttctggtatcgcttggcctcctcaataggatctcggttctggccgtacagacctcggccgacaattatgatatccgttccggtagacatgacatcctcaacagttcggtactgctgtccgagagcgtctcccttgtcgtcaagacccaccccgggggtcagaataagccagtcctcagagtcgcccttaggtcggttctgggcaatgaagccaaccacaaactcggggtcggatcgggcaagctcaatggtctgcttggagtactcgccagtggccagagagcccttgcaagacagctcggccagcatgagcagacctctggccagcttctcgttgggagaggggactaggaactccttgtactgggagttctcgtagtcagagacgtcctccttcttctgttcagagacagtttcctcggcaccagctcgcaggccagcaatgattccggttccgggtacaccgtgggcgttggtgatatcggaccactcggcgattcggtgacaccggtactggtgcttgacagtgttgccaatatctgcgaactttctgtcctcgaacaggaagaaaccgtgcttaagagcaagttccttgagggggagcacagtgccggcgtaggtgaagtcgtcaatgatgtcgatatgggttttgatcatgcacacataaggtccgaccttatcggcaagctcaatgagctccttggtggtggtaacatccagagaagcacacaggttggttttcttggctgccacgagcttgagcactcgagcggcaaaggcggacttgtggacgttagctcgagcttcgtaggagggcattttggtggtgaagaggagactgaaataaatttagtctgcagaactttttatcggaaccttatctggggcagtgaagtatatgttatggtaatagttacgagttagttgaacttatagatagactggactatacggctatcggtccaaattagaaagaacgtcaatggctctctgggcgtcgcctttgccgacaaaaatgtgatcatgatgaaagccagcaatgacgttgcagctgatattgttgtcggccaaccgcgccgaaaacgcagctgtcagacccacagcctccaacgaagaatgtatcgtcaaagtgatccaagcacactcatagttggagtcgtactccaaaggcggcaatgacgagtcagacagatactcgtcgacgtttaaaccatcatctaagggcctcaaaactacctcggaactgctgcgctgatctggacaccacagaggttccgagcactttaggttgcaccaaatgtcccaccaggtgcaggcagaaaacgctggaacagcgtgtacagtttgtcttaacaaaaagtgagggcgctgaggtcgagcagggtggtgtgacttgttatagcctttagagctgcgaaagcgcgtatggatttggctcatcaggccagattgagggtctgtggacacatgtcatgttagtgtacttcaatcgccccctggatatagccccgacaataggccgtggcctcatttttttgccttccgcacatttccattgctcggtacccacaccttgcttctcctgcacttgccaaccttaatactggtttacattgaccaacatcttacaagcggggggcttgtctagggtatatataaacagtggctctcccaatcggttgccagtctcttttttcctttctttccccacagattcgaaatctaaactacacatcacac

SEQ ID NO: 65 - DNA, 11926 bp, Artificial sequence
  pRF626
catggacaagaaatactccatcggcctggacattggaaccaactctgtcggctgggctgtcatcaccgacgagtacaaggtgccctccaagaaattcaaggtcctcggaaacaccgatcgacactccatcaagaaaaacctcattggtgccctgttgttcgattctggcgagactgccgaagctaccagactcaagcgaactgctcggcgacgttacacccgacggaagaaccgaatctgctacctgcaggagatcttttccaacgagatggccaaggtggacgattcgttctttcatcgactggaggaatccttcctcgtcgaggaagacaagaaacacgagcgtcatcccatctttggcaacattgtggacgaggttgcttaccacgagaagtatcctaccatctaccacctgcgaaagaaactcgtcgattccaccgacaaggcggatctcagacttatctacctcgctctggcacacatgatcaagtttcgaggtcatttcctcatcgagggcgatctcaatcccgacaacagcgatgtggacaagctgttcattcagctcgttcagacctacaaccagctgttcgaggaaaaccccatcaatgcctccggagtcgatgcaaaggccatcttgtctgctcgactctcgaagagcagacgactggagaacctcattgcccaacttcctggcgagaaaaagaacggactgtttggcaacctcattgccctttctcttggtctcacacccaacttcaagtccaacttcgatctggcggaggacgccaagctccagctgtccaaggacacctacgacgatgacctcgacaacctgcttgcacagattggcgatcagtacgccgacctgtttctcgctgccaagaacctttcggatgctattctcttgtctgacattctgcgagtcaacaccgagatcacaaaggctcccctttctgcctccatgatcaagcgatacgacgagcaccatcaggatctcacactgctcaaggctcttgtccgacagcaactgcccgagaagtacaaggagatctttttcgatcagtcgaagaacggctacgctggatacatcgacggcggagcctctcaggaagagttctacaagttcatcaagccaattctcgagaagatggacggaaccgaggaactgcttgtcaagctcaatcgagaggatctgcttcggaagcaacgaaccttcgacaacggcagcattcctcatcagatccacctcggtgagctgcacgccattcttcgacgtcaggaagacttctacccctttctcaaggacaaccgagagaagatcgagaagattcttacctttcgaatcccctactatgttggtcctcttgccagaggaaactctcgatttgcttggatgactcgaaagtccgaggaaaccatcactccctggaacttcgaggaagtcgtggacaagggtgcctctgcacagtccttcatcgagcgaatgaccaacttcgacaagaatctgcccaacgagaaggttcttcccaagcattcgctgctctacgagtactttacagtctacaacgaactcaccaaagtcaagtacgttaccgagggaatgcgaaagcctgccttcttgtctggcgaacagaagaaagccattgtcgatctcctgttcaagaccaaccgaaaggtcactgttaagcagctcaaggaggactacttcaagaaaatcgagtgtttcgacagcgtcgagatttccggagttgaggaccgattcaacgcctctttgggcacctatcacgatctgctcaagattatcaaggacaaggattttctcgacaacgaggaaaacgaggacattctggaggacatcgtgctcactcttaccctgttcgaagatcgggagatgatcgaggaacgactcaagacatacgctcacctgttcgacgacaaggtcatgaaacaactcaagcgacgtagatacaccggctggggaagactttcgcgaaagctcatcaacggcatcagagacaagcagtccggaaagaccattctggactttctcaagtccgatggctttgccaaccgaaacttcatgcagctcattcacgacgattctcttaccttcaaggaggacatccagaaggcacaagtgtccggtcagggcgacagcttgcacgaacatattgccaacctggctggttcgccagccatcaagaaaggcattctccagactgtcaaggttgtcgacgagctggtgaaggtcatgggacgtcacaagcccgagaacattgtgatcgagatggccagagagaaccagacaactcaaaagggtcagaaaaactcgcgagagcggatgaagcgaatcgaggaaggcatcaaggagctgggatcccagattctcaaggagcatcccgtcgagaacactcaactgcagaacgagaagctgtatctctactatctgcagaatggtcgagacatgtacgtggatcaggaactggacatcaatcgtctcagcgactacgatgtggaccacattgtccctcaatcctttctcaaggacgattctatcgacaacaaggtccttacacgatccgacaagaacagaggcaagtcggacaacgttcccagcgaagaggtggtcaaaaagatgaagaactactggcgacagctgctcaacgccaagctcattacccagcgaaagttcgacaatcttaccaaggccgagcgaggcggtctgtccgagctcgacaaggctggcttcatcaagcgtcaactcgtcgagaccagacagatcacaaagcacgtcgcacagattctcgattctcggatgaacaccaagtacgacgagaacgacaagctcatccgagaggtcaaggtgattactctcaagtccaaactggtctccgatttccgaaaggactttcagttctacaaggtgcgagagatcaacaattaccaccatgcccacgatgcttacctcaacgccgtcgttggcactgcgctcatcaagaaataccccaagctcgaaagcgagttcgtttacggcgattacaaggtctacgacgttcgaaagatgattgccaagtccgaacaggagattggcaaggctactgccaagtacttcttttactccaacatcatgaactttttcaagaccgagatcaccttggccaacggagagattcgaaagagaccacttatcgagaccaacggcgaaactggagagatcgtgtgggacaagggtcgagactttgcaaccgtgcgaaaggttctgtcgatgcctcaggtcaacatcgtcaagaaaaccgaggttcagactggcggattctccaaggagtcgattctgcccaagcgaaactccgacaagctcatcgctcgaaagaaagactgggatcccaagaaatacggtggcttcgattctcctaccgtcgcctattccgtgcttgtcgttgcgaaggtcgagaagggcaagtccaaaaagctcaagtccgtcaaggagctgctcggaattaccatcatggagcgatcgagcttcgagaagaatcccatcgacttcttggaagccaagggttacaaggaggtcaagaaagacctcattatcaagctgcccaagtactctctgttcgaactggagaacggtcgaaagcgtatgctcgcctccgctggcgagctgcagaagggaaacgagcttgccttgccttcgaagtacgtcaactttctctatctggcttctcactacgagaagctcaagggttctcccgaggacaacgaacagaagcaactcttcgttgagcagcacaaacattacctcgacgagattatcgagcagatttccgagttttcgaagcgagtcatcctggctgatgccaacttggacaaggtgctctctgcctacaacaagcatcgggacaaacccattcgagaacaggcggagaacatcattcacctgtttactcttaccaacctgggtgctcctgcagctttcaagtacttcgataccactatcgaccgaaagcggtacacatccaccaaggaggttctcgatgccaccctgattcaccagtccatcactggcctgtacgagacccgaatcgacctgtctcagcttggtggcgactccagagccgatcccaagaaaaagcgaaaggtctaagcggccgcaagtgtggatggggaagtgagtgcccggttctgtgtgcacaattggcaatccaagatggatggattcaacacagggatatagcgagctacgtggtggtgcgaggatatagcaacggatatttatgtttgacacttgagaatgtacgatacaagcactgtccaagtacaatactaaacatactgtacatactcatactcgtacccgggcaacggtttcacttgagtgcagtggctagtgctcttactcgtacagtgtgcaatactgcgtatcatagtctttgatgtatatcgtattcattcatgttagttgcgtacgagccggaagcataaagtgtaaagcctggggtgcctaatgagtgagctaactcacattaattgcgttgcgctcactgcccgctttccagtcgggaaacctgtcgtgccagctgcattaatgaatcggccaacgcgcggggagaggcggtttgcgtattgggcgctcttccgcttcctcgctcactgactcgctgcgctcggtcgttcggctgcggcgagcggtatcagctcactcaaaggcggtaatacggttatccacagaatcaggggataacgcaggaaagaacatgtgagcaaaaggccagcaaaaggccaggaaccgtaaaaaggccgcgttgctggcgtttttccataggctccgcccccctgacgagcatcacaaaaatcgacgctcaagtcagaggtggcgaaacccgacaggactataaagataccaggcgtttccccctggaagctccctcgtgcgctctcctgttccgaccctgccgcttaccggatacctgtccgcctttctcccttcgggaagcgtggcgctttctcatagctcacgctgtaggtatctcagttcggtgtaggtcgttcgctccaagctgggctgtgtgcacgaaccccccgttcagcccgaccgctgcgccttatccggtaactatcgtcttgagtccaacccggtaagacacgacttatcgccactggcagcagccactggtaacaggattagcagagcgaggtatgtaggcggtgctacagagttcttgaagtggtggcctaactacggctacactagaaggacagtatttggtatctgcgctctgctgaagccagttaccttcggaaaaagagttggtagctcttgatccggcaaacaaaccaccgctggtagcggtggtttttttgtttgcaagcagcagattacgcgcagaaaaaaaggatctcaagaagatcctttgatcttttctacggggtctgacgctcagtggaacgaaaactcacgttaagggattttggtcatgagattatcaaaaaggatcttcacctagatccttttaaattaaaaatgaagttttaaatcaatctaaagtatatatgagtaaacttggtctgacagttaccaatgcttaatcagtgaggcacctatctcagcgatctgtctatttcgttcatccatagttgcctgactccccgtcgtgtagataactacgatacgggagggcttaccatctggccccagtgctgcaatgataccgcgagacccacgctcaccggctccagatttatcagcaataaaccagccagccggaagggccgagcgcagaagtggtcctgcaactttatccgcctccatccagtctattaattgttgccgggaagctagagtaagtagttcgccagttaatagtttgcgcaacgttgttgccattgctacaggcatcgtggtgtcacgctcgtcgtttggtatggcttcattcagctccggttcccaacgatcaaggcgagttacatgatcccccatgttgtgcaaaaaagcggttagctccttcggtcctccgatcgttgtcagaagtaagttggccgcagtgttatcactcatggttatggcagcactgcataattctcttactgtcatgccatccgtaagatgcttttctgtgactggtgagtactcaaccaagtcattctgagaatagtgtatgcggcgaccgagttgctcttgcccggcgtcaatacgggataataccgcgccacatagcagaactttaaaagtgctcatcattggaaaacgttcttcggggcgaaaactctcaaggatcttaccgctgttgagatccagttcgatgtaacccactcgtgcacccaactgatcttcagcatcttttactttcaccagcgtttctgggtgagcaaaaacaggaaggcaaaatgccgcaaaaaagggaataagggcgacacggaaatgttgaatactcatactcttcctttttcaatattattgaagcatttatcagggttattgtctcatgagcggatacatatttgaatgtatttagaaaaataaacaaataggggttccgcgcacatttccccgaaaagtgccacctgacgcgccctgtagcggcgcattaagcgcggcgggtgtggtggttacgcgcagcgtgaccgctacacttgccagcgccctagcgcccgctcctttcgctttcttcccttcctttctcgccacgttcgccggctttccccgtcaagctctaaatcgggggctccctttagggttccgatttagtgctttacggcacctcgaccccaaaaaacttgattagggtgatggttcacgtagtgggccatcgccctgatagacggtttttcgccctttgacgttggagtccacgttctttaatagtggactcttgttccaaactggaacaacactcaaccctatctcggtctattcttttgatttataagggattttgccgatttcggcctattggttaaaaaatgagctgatttaacaaaaatttaacgcgaattttaacaaaatattaacgcttacaatttccattcgccattcaggctgcgcaactgttgggaagggcgatcggtgcgggcctcttcgctattacgccagctggcgaaagggggatgtgctgcaaggcgattaagttgggtaacgccagggttttcccagtcacgacgttgtaaaacgacggccagtgaattgtaatacgactcactatagggcgaattgggtaccgggccccccctcgaggtcgatggtgtcgataagcttgatatcgaattcatgtcacacaaaccgatcttcgcctcaaggaaacctaattctacatccgagagactgccgagatccagtctacactgattaattttcgggccaataatttaaaaaaatcgtgttatataatattatatgtattatatatatacatcatgatgatactgacagtcatgtcccattgctaaatagacagactccatctgccgcctccaactgatgttctcaatatttaaggggtcatctcgcattgtttaataataaacagactccatctaccgcctccaaatgatgttctcaaaatatattgtatgaacttatttttattacttagtattattagacaacttacttgctttatgaaaaacacttcctatttaggaaacaatttataatggcagttcgttcatttaacaatttatgtagaataaatgttataaatgcgtatgggaaatcttaaatatggatagcataaatgatatctgcattgcctaattcgaaatcaacagcaacgaaaaaaatcccttgtacaacataaatagtcatcgagaaatatcaactatcaaagaacagctattcacacgttactattgagattattattggacgagaatcacacactcaactgtctttctctcttctagaaatacaggtacaagtatgtactattctcattgttcatacttctagtcatttcatcccacatattccttggatttctctccaatgaatgacattctatcttgcaaattcaacaattataataagatataccaaagtagcggtatagtggcaatcaaaaagcttctctggtgtgcttctcgtatttatttttattctaatgatccattaaaggtatatatttatttcttgttatataatccttttgtttattacatgggctggatacataaaggtattttgatttaattttttgcttaaattcaatcccccctcgttcagtgtcaactgtaatggtaggaaattaccatacttttgaagaagcaaaaaaaatgaaagaaaaaaaaaatcgtatttccaggttagacgttccgcagaatctagaatgcggtatgcggtacattgttcttcgaacgtaaaagttgcgctccctgagatattgtacatttttgcttttacaagtacaagtacatcgtacaactatgtactactgttgatgcatccacaacagtttgttttgtttttttttgttttttttttttctaatgattcattaccgctatgtatacctacttgtacttgtagtaagccgggttattggcgttcaattaatcatagacttatgaatctgcacggtgtgcgctgcgagttacttttagcttatgcatgctacttgggtgtaatattgggatctgttcggaaatcaacggatgctcaatcgattggaagagatttcgaagcacgttgtttgatactccaatattttgactacttgtatttttgtttgcatgcatactccgaacttaacttgtcgaaaacatggcgacaggcaccgcaagatacagcatgtacatccttctacttgtagctcggtgaagatgaatatgtaaatactaaatatggatatatagataggagggatgtatatactcatcattgagcagttattaagtcattacctgctatatcgccgcatatcccaggttaccacccagagttgtcatcatcttaaccctgctttccctaaactgtaggtgctgagatatcagcctcaactgaacacaactgaatgcgtctgcttgaatcagcctctgaaagacgactgcgcatttaaaaacaatagaactactgcacgtcgcacctcagaaggtaacactctcttcgtggtcactaagcatactgcccaagtgttgttgtcccaaagtatgccacacccacacacacctctgggcacagctgacttccaggatattattacttctgttcataccatctccgttcatgaagtgttacaaaacagttacttatacgagtaataggagctcatgcaataaaacacgactacacccttcaatgaatggagtacacagctatgacactggggttacacttctcaaactacactcaccttgacttcgattcatacaatcgttctttaaattacatacagcagaaaacgagcaaaggcttgcacaacagcaatcaccacacgcggccaaaagcaccaccgactcggtgccactttttcaagttgataacggactagccttattttaacttgctatttctagctctaaaacgagggtgggtaatcgtttgattgacaaggagagagagaaaagaagaggaaaggtaattcggggacggtggtcttttatacccttggctaaagtcccaaccacaaagcaaaaaaattttcagtagtctattttgcgtccggcatgggttacccggatggccagacaaagaaactagtacaaagtctgaacaagcgtagattccagactgcagtaccctacgcccttaacggcaagtgtgggaaccgggggaggtttgatatgtggggagaagggggctctcgccggggttgggcccgctactgggtcaatttggggtcaattggggcaattggggctgttttttgggacacaaatgcgccgccaacccggtctctttaattaagtcatacacaagtcagctttcttcgagcctcatataagtataagtagttcaacgtattagcactgtacccagcatctccgtatcgagaaacacaacaacatgccccattggacagatcatgcggatacacaggttgtgcagtatcatacatactcgatcagacaggtcgtctgaccatcatacaagctgaacaagcgctccatacttgcacgctctctatatacacagttaaattacatatccatagtctaacctctaacagttaatcttctggtaagcctcccagccagccttctggtatcgcttggcctcctcaataggatctcggttctggccgtacagacctcggccgacaattatgatatccgttccggtagacatgacatcctcaacagttcggtactgctgtccgagagcgtctcccttgtcgtcaagacccaccccgggggtcagaataagccagtcctcagagtcgcccttaggtcggttctgggcaatgaagccaaccacaaactcggggtcggatcgggcaagctcaatggtctgcttggagtactcgccagtggccagagagcccttgcaagacagctcggccagcatgagcagacctctggccagcttctcgttgggagaggggactaggaactccttgtactgggagttctcgtagtcagagacgtcctccttcttctgttcagagacagtttcctcggcaccagctcgcaggccagcaatgattccggttccgggtacaccgtgggcgttggtgatatcggaccactcggcgattcggtgacaccggtactggtgcttgacagtgttgccaatatctgcgaactttctgtcctcgaacaggaagaaaccgtgcttaagagcaagttccttgagggggagcacagtgccggcgtaggtgaagtcgtcaatgatgtcgatatgggttttgatcatgcacacataaggtccgaccttatcggcaagctcaatgagctccttggtggtggtaacatccagagaagcacacaggttggttttcttggctgccacgagcttgagcactcgagcggcaaaggcggacttgtggacgttagctcgagcttcgtaggagggcattttggtggtgaagaggagactgaaataaatttagtctgcagaactttttatcggaaccttatctggggcagtgaagtatatgttatggtaatagttacgagttagttgaacttatagatagactggactatacggctatcggtccaaattagaaagaacgtcaatggctctctgggcgtcgcctttgccgacaaaaatgtgatcatgatgaaagccagcaatgacgttgcagctgatattgttgtcggccaaccgcgccgaaaacgcagctgtcagacccacagcctccaacgaagaatgtatcgtcaaagtgatccaagcacactcatagttggagtcgtactccaaaggcggcaatgacgagtcagacagatactcgtcgacgtttaaaccatcatctaagggcctcaaaactacctcggaactgctgcgctgatctggacaccacagaggttccgagcactttaggttgcaccaaatgtcccaccaggtgcaggcagaaaacgctggaacagcgtgtacagtttgtcttaacaaaaagtgagggcgctgaggtcgagcagggtggtgtgacttgttatagcctttagagctgcgaaagcgcgtatggatttggctcatcaggccagattgagggtctgtggacacatgtcatgttagtgtacttcaatcgccccctggatatagccccgacaataggccgtggcctcatttttttgccttccgcacatttccattgctcggtacccacaccttgcttctcctgcacttgccaaccttaatactggtttacattgaccaacatcttacaagcggggggcttgtctagggtatatataaacagtggctctcccaatcggttgccagtctcttttttcctttctttccccacagattcgaaatctaaactacacatcacac

SEQ ID NO: 66 - DNA, 11993 bp, Artificial sequence
  pRF625
catggacaagaaatactccatcggcctggacattggaaccaactctgtcggctgggctgtcatcaccgacgagtacaaggtgccctccaagaaattcaaggtcctcggaaacaccgatcgacactccatcaagaaaaacctcattggtgccctgttgttcgattctggcgagactgccgaagctaccagactcaagcgaactgctcggcgacgttacacccgacggaagaaccgaatctgctacctgcaggagatcttttccaacgagatggccaaggtggacgattcgttctttcatcgactggaggaatccttcctcgtcgaggaagacaagaaacacgagcgtcatcccatctttggcaacattgtggacgaggttgcttaccacgagaagtatcctaccatctaccacctgcgaaagaaactcgtcgattccaccgacaaggcggatctcagacttatctacctcgctctggcacacatgatcaagtttcgaggtcatttcctcatcgagggcgatctcaatcccgacaacagcgatgtggacaagctgttcattcagctcgttcagacctacaaccagctgttcgaggaaaaccccatcaatgcctccggagtcgatgcaaaggccatcttgtctgctcgactctcgaagagcagacgactggagaacctcattgcccaacttcctggcgagaaaaagaacggactgtttggcaacctcattgccctttctcttggtctcacacccaacttcaagtccaacttcgatctggcggaggacgccaagctccagctgtccaaggacacctacgacgatgacctcgacaacctgcttgcacagattggcgatcagtacgccgacctgtttctcgctgccaagaacctttcggatgctattctcttgtctgacattctgcgagtcaacaccgagatcacaaaggctcccctttctgcctccatgatcaagcgatacgacgagcaccatcaggatctcacactgctcaaggctcttgtccgacagcaactgcccgagaagtacaaggagatctttttcgatcagtcgaagaacggctacgctggatacatcgacggcggagcctctcaggaagagttctacaagttcatcaagccaattctcgagaagatggacggaaccgaggaactgcttgtcaagctcaatcgagaggatctgcttcggaagcaacgaaccttcgacaacggcagcattcctcatcagatccacctcggtgagctgcacgccattcttcgacgtcaggaagacttctacccctttctcaaggacaaccgagagaagatcgagaagattcttacctttcgaatcccctactatgttggtcctcttgccagaggaaactctcgatttgcttggatgactcgaaagtccgaggaaaccatcactccctggaacttcgaggaagtcgtggacaagggtgcctctgcacagtccttcatcgagcgaatgaccaacttcgacaagaatctgcccaacgagaaggttcttcccaagcattcgctgctctacgagtactttacagtctacaacgaactcaccaaagtcaagtacgttaccgagggaatgcgaaagcctgccttcttgtctggcgaacagaagaaagccattgtcgatctcctgttcaagaccaaccgaaaggtcactgttaagcagctcaaggaggactacttcaagaaaatcgagtgtttcgacagcgtcgagatttccggagttgaggaccgattcaacgcctctttgggcacctatcacgatctgctcaagattatcaaggacaaggattttctcgacaacgaggaaaacgaggacattctggaggacatcgtgctcactcttaccctgttcgaagatcgggagatgatcgaggaacgactcaagacatacgctcacctgttcgacgacaaggtcatgaaacaactcaagcgacgtagatacaccggctggggaagactttcgcgaaagctcatcaacggcatcagagacaagcagtccggaaagaccattctggactttctcaagtccgatggctttgccaaccgaaacttcatgcagctcattcacgacgattctcttaccttcaaggaggacatccagaaggcacaagtgtccggtcagggcgacagcttgcacgaacatattgccaacctggctggttcgccagccatcaagaaaggcattctccagactgtcaaggttgtcgacgagctggtgaaggtcatgggacgtcacaagcccgagaacattgtgatcgagatggccagagagaaccagacaactcaaaagggtcagaaaaactcgcgagagcggatgaagcgaatcgaggaaggcatcaaggagctgggatcccagattctcaaggagcatcccgtcgagaacactcaactgcagaacgagaagctgtatctctactatctgcagaatggtcgagacatgtacgtggatcaggaactggacatcaatcgtctcagcgactacgatgtggaccacattgtccctcaatcctttctcaaggacgattctatcgacaacaaggtccttacacgatccgacaagaacagaggcaagtcggacaacgttcccagcgaagaggtggtcaaaaagatgaagaactactggcgacagctgctcaacgccaagctcattacccagcgaaagttcgacaatcttaccaaggccgagcgaggcggtctgtccgagctcgacaaggctggcttcatcaagcgtcaactcgtcgagaccagacagatcacaaagcacgtcgcacagattctcgattctcggatgaacaccaagtacgacgagaacgacaagctcatccgagaggtcaaggtgattactctcaagtccaaactggtctccgatttccgaaaggactttcagttctacaaggtgcgagagatcaacaattaccaccatgcccacgatgcttacctcaacgccgtcgttggcactgcgctcatcaagaaataccccaagctcgaaagcgagttcgtttacggcgattacaaggtctacgacgttcgaaagatgattgccaagtccgaacaggagattggcaaggctactgccaagtacttcttttactccaacatcatgaactttttcaagaccgagatcaccttggccaacggagagattcgaaagagaccacttatcgagaccaacggcgaaactggagagatcgtgtgggacaagggtcgagactttgcaaccgtgcgaaaggttctgtcgatgcctcaggtcaacatcgtcaagaaaaccgaggttcagactggcggattctccaaggagtcgattctgcccaagcgaaactccgacaagctcatcgctcgaaagaaagactgggatcccaagaaatacggtggcttcgattctcctaccgtcgcctattccgtgcttgtcgttgcgaaggtcgagaagggcaagtccaaaaagctcaagtccgtcaaggagctgctcggaattaccatcatggagcgatcgagcttcgagaagaatcccatcgacttcttggaagccaagggttacaaggaggtcaagaaagacctcattatcaagctgcccaagtactctctgttcgaactggagaacggtcgaaagcgtatgctcgcctccgctggcgagctgcagaagggaaacgagcttgccttgccttcgaagtacgtcaactttctctatctggcttctcactacgagaagctcaagggttctcccgaggacaacgaacagaagcaactcttcgttgagcagcacaaacattacctcgacgagattatcgagcagatttccgagttttcgaagcgagtcatcctggctgatgccaacttggacaaggtgctctctgcctacaacaagcatcgggacaaacccattcgagaacaggcggagaacatcattcacctgtttactcttaccaacctgggtgctcctgcagctttcaagtacttcgataccactatcgaccgaaagcggtacacatccaccaaggaggttctcgatgccaccctgattcaccagtccatcactggcctgtacgagacccgaatcgacctgtctcagcttggtggcgactccagagccgatcccaagaaaaagcgaaaggtctaagcggccgcaagtgtggatggggaagtgagtgcccggttctgtgtgcacaattggcaatccaagatggatggattcaacacagggatatagcgagctacgtggtggtgcgaggatatagcaacggatatttatgtttgacacttgagaatgtacgatacaagcactgtccaagtacaatactaaacatactgtacatactcatactcgtacccgggcaacggtttcacttgagtgcagtggctagtgctcttactcgtacagtgtgcaatactgcgtatcatagtctttgatgtatatcgtattcattcatgttagttgcgtacgagccggaagcataaagtgtaaagcctggggtgcctaatgagtgagctaactcacattaattgcgttgcgctcactgcccgctttccagtcgggaaacctgtcgtgccagctgcattaatgaatcggccaacgcgcggggagaggcggtttgcgtattgggcgctcttccgcttcctcgctcactgactcgctgcgctcggtcgttcggctgcggcgagcggtatcagctcactcaaaggcggtaatacggttatccacagaatcaggggataacgcaggaaagaacatgtgagcaaaaggccagcaaaaggccaggaaccgtaaaaaggccgcgttgctggcgtttttccataggctccgcccccctgacgagcatcacaaaaatcgacgctcaagtcagaggtggcgaaacccgacaggactataaagataccaggcgtttccccctggaagctccctcgtgcgctctcctgttccgaccctgccgcttaccggatacctgtccgcctttctcccttcgggaagcgtggcgctttctcatagctcacgctgtaggtatctcagttcggtgtaggtcgttcgctccaagctgggctgtgtgcacgaaccccccgttcagcccgaccgctgcgccttatccggtaactatcgtcttgagtccaacccggtaagacacgacttatcgccactggcagcagccactggtaacaggattagcagagcgaggtatgtaggcggtgctacagagttcttgaagtggtggcctaactacggctacactagaaggacagtatttggtatctgcgctctgctgaagccagttaccttcggaaaaagagttggtagctcttgatccggcaaacaaaccaccgctggtagcggtggtttttttgtttgcaagcagcagattacgcgcagaaaaaaaggatctcaagaagatcctttgatcttttctacggggtctgacgctcagtggaacgaaaactcacgttaagggattttggtcatgagattatcaaaaaggatcttcacctagatccttttaaattaaaaatgaagttttaaatcaatctaaagtatatatgagtaaacttggtctgacagttaccaatgcttaatcagtgaggcacctatctcagcgatctgtctatttcgttcatccatagttgcctgactccccgtcgtgtagataactacgatacgggagggcttaccatctggccccagtgctgcaatgataccgcgagacccacgctcaccggctccagatttatcagcaataaaccagccagccggaagggccgagcgcagaagtggtcctgcaactttatccgcctccatccagtctattaattgttgccgggaagctagagtaagtagttcgccagttaatagtttgcgcaacgttgttgccattgctacaggcatcgtggtgtcacgctcgtcgtttggtatggcttcattcagctccggttcccaacgatcaaggcgagttacatgatcccccatgttgtgcaaaaaagcggttagctccttcggtcctccgatcgttgtcagaagtaagttggccgcagtgttatcactcatggttatggcagcactgcataattctcttactgtcatgccatccgtaagatgcttttctgtgactggtgagtactcaaccaagtcattctgagaatagtgtatgcggcgaccgagttgctcttgcccggcgtcaatacgggataataccgcgccacatagcagaactttaaaagtgctcatcattggaaaacgttcttcggggcgaaaactctcaaggatcttaccgctgttgagatccagttcgatgtaacccactcgtgcacccaactgatcttcagcatcttttactttcaccagcgtttctgggtgagcaaaaacaggaaggcaaaatgccgcaaaaaagggaataagggcgacacggaaatgttgaatactcatactcttcctttttcaatattattgaagcatttatcagggttattgtctcatgagcggatacatatttgaatgtatttagaaaaataaacaaataggggttccgcgcacatttccccgaaaagtgccacctgacgcgccctgtagcggcgcattaagcgcggcgggtgtggtggttacgcgcagcgtgaccgctacacttgccagcgccctagcgcccgctcctttcgctttcttcccttcctttctcgccacgttcgccggctttccccgtcaagctctaaatcgggggctccctttagggttccgatttagtgctttacggcacctcgaccccaaaaaacttgattagggtgatggttcacgtagtgggccatcgccctgatagacggtttttcgccctttgacgttggagtccacgttctttaatagtggactcttgttccaaactggaacaacactcaaccctatctcggtctattcttttgatttataagggattttgccgatttcggcctattggttaaaaaatgagctgatttaacaaaaatttaacgcgaattttaacaaaatattaacgcttacaatttccattcgccattcaggctgcgcaactgttgggaagggcgatcggtgcgggcctcttcgctattacgccagctggcgaaagggggatgtgctgcaaggcgattaagttgggtaacgccagggttttcccagtcacgacgttgtaaaacgacggccagtgaattgtaatacgactcactatagggcgaattgggtaccgggccccccctcgaggtcgatggtgtcgataagcttgatatcgaattcatgtcacacaaaccgatcttcgcctcaaggaaacctaattctacatccgagagactgccgagatccagtctacactgattaattttcgggccaataatttaaaaaaatcgtgttatataatattatatgtattatatatatacatcatgatgatactgacagtcatgtcccattgctaaatagacagactccatctgccgcctccaactgatgttctcaatatttaaggggtcatctcgcattgtttaataataaacagactccatctaccgcctccaaatgatgttctcaaaatatattgtatgaacttatttttattacttagtattattagacaacttacttgctttatgaaaaacacttcctatttaggaaacaatttataatggcagttcgttcatttaacaatttatgtagaataaatgttataaatgcgtatgggaaatcttaaatatggatagcataaatgatatctgcattgcctaattcgaaatcaacagcaacgaaaaaaatcccttgtacaacataaatagtcatcgagaaatatcaactatcaaagaacagctattcacacgttactattgagattattattggacgagaatcacacactcaactgtctttctctcttctagaaatacaggtacaagtatgtactattctcattgttcatacttctagtcatttcatcccacatattccttggatttctctccaatgaatgacattctatcttgcaaattcaacaattataataagatataccaaagtagcggtatagtggcaatcaaaaagcttctctggtgtgcttctcgtatttatttttattctaatgatccattaaaggtatatatttatttcttgttatataatccttttgtttattacatgggctggatacataaaggtattttgatttaattttttgcttaaattcaatcccccctcgttcagtgtcaactgtaatggtaggaaattaccatacttttgaagaagcaaaaaaaatgaaagaaaaaaaaaatcgtatttccaggttagacgttccgcagaatctagaatgcggtatgcggtacattgttcttcgaacgtaaaagttgcgctccctgagatattgtacatttttgcttttacaagtacaagtacatcgtacaactatgtactactgttgatgcatccacaacagtttgttttgtttttttttgttttttttttttctaatgattcattaccgctatgtatacctacttgtacttgtagtaagccgggttattggcgttcaattaatcatagacttatgaatctgcacggtgtgcgctgcgagttacttttagcttatgcatgctacttgggtgtaatattgggatctgttcggaaatcaacggatgctcaatcgattggaagagatttcgaagcacgttgtttgatactccaatattttgactacttgtatttttgtttgcatgcatactccgaacttaacttgtcgaaaacatggcgacaggcaccgcaagatacagcatgtacatccttctacttgtagctcggtgaagatgaatatgtaaatactaaatatggatatatagataggagggatgtatatactcatcattgagcagttattaagtcattacctgctatatcgccgcatatcccaggttaccacccagagttgtcatcatcttaaccctgctttccctaaactgtaggtgctgagatatcagcctcaactgaacacaactgaatgcgtctgcttgaatcagcctctgaaagacgactgcgcatttaaaaacaatagaactactgcacgtcgcacctcagaaggtaacactctcttcgtggtcactaagcatactgcccaagtgttgttgtcccaaagtatgccacacccacacacacctctgggcacagctgacttccaggatattattacttctgttcataccatctccgttcatgaagtgttacaaaacagttacttatacgagtaataggagctcatgcaataaaacacgactacacccttcaatgaatggagtacacagctatgacactggggttacacttctcaaactacactcaccttgacttcgattcatacaatcgttctttaaattacatacagcagaaaacgagcaaaggcttgcacaacagcaatcaccacacgcggcctcccattcgccatgccgaagcatgttgcccagccggcgccagcgaggaggctgggaccatgccggccaaaagcaccaccgactcggtgccactttttcaagttgataacggactagccttattttaacttgctatttctagctctaaaacgagggtgggtaatcgtttgattgacaaggagagagagaaaagaagaggaaaggtaattcggggacggtggtcttttatacccttggctaaagtcccaaccacaaagcaaaaaaattttcagtagtctattttgcgtccggcatgggttacccggatggccagacaaagaaactagtacaaagtctgaacaagcgtagattccagactgcagtaccctacgcccttaacggcaagtgtgggaaccgggggaggtttgatatgtggggagaagggggctctcgccggggttgggcccgctactgggtcaatttggggtcaattggggcaattggggctgttttttgggacacaaatgcgccgccaacccggtctctttaattaagtcatacacaagtcagctttcttcgagcctcatataagtataagtagttcaacgtattagcactgtacccagcatctccgtatcgagaaacacaacaacatgccccattggacagatcatgcggatacacaggttgtgcagtatcatacatactcgatcagacaggtcgtctgaccatcatacaagctgaacaagcgctccatacttgcacgctctctatatacacagttaaattacatatccatagtctaacctctaacagttaatcttctggtaagcctcccagccagccttctggtatcgcttggcctcctcaataggatctcggttctggccgtacagacctcggccgacaattatgatatccgttccggtagacatgacatcctcaacagttcggtactgctgtccgagagcgtctcccttgtcgtcaagacccaccccgggggtcagaataagccagtcctcagagtcgcccttaggtcggttctgggcaatgaagccaaccacaaactcggggtcggatcgggcaagctcaatggtctgcttggagtactcgccagtggccagagagcccttgcaagacagctcggccagcatgagcagacctctggccagcttctcgttgggagaggggactaggaactccttgtactgggagttctcgtagtcagagacgtcctccttcttctgttcagagacagtttcctcggcaccagctcgcaggccagcaatgattccggttccgggtacaccgtgggcgttggtgatatcggaccactcggcgattcggtgacaccggtactggtgcttgacagtgttgccaatatctgcgaactttctgtcctcgaacaggaagaaaccgtgcttaagagcaagttccttgagggggagcacagtgccggcgtaggtgaagtcgtcaatgatgtcgatatgggttttgatcatgcacacataaggtccgaccttatcggcaagctcaatgagctccttggtggtggtaacatccagagaagcacacaggttggttttcttggctgccacgagcttgagcactcgagcggcaaaggcggacttgtggacgttagctcgagcttcgtaggagggcattttggtggtgaagaggagactgaaataaatttagtctgcagaactttttatcggaaccttatctggggcagtgaagtatatgttatggtaatagttacgagttagttgaacttatagatagactggactatacggctatcggtccaaattagaaagaacgtcaatggctctctgggcgtcgcctttgccgacaaaaatgtgatcatgatgaaagccagcaatgacgttgcagctgatattgttgtcggccaaccgcgccgaaaacgcagctgtcagacccacagcctccaacgaagaatgtatcgtcaaagtgatccaagcacactcatagttggagtcgtactccaaaggcggcaatgacgagtcagacagatactcgtcgacgtttaaaccatcatctaagggcctcaaaactacctcggaactgctgcgctgatctggacaccacagaggttccgagcactttaggttgcaccaaatgtcccaccaggtgcaggcagaaaacgctggaacagcgtgtacagtttgtcttaacaaaaagtgagggcgctgaggtcgagcagggtggtgtgacttgttatagcctttagagctgcgaaagcgcgtatggatttggctcatcaggccagattgagggtctgtggacacatgtcatgttagtgtacttcaatcgccccctggatatagccccgacaataggccgtggcctcatttttttgccttccgcacatttccattgctcggtacccacaccttgcttctcctgcacttgccaaccttaatactggtttacattgaccaacatcttacaagcggggggcttgtctagggtatatataaacagtggctctcccaatcggttgccagtctcttttttcctttctttccccacagattcgaaatctaaactacacatcacac

SEQ ID NO: 67 - DNA, 11993 bp, Artificial sequence; identical to SEQ ID NO: 66
  pRF623

SEQ ID NO: 68 - DNA, 12045 bp, artificial sequence
  pRF621
catggacaagaaatactccatcggcctggacattggaaccaactctgtcggctgggctgtcatcaccgacgagtacaaggtgccctccaagaaattcaaggtcctcggaaacaccgatcgacactccatcaagaaaaacctcattggtgccctgttgttcgattctggcgagactgccgaagctaccagactcaagcgaactgctcggcgacgttacacccgacggaagaaccgaatctgctacctgcaggagatcttttccaacgagatggccaaggtggacgattcgttctttcatcgactggaggaatccttcctcgtcgaggaagacaagaaacacgagcgtcatcccatctttggcaacattgtggacgaggttgcttaccacgagaagtatcctaccatctaccacctgcgaaagaaactcgtcgattccaccgacaaggcggatctcagacttatctacctcgctctggcacacatgatcaagtttcgaggtcatttcctcatcgagggcgatctcaatcccgacaacagcgatgtggacaagctgttcattcagctcgttcagacctacaaccagctgttcgaggaaaaccccatcaatgcctccggagtcgatgcaaaggccatcttgtctgctcgactctcgaagagcagacgactggagaacctcattgcccaacttcctggcgagaaaaagaacggactgtttggcaacctcattgccctttctcttggtctcacacccaacttcaagtccaacttcgatctggcggaggacgccaagctccagctgtccaaggacacctacgacgatgacctcgacaacctgcttgcacagattggcgatcagtacgccgacctgtttctcgctgccaagaacctttcggatgctattctcttgtctgacattctgcgagtcaacaccgagatcacaaaggctcccctttctgcctccatgatcaagcgatacgacgagcaccatcaggatctcacactgctcaaggctcttgtccgacagcaactgcccgagaagtacaaggagatctttttcgatcagtcgaagaacggctacgctggatacatcgacggcggagcctctcaggaagagttctacaagttcatcaagccaattctcgagaagatggacggaaccgaggaactgcttgtcaagctcaatcgagaggatctgcttcggaagcaacgaaccttcgacaacggcagcattcctcatcagatccacctcggtgagctgcacgccattcttcgacgtcaggaagacttctacccctttctcaaggacaaccgagagaagatcgagaagattcttacctttcgaatcccctactatgttggtcctcttgccagaggaaactctcgatttgcttggatgactcgaaagtccgaggaaaccatcactccctggaacttcgaggaagtcgtggacaagggtgcctctgcacagtccttcatcgagcgaatgaccaacttcgacaagaatctgcccaacgagaaggttcttcccaagcattcgctgctctacgagtactttacagtctacaacgaactcaccaaagtcaagtacgttaccgagggaatgcgaaagcctgccttcttgtctggcgaacagaagaaagccattgtcgatctcctgttcaagaccaaccgaaaggtcactgttaagcagctcaaggaggactacttcaagaaaatcgagtgtttcgacagcgtcgagatttccggagttgaggaccgattcaacgcctctttgggcacctatcacgatctgctcaagattatcaaggacaaggattttctcgacaacgaggaaaacgaggacattctggaggacatcgtgctcactcttaccctgttcgaagatcgggagatgatcgaggaacgactcaagacatacgctcacctgttcgacgacaaggtcatgaaacaactcaagcgacgtagatacaccggctggggaagactttcgcgaaagctcatcaacggcatcagagacaagcagtccggaaagaccattctggactttctcaagtccgatggctttgccaaccgaaacttcatgcagctcattcacgacgattctcttaccttcaaggaggacatccagaaggcacaagtgtccggtcagggcgacagcttgcacgaacatattgccaacctggctggttcgccagccatcaagaaaggcattctccagactgtcaaggttgtcgacgagctggtgaaggtcatgggacgtcacaagcccgagaacattgtgatcgagatggccagagagaaccagacaactcaaaagggtcagaaaaactcgcgagagcggatgaagcgaatcgaggaaggcatcaaggagctgggatcccagattctcaaggagcatcccgtcgagaacactcaactgcagaacgagaagctgtatctctactatctgcagaatggtcgagacatgtacgtggatcaggaactggacatcaatcgtctcagcgactacgatgtggaccacattgtccctcaatcctttctcaaggacgattctatcgacaacaaggtccttacacgatccgacaagaacagaggcaagtcggacaacgttcccagcgaagaggtggtcaaaaagatgaagaactactggcgacagctgctcaacgccaagctcattacccagcgaaagttcgacaatcttaccaaggccgagcgaggcggtctgtccgagctcgacaaggctggcttcatcaagcgtcaactcgtcgagaccagacagatcacaaagcacgtcgcacagattctcgattctcggatgaacaccaagtacgacgagaacgacaagctcatccgagaggtcaaggtgattactctcaagtccaaactggtctccgatttccgaaaggactttcagttctacaaggtgcgagagatcaacaattaccaccatgcccacgatgcttacctcaacgccgtcgttggcactgcgctcatcaagaaataccccaagctcgaaagcgagttcgtttacggcgattacaaggtctacgacgttcgaaagatgattgccaagtccgaacaggagattggcaaggctactgccaagtacttcttttactccaacatcatgaactttttcaagaccgagatcaccttggccaacggagagattcgaaagagaccacttatcgagaccaacggcgaaactggagagatcgtgtgggacaagggtcgagactttgcaaccgtgcgaaaggttctgtcgatgcctcaggtcaacatcgtcaagaaaaccgaggttcagactggcggattctccaaggagtcgattctgcccaagcgaaactccgacaagctcatcgctcgaaagaaagactgggatcccaagaaatacggtggcttcgattctcctaccgtcgcctattccgtgcttgtcgttgcgaaggtcgagaagggcaagtccaaaaagctcaagtccgtcaaggagctgctcggaattaccatcatggagcgatcgagcttcgagaagaatcccatcgacttcttggaagccaagggttacaaggaggtcaagaaagacctcattatcaagctgcccaagtactctctgttcgaactggagaacggtcgaaagcgtatgctcgcctccgctggcgagctgcagaagggaaacgagcttgccttgccttcgaagtacgtcaactttctctatctggcttctcactacgagaagctcaagggttctcccgaggacaacgaacagaagcaactcttcgttgagcagcacaaacattacctcgacgagattatcgagcagatttccgagttttcgaagcgagtcatcctggctgatgccaacttggacaaggtgctctctgcctacaacaagcatcgggacaaacccattcgagaacaggcggagaacatcattcacctgtttactcttaccaacctgggtgctcctgcagctttcaagtacttcgataccactatcgaccgaaagcggtacacatccaccaaggaggttctcgatgccaccctgattcaccagtccatcactggcctgtacgagacccgaatcgacctgtctcagcttggtggcgactccagagccgatcccaagaaaaagcgaaaggtctaagcggccgcaagtgtggatggggaagtgagtgcccggttctgtgtgcacaattggcaatccaagatggatggattcaacacagggatatagcgagctacgtggtggtgcgaggatatagcaacggatatttatgtttgacacttgagaatgtacgatacaagcactgtccaagtacaatactaaacatactgtacatactcatactcgtacccgggcaacggtttcacttgagtgcagtggctagtgctcttactcgtacagtgtgcaatactgcgtatcatagtctttgatgtatatcgtattcattcatgttagttgcgtacgagccggaagcataaagtgtaaagcctggggtgcctaatgagtgagctaactcacattaattgcgttgcgctcactgcccgctttccagtcgggaaacctgtcgtgccagctgcattaatgaatcggccaacgcgcggggagaggcggtttgcgtattgggcgctcttccgcttcctcgctcactgactcgctgcgctcggtcgttcggctgcggcgagcggtatcagctcactcaaaggcggtaatacggttatccacagaatcaggggataacgcaggaaagaacatgtgagcaaaaggccagcaaaaggccaggaaccgtaaaaaggccgcgttgctggcgtttttccataggctccgcccccctgacgagcatcacaaaaatcgacgctcaagtcagaggtggcgaaacccgacaggactataaagataccaggcgtttccccctggaagctccctcgtgcgctctcctgttccgaccctgccgcttaccggatacctgtccgcctttctcccttcgggaagcgtggcgctttctcatagctcacgctgtaggtatctcagttcggtgtaggtcgttcgctccaagctgggctgtgtgcacgaaccccccgttcagcccgaccgctgcgccttatccggtaactatcgtcttgagtccaacccggtaagacacgacttatcgccactggcagcagccactggtaacaggattagcagagcgaggtatgtaggcggtgctacagagttcttgaagtggtggcctaactacggctacactagaaggacagtatttggtatctgcgctctgctgaagccagttaccttcggaaaaagagttggtagctcttgatccggcaaacaaaccaccgctggtagcggtggtttttttgtttgcaagcagcagattacgcgcagaaaaaaaggatctcaagaagatcctttgatcttttctacggggtctgacgctcagtggaacgaaaactcacgttaagggattttggtcatgagattatcaaaaaggatcttcacctagatccttttaaattaaaaatgaagttttaaatcaatctaaagtatatatgagtaaacttggtctgacagttaccaatgcttaatcagtgaggcacctatctcagcgatctgtctatttcgttcatccatagttgcctgactccccgtcgtgtagataactacgatacgggagggcttaccatctggccccagtgctgcaatgataccgcgagacccacgctcaccggctccagatttatcagcaataaaccagccagccggaagggccgagcgcagaagtggtcctgcaactttatccgcctccatccagtctattaattgttgccgggaagctagagtaagtagttcgccagttaatagtttgcgcaacgttgttgccattgctacaggcatcgtggtgtcacgctcgtcgtttggtatggcttcattcagctccggttcccaacgatcaaggcgagttacatgatcccccatgttgtgcaaaaaagcggttagctccttcggtcctccgatcgttgtcagaagtaagttggccgcagtgttatcactcatggttatggcagcactgcataattctcttactgtcatgccatccgtaagatgcttttctgtgactggtgagtactcaaccaagtcattctgagaatagtgtatgcggcgaccgagttgctcttgcccggcgtcaatacgggataataccgcgccacatagcagaactttaaaagtgctcatcattggaaaacgttcttcggggcgaaaactctcaaggatcttaccgctgttgagatccagttcgatgtaacccactcgtgcacccaactgatcttcagcatcttttactttcaccagcgtttctgggtgagcaaaaacaggaaggcaaaatgccgcaaaaaagggaataagggcgacacggaaatgttgaatactcatactcttcctttttcaatattattgaagcatttatcagggttattgtctcatgagcggatacatatttgaatgtatttagaaaaataaacaaataggggttccgcgcacatttccccgaaaagtgccacctgacgcgccctgtagcggcgcattaagcgcggcgggtgtggtggttacgcgcagcgtgaccgctacacttgccagcgccctagcgcccgctcctttcgctttcttcccttcctttctcgccacgttcgccggctttccccgtcaagctctaaatcgggggctccctttagggttccgatttagtgctttacggcacctcgaccccaaaaaacttgattagggtgatggttcacgtagtgggccatcgccctgatagacggtttttcgccctttgacgttggagtccacgttctttaatagtggactcttgttccaaactggaacaacactcaaccctatctcggtctattcttttgatttataagggattttgccgatttcggcctattggttaaaaaatgagctgatttaacaaaaatttaacgcgaattttaacaaaatattaacgcttacaatttccattcgccattcaggctgcgcaactgttgggaagggcgatcggtgcgggcctcttcgctattacgccagctggcgaaagggggatgtgctgcaaggcgattaagttgggtaacgccagggttttcccagtcacgacgttgtaaaacgacggccagtgaattgtaatacgactcactatagggcgaattgggtaccgggccccccctcgaggtcgatggtgtcgataagcttgatatcgaattcatgtcacacaaaccgatcttcgcctcaaggaaacctaattctacatccgagagactgccgagatccagtctacactgattaattttcgggccaataatttaaaaaaatcgtgttatataatattatatgtattatatatatacatcatgatgatactgacagtcatgtcccattgctaaatagacagactccatctgccgcctccaactgatgttctcaatatttaaggggtcatctcgcattgtttaataataaacagactccatctaccgcctccaaatgatgttctcaaaatatattgtatgaacttatttttattacttagtattattagacaacttacttgctttatgaaaaacacttcctatttaggaaacaatttataatggcagttcgttcatttaacaatttatgtagaataaatgttataaatgcgtatgggaaatcttaaatatggatagcataaatgatatctgcattgcctaattcgaaatcaacagcaacgaaaaaaatcccttgtacaacataaatagtcatcgagaaatatcaactatcaaagaacagctattcacacgttactattgagattattattggacgagaatcacacactcaactgtctttctctcttctagaaatacaggtacaagtatgtactattctcattgttcatacttctagtcatttcatcccacatattccttggatttctctccaatgaatgacattctatcttgcaaattcaacaattataataagatataccaaagtagcggtatagtggcaatcaaaaagcttctctggtgtgcttctcgtatttatttttattctaatgatccattaaaggtatatatttatttcttgttatataatccttttgtttattacatgggctggatacataaaggtattttgatttaattttttgcttaaattcaatcccccctcgttcagtgtcaactgtaatggtaggaaattaccatacttttgaagaagcaaaaaaaatgaaagaaaaaaaaaatcgtatttccaggttagacgttccgcagaatctagaatgcggtatgcggtacattgttcttcgaacgtaaaagttgcgctccctgagatattgtacatttttgcttttacaagtacaagtacatcgtacaactatgtactactgttgatgcatccacaacagtttgttttgtttttttttgttttttttttttctaatgattcattaccgctatgtatacctacttgtacttgtagtaagccgggttattggcgttcaattaatcatagacttatgaatctgcacggtgtgcgctgcgagttacttttagcttatgcatgctacttgggtgtaatattgggatctgttcggaaatcaacggatgctcaatcgattggaagagatttcgaagcacgttgtttgatactccaatattttgactacttgtatttttgtttgcatgcatactccgaacttaacttgtcgaaaacatggcgacaggcaccgcaagatacagcatgtacatccttctacttgtagctcggtgaagatgaatatgtaaatactaaatatggatatatagataggagggatgtatatactcatcattgagcagttattaagtcattacctgctatatcgccgcatatcccaggttaccacccagagttgtcatcatcttaaccctgctttccctaaactgtaggtgctgagatatcagcctcaactgaacacaactgaatgcgtctgcttgaatcagcctctgaaagacgactgcgcatttaaaaacaatagaactactgcacgtcgcacctcagaaggtaacactctcttcgtggtcactaagcatactgcccaagtgttgttgtcccaaagtatgccacacccacacacacctctgggcacagctgacttccaggatattattacttctgttcataccatctccgttcatgaagtgttacaaaacagttacttatacgagtaataggagctcatgcaataaaacacgactacacccttcaatgaatggagtacacagctatgacactggggttacacttctcaaactacactcaccttgacttcgattcatacaatcgttctttaaattacatacagcagaaaacgagcaaaggcttgcacaacagcaatcaccacacgcggcctcccattcgccatgccgaagcatgttgcccagccggcgccagcgaggaggctgggaccatgccggccaaaagcaccaccgactcggtgccactttttcaagttgataacggactagccttattttaacttgctatttctagctctaaaacgagggtgggtaatcgtttgatttgaatgattcttatactcagaaggaaatgcttaacgatttcgggtgtgagttgacaaggagagagagaaaagaagaggaaaggtaattcggggacggtggtcttttatacccttggctaaagtcccaaccacaaagcaaaaaaattttcagtagtctattttgcgtccggcatgggttacccggatggccagacaaagaaactagtacaaagtctgaacaagcgtagattccagactgcagtaccctacgcccttaacggcaagtgtgggaaccgggggaggtttgatatgtggggagaagggggctctcgccggggttgggcccgctactgggtcaatttggggtcaattggggcaattggggctgttttttgggacacaaatgcgccgccaacccggtctctttaattaagtcatacacaagtcagctttcttcgagcctcatataagtataagtagttcaacgtattagcactgtacccagcatctccgtatcgagaaacacaacaacatgccccattggacagatcatgcggatacacaggttgtgcagtatcatacatactcgatcagacaggtcgtctgaccatcatacaagctgaacaagcgctccatacttgcacgctctctatatacacagttaaattacatatccatagtctaacctctaacagttaatcttctggtaagcctcccagccagccttctggtatcgcttggcctcctcaataggatctcggttctggccgtacagacctcggccgacaattatgatatccgttccggtagacatgacatcctcaacagttcggtactgctgtccgagagcgtctcccttgtcgtcaagacccaccccgggggtcagaataagccagtcctcagagtcgcccttaggtcggttctgggcaatgaagccaaccacaaactcggggtcggatcgggcaagctcaatggtctgcttggagtactcgccagtggccagagagcccttgcaagacagctcggccagcatgagcagacctctggccagcttctcgttgggagaggggactaggaactccttgtactgggagttctcgtagtcagagacgtcctccttcttctgttcagagacagtttcctcggcaccagctcgcaggccagcaatgattccggttccgggtacaccgtgggcgttggtgatatcggaccactcggcgattcggtgacaccggtactggtgcttgacagtgttgccaatatctgcgaactttctgtcctcgaacaggaagaaaccgtgcttaagagcaagttccttgagggggagcacagtgccggcgtaggtgaagtcgtcaatgatgtcgatatgggttttgatcatgcacacataaggtccgaccttatcggcaagctcaatgagctccttggtggtggtaacatccagagaagcacacaggttggttttcttggctgccacgagcttgagcactcgagcggcaaaggcggacttgtggacgttagctcgagcttcgtaggagggcattttggtggtgaagaggagactgaaataaatttagtctgcagaactttttatcggaaccttatctggggcagtgaagtatatgttatggtaatagttacgagttagttgaacttatagatagactggactatacggctatcggtccaaattagaaagaacgtcaatggctctctgggcgtcgcctttgccgacaaaaatgtgatcatgatgaaagccagcaatgacgttgcagctgatattgttgtcggccaaccgcgccgaaaacgcagctgtcagacccacagcctccaacgaagaatgtatcgtcaaagtgatccaagcacactcatagttggagtcgtactccaaaggcggcaatgacgagtcagacagatactcgtcgacgtttaaaccatcatctaagggcctcaaaactacctcggaactgctgcgctgatctggacaccacagaggttccgagcactttaggttgcaccaaatgtcccaccaggtgcaggcagaaaacgctggaacagcgtgtacagtttgtcttaacaaaaagtgagggcgctgaggtcgagcagggtggtgtgacttgttatagcctttagagctgcgaaagcgcgtatggatttggctcatcaggccagattgagggtctgtggacacatgtcatgttagtgtacttcaatcgccccctggatatagccccgacaataggccgtggcctcatttttttgccttccgcacatttccattgctcggtacccacaccttgcttctcctgcacttgccaaccttaatactggtttacattgaccaacatcttacaagcggggggcttgtctagggtatatataaacagtggctctcccaatcggttgccagtctcttttttcctttctttccccacagattcgaaatctaaactacacatcacac

SEQ ID NO: 69 - DNA, 23 bp, Yarrowia lipolytica
tcaaacgattacccaccctccgg

SEQ ID NO: 70 - DNA, 11176 bp, Artificial Sequence
  pRF303
tctaaaacgagggtgggtaatcgtttgagtcccattcgccatgccgaagcatgttgcccagccggcgccagcgaggaggctgggaccatgccggccattattttgcgttaagtttctaatcatcacgaaattatctatcaaaaataactaggtcccaccgagattcgaactcgggaccttaagatttgcaatctcacgcgctaccgctgtgccataggaccgaagttaaaatttggccaaagaaggacctgggcaccctggactgtgggttagggtaatattccttatggagacaatgggctagggtaaattacctaaaatgggtcgataaagaggggtgttcccagttgggaagtgtaattgaagacggggtcaaaaaagaaaatcaaaaaaaatttaattaagtcatacacaagtcagctttcttcgagcctcatataagtataagtagttcaacgtattagcactgtacccagcatctccgtatcgagaaacacaacaacatgccccattggacagatcatgcggatacacaggttgtgcagtatcatacatactcgatcagacaggtcgtctgaccatcatacaagctgaacaagcgctccatacttgcacgctctctatatacacagttaaattacatatccatagtctaacctctaacagttaatcttctggtaagcctcccagccagccttctggtatcgcttggcctcctcaataggatctcggttctggccgtacagacctcggccgacaattatgatatccgttccggtagacatgacatcctcaacagttcggtactgctgtccgagagcgtctcccttgtcgtcaagacccaccccgggggtcagaataagccagtcctcagagtcgcccttaggtcggttctgggcaatgaagccaaccacaaactcggggtcggatcgggcaagctcaatggtctgcttggagtactcgccagtggccagagagcccttgcaagacagctcggccagcatgagcagacctctggccagcttctcgttgggagaggggactaggaactccttgtactgggagttctcgtagtcagagacgtcctccttcttctgttcagagacagtttcctcggcaccagctcgcaggccagcaatgattccggttccgggtacaccgtgggcgttggtgatatcggaccactcggcgattcggtgacaccggtactggtgcttgacagtgttgccaatatctgcgaactttctgtcctcgaacaggaagaaaccgtgcttaagagcaagttccttgagggggagcacagtgccggcgtaggtgaagtcgtcaatgatgtcgatatgggttttgatcatgcacacataaggtccgaccttatcggcaagctcaatgagctccttggtggtggtaacatccagagaagcacacaggttggttttcttggctgccacgagcttgagcactcgagcggcaaaggcggacttgtggacgttagctcgagcttcgtaggagggcattttggtggtgaagaggagactgaaataaatttagtctgcagaactttttatcggaaccttatctggggcagtgaagtatatgttatggtaatagttacgagttagttgaacttatagatagactggactatacggctatcggtccaaattagaaagaacgtcaatggctctctgggcgtcgcctttgccgacaaaaatgtgatcatgatgaaagccagcaatgacgttgcagctgatattgttgtcggccaaccgcgccgaaaacgcagctgtcagacccacagcctccaacgaagaatgtatcgtcaaagtgatccaagcacactcatagttggagtcgtactccaaaggcggcaatgacgagtcagacagatactcgtcgacgtttaaaccatcatctaagggcctcaaaactacctcggaactgctgcgctgatctggacaccacagaggttccgagcactttaggttgcaccaaatgtcccaccaggtgcaggcagaaaacgctggaacagcgtgtacagtttgtcttaacaaaaagtgagggcgctgaggtcgagcagggtggtgtgacttgttatagcctttagagctgcgaaagcgcgtatggatttggctcatcaggccagattgagggtctgtggacacatgtcatgttagtgtacttcaatcgccccctggatatagccccgacaataggccgtggcctcatttttttgccttccgcacatttccattgctcggtacccacaccttgcttctcctgcacttgccaaccttaatactggtttacattgaccaacatcttacaagcggggggcttgtctagggtatatataaacagtggctctcccaatcggttgccagtctcttttttcctttctttccccacagattcgaaatctaaactacacatcacaccatggacaagaaatactccatcggcctggacattggaaccaactctgtcggctgggctgtcatcaccgacgagtacaaggtgccctccaagaaattcaaggtcctcggaaacaccgatcgacactccatcaagaaaaacctcattggtgccctgttgttcgattctggcgagactgccgaagctaccagactcaagcgaactgctcggcgacgttacacccgacggaagaaccgaatctgctacctgcaggagatcttttccaacgagatggccaaggtggacgattcgttctttcatcgactggaggaatccttcctcgtcgaggaagacaagaaacacgagcgtcatcccatctttggcaacattgtggacgaggttgcttaccacgagaagtatcctaccatctaccatctccgaaagaaactcgtcgattccaccgacaaggcggatctcagacttatctacctcgctctggcacacatgatcaagtttcgaggtcatttcctcatcgagggcgatctcaatcccgacaacagcgatgtggacaagctgttcattcagctcgttcagacctacaaccagctgttcgaggaaaaccccatcaatgcctccggagtcgatgcaaaggccatcttgtctgctcgactctcgaagagcagacgactggagaacctcattgcccaacttcctggcgagaaaaagaacggactgtttggcaacctcattgccctttctcttggtctcacacccaacttcaagtccaacttcgatctggcggaggacgccaagctccagctgtccaaggacacctacgacgatgacctcgacaacctgcttgcacagattggcgatcagtacgccgacctgtttctcgctgccaagaacctttcggatgctattctcttgtctgacattctgcgagtcaacaccgagatcacaaaggctcccctttctgcctccatgatcaagcgatacgacgagcaccatcaggatctcacactgctcaaggctcttgtccgacagcaactgcccgagaagtacaaggagatctttttcgatcagtcgaagaacggctacgctggatacatcgacggcggagcctctcaggaagagttctacaagttcatcaagccaattctcgagaagatggacggaaccgaggaactgcttgtcaagctcaatcgagaggatctgcttcggaagcaacgaaccttcgacaacggcagcattcctcatcagatccacctcggtgagctgcacgccattcttcgacgtcaggaagacttctacccctttctcaaggacaaccgagagaagatcgagaagattcttacctttcgaatcccctactatgttggtcctcttgccagaggaaactctcgatttgcttggatgactcgaaagtccgaggaaaccatcactccctggaacttcgaggaagtcgtggacaagggtgcctctgcacagtccttcatcgagcgaatgaccaacttcgacaagaatctgcccaacgagaaggttcttcccaagcattcgctgctctacgagtactttacagtctacaacgaactcaccaaagtcaagtacgttaccgagggaatgcgaaagcctgccttcttgtctggcgaacagaagaaagccattgtcgatctcctgttcaagaccaaccgaaaggtcactgttaagcagctcaaggaggactacttcaagaaaatcgagtgtttcgacagcgtcgagatttccggagttgaggaccgattcaacgcctctttgggcacctatcacgatctgctcaagattatcaaggacaaggattttctcgacaacgaggaaaacgaggacattctggaggacatcgtgctcactcttaccctgttcgaagatcgggagatgatcgaggaacgactcaagacatacgctcacctgttcgacgacaaggtcatgaaacaactcaagcgacgtagatacaccggctggggaagactttcgcgaaagctcatcaacggcatcagagacaagcagtccggaaagaccattctggactttctcaagtccgatggctttgccaaccgaaacttcatgcagctcattcacgacgattctcttaccttcaaggaggacatccagaaggcacaagtgtccggtcagggcgacagcttgcacgaacatattgccaacctggctggttcgccagccatcaagaaaggcattctccagactgtcaaggttgtcgacgagctggtgaaggtcatgggacgtcacaagcccgagaacattgtgatcgagatggccagagagaaccagacaactcaaaagggtcagaaaaactcgcgagagcggatgaagcgaatcgaggaaggcatcaaggagctgggatcccagattctcaaggagcatcccgtcgagaacactcaactgcagaacgagaagctgtatctctactatctgcagaatggtcgagacatgtacgtggatcaggaactggacatcaatcgtctcagcgactacgatgtggaccacattgtccctcaatcctttctcaaggacgattctatcgacaacaaggtccttacacgatccgacaagaacagaggcaagtcggacaacgttcccagcgaagaggtggtcaaaaagatgaagaactactggcgacagctgctcaacgccaagctcattacccagcgaaagttcgacaatcttaccaaggccgagcgaggcggtctgtccgagctcgacaaggctggcttcatcaagcgtcaactcgtcgagaccagacagatcacaaagcacgtcgcacagattctcgattctcggatgaacaccaagtacgacgagaacgacaagctcatccgagaggtcaaggtgattactctcaagtccaaactggtctccgatttccgaaaggactttcagttctacaaggtgcgagagatcaacaattaccaccatgcccacgatgcttacctcaacgccgtcgttggcactgcgctcatcaagaaataccccaagctcgaaagcgagttcgtttacggcgattacaaggtctacgacgttcgaaagatgattgccaagtccgaacaggagattggcaaggctactgccaagtacttcttttactccaacatcatgaactttttcaagaccgagatcaccttggccaacggagagattcgaaagagaccacttatcgagaccaacggcgaaactggagagatcgtgtgggacaagggtcgagactttgcaaccgtgcgaaaggttctgtcgatgcctcaggtcaacatcgtcaagaaaaccgaggttcagactggcggattctccaaggagtcgattctgcccaagcgaaactccgacaagctcatcgctcgaaagaaagactgggatcccaagaaatacggtggcttcgattctcctaccgtcgcctattccgtgcttgtcgttgcgaaggtcgagaagggcaagtccaaaaagctcaagtccgtcaaggagctgctcggaattaccatcatggagcgatcgagcttcgagaagaatcccatcgacttcttggaagccaagggttacaaggaggtcaagaaagacctcattatcaagctgcccaagtactctctgttcgaactggagaacggtcgaaagcgtatgctcgcctccgctggcgagctgcagaagggaaacgagcttgccttgccttcgaagtacgtcaactttctctatctggcttctcactacgagaagctcaagggttctcccgaggacaacgaacagaagcaactcttcgttgagcagcacaaacattacctcgacgagattatcgagcagatttccgagttttcgaagcgagtcatcctggctgatgccaacttggacaaggtgctctctgcctacaacaagcatcgggacaaacccattcgagaacaggcggagaacatcattcacctgtttactcttaccaacctgggtgctcctgcagctttcaagtacttcgataccactatcgaccgaaagcggtacacatccaccaaggaggttctcgatgccaccctgattcaccagtccatcactggcctgtacgagacccgaatcgacctgtctcagcttggtggcgactccagagccgatcccaagaaaaagcgaaaggtctaagcggccgcaagtgtggatggggaagtgagtgcccggttctgtgtgcacaattggcaatccaagatggatggattcaacacagggatatagcgagctacgtggtggtgcgaggatatagcaacggatatttatgtttgacacttgagaatgtacgatacaagcactgtccaagtacaatactaaacatactgtacatactcatactcgtacccgggcaacggtttcacttgagtgcagtggctagtgctcttactcgtacagtgtgcaatactgcgtatcatagtctttgatgtatatcgtattcattcatgttagttgcgtacgagccggaagcataaagtgtaaagcctggggtgcctaatgagtgagctaactcacattaattgcgttgcgctcactgcccgctttccagtcgggaaacctgtcgtgccagctgcattaatgaatcggccaacgcgcggggagaggcggtttgcgtattgggcgctcttccgcttcctcgctcactgactcgctgcgctcggtcgttcggctgcggcgagcggtatcagctcactcaaaggcggtaatacggttatccacagaatcaggggataacgcaggaaagaacatgtgagcaaaaggccagcaaaaggccaggaaccgtaaaaaggccgcgttgctggcgtttttccataggctccgcccccctgacgagcatcacaaaaatcgacgctcaagtcagaggtggcgaaacccgacaggactataaagataccaggcgtttccccctggaagctccctcgtgcgctctcctgttccgaccctgccgcttaccggatacctgtccgcctttctcccttcgggaagcgtggcgctttctcatagctcacgctgtaggtatctcagttcggtgtaggtcgttcgctccaagctgggctgtgtgcacgaaccccccgttcagcccgaccgctgcgccttatccggtaactatcgtcttgagtccaacccggtaagacacgacttatcgccactggcagcagccactggtaacaggattagcagagcgaggtatgtaggcggtgctacagagttcttgaagtggtggcctaactacggctacactagaaggacagtatttggtatctgcgctctgctgaagccagttaccttcggaaaaagagttggtagctcttgatccggcaaacaaaccaccgctggtagcggtggtttttttgtttgcaagcagcagattacgcgcagaaaaaaaggatctcaagaagatcctttgatcttttctacggggtctgacgctcagtggaacgaaaactcacgttaagggattttggtcatgagattatcaaaaaggatcttcacctagatccttttaaattaaaaatgaagttttaaatcaatctaaagtatatatgagtaaacttggtctgacagttaccaatgcttaatcagtgaggcacctatctcagcgatctgtctatttcgttcatccatagttgcctgactccccgtcgtgtagataactacgatacgggagggcttaccatctggccccagtgctgcaatgataccgcgagacccacgctcaccggctccagatttatcagcaataaaccagccagccggaagggccgagcgcagaagtggtcctgcaactttatccgcctccatccagtctattaattgttgccgggaagctagagtaagtagttcgccagttaatagtttgcgcaacgttgttgccattgctacaggcatcgtggtgtcacgctcgtcgtttggtatggcttcattcagctccggttcccaacgatcaaggcgagttacatgatcccccatgttgtgcaaaaaagcggttagctccttcggtcctccgatcgttgtcagaagtaagttggccgcagtgttatcactcatggttatggcagcactgcataattctcttactgtcatgccatccgtaagatgcttttctgtgactggtgagtactcaaccaagtcattctgagaatagtgtatgcggcgaccgagttgctcttgcccggcgtcaatacgggataataccgcgccacatagcagaactttaaaagtgctcatcattggaaaacgttcttcggggcgaaaactctcaaggatcttaccgctgttgagatccagttcgatgtaacccactcgtgcacccaactgatcttcagcatcttttactttcaccagcgtttctgggtgagcaaaaacaggaaggcaaaatgccgcaaaaaagggaataagggcgacacggaaatgttgaatactcatactcttcctttttcaatattattgaagcatttatcagggttattgtctcatgagcggatacatatttgaatgtatttagaaaaataaacaaataggggttccgcgcacatttccccgaaaagtgccacctgacgcgccctgtagcggcgcattaagcgcggcgggtgtggtggttacgcgcagcgtgaccgctacacttgccagcgccctagcgcccgctcctttcgctttcttcccttcctttctcgccacgttcgccggctttccccgtcaagctctaaatcgggggctccctttagggttccgatttagtgctttacggcacctcgaccccaaaaaacttgattagggtgatggttcacgtagtgggccatcgccctgatagacggtttttcgccctttgacgttggagtccacgttctttaatagtggactcttgttccaaactggaacaacactcaaccctatctcggtctattcttttgatttataagggattttgccgatttcggcctattggttaaaaaatgagctgatttaacaaaaatttaacgcgaattttaacaaaatattaacgcttacaatttccattcgccattcaggctgcgcaactgttgggaagggcgatcggtgcgggcctcttcgctattacgccagctggcgaaagggggatgtgctgcaaggcgattaagttgggtaacgccagggttttcccagtcacgacgttgtaaaacgacggccagtgaattgtaatacgactcactatagggcgaattgggtaccgggccccccctcgaggtcgatggtgtcgataagcttgatatcgaattcatgtcacacaaaccgatcttcgcctcaaggaaacctaattctacatccgagagactgccgagatccagtctacactgattaattttcgggccaataatttaaaaaaatcgtgttatataatattatatgtattatatatatacatcatgatgatactgacagtcatgtcccattgctaaatagacagactccatctgccgcctccaactgatgttctcaatatttaaggggtcatctcgcattgtttaataataaacagactccatctaccgcctccaaatgatgttctcaaaatatattgtatgaacttatttttattacttagtattattagacaacttacttgctttatgaaaaacacttcctatttaggaaacaatttataatggcagttcgttcatttaacaatttatgtagaataaatgttataaatgcgtatgggaaatcttaaatatggatagcataaatgatatctgcattgcctaattcgaaatcaacagcaacgaaaaaaatcccttgtacaacataaatagtcatcgagaaatatcaactatcaaagaacagctattcacacgttactattgagattattattggacgagaatcacacactcaactgtctttctctcttctagaaatacaggtacaagtatgtactattctcattgttcatacttctagtcatttcatcccacatattccttggatttctctccaatgaatgacattctatcttgcaaattcaacaattataataagatataccaaagtagcggtatagtggcaatcaaaaagcttctctggtgtgcttctcgtatttatttttattctaatgatccattaaaggtatatatttatttcttgttatataatccttttgtttattacatgggctggatacataaaggtattttgatttaattttttgcttaaattcaatcccccctcgttcagtgtcaactgtaatggtaggaaattaccatacttttgaagaagcaaaaaaaatgaaagaaaaaaaaaatcgtatttccaggttagacgttccgcagaatctagaatgcggtatgcggtacattgttcttcgaacgtaaaagttgcgctccctgagatattgtacatttttgcttttacaagtacaagtacatcgtacaactatgtactactgttgatgcatccacaacagtttgttttgtttttttttgttttttttttttctaatgattcattaccgctatgtatacctacttgtacttgtagtaagccgggttattggcgttcaattaatcatagacttatgaatctgcacggtgtgcgctgcgagttacttttagcttatgcatgctacttgggtgtaatattgggatctgttcggaaatcaacggatgctcaatcgataaaaaacaaaaaaaaaagcaccgactcggtgccactttttcaagttgataacggactagccttattttaacttgctatttctagc